European Patent Specification EP 3 592 861 B1, published September 3, 2025. Title: RNA profiling for individualized diet and treatment advice. Applicant: Stichting Katholieke Universiteit. The sequence listing filed with the application follows.

SEQUENCE LISTING (951 sequences)

SEQ ID NO: 1 - DNA, 83 bp, Artificial Sequence
  smMIP
  misc_feature (29)..(36): n is a, c, g, or t
cgttgaatttgattatgatgggcctctgnnnnnnnncttcagcttcccgatatccgacggtagtgttgtccctcaaggggtca

SEQ ID NO: 2 - DNA, 82 bp, Artificial Sequence
  smMIP
  misc_feature (23)..(30): n is a, c, g, or t
caacagacccgccctcggaatcnnnnnnnncttcagcttcccgatatccgacggtagtgtttacctggttgatgtggacggc

SEQ ID NO: 3 - DNA, 83 bp, Artificial Sequence
  smMIP
  misc_feature (28)..(35): n is a, c, g, or t
cctctccttcatgggcgcgttccatggnnnnnnnncttcagcttcccgatatccgacggtagtgtaaaacgccttaaagacca

SEQ ID NO: 4 - DNA, 83 bp, Artificial Sequence
  smMIP
  misc_feature (30)..(37): n is a, c, g, or t
gccttcttggtggacgaggtccagaccggnnnnnnnncttcagcttcccgatatccgacggtagtgtggaaaaagaagaagac

SEQ ID NO: 5 - DNA, 83 bp, Artificial Sequence
  smMIP
  misc_feature (30)..(37): n is a, c, g, or t
gattccatacggaataagctcattttaatnnnnnnnncttcagcttcccgatatccgacggtagtgtataatgcagcccatgc

SEQ ID NO: 6 - DNA, 81 bp, Artificial Sequence
  smMIP
  misc_feature (27)..(34): n is a, c, g, or t
gctcattttggaggaataatggatgannnnnnnncttcagcttcccgatatccgacggtagtgtagaggcccaaattgagg

SEQ ID NO: 7 - DNA, 83 bp, Artificial Sequence
  smMIP
  misc_feature (30)..(37): n is a, c, g, or t
gctgggaagttaatccagtacattgtagannnnnnnncttcagcttcccgatatccgacggtagtgtatgatggcagcagtta

SEQ ID NO: 8 - DNA, 83 bp, Artificial Sequence
  smMIP
  misc_feature (20)..(27): n is a, c, g, or t
ctcctccaacctcaaccacnnnnnnnncttcagcttcccgatatccgacggtagtgttattgcctatgaacttaacagcgtac

SEQ ID NO: 9 - DNA, 83 bp, Artificial Sequence
  smMIP
  misc_feature (27)..(34): n is a, c, g, or t
gcaatgacatcacataccgaattgggnnnnnnnncttcagcttcccgatatccgacggtagtgtggatgatcaaggtcagctg

SEQ ID NO: 10 - DNA, 83 bp, Artificial Sequence
  smMIP
  misc_feature (30)..(37): n is a, c, g, or t
gcgctggtttgtggaagtggaaggaacagnnnnnnnncttcagcttcccgatatccgacggtagtgtaaaacatcccgtacct

SEQ ID NO: 11 - DNA, 83 bp, Artificial Sequence
  smMIP
  misc_feature (20)..(27): n is a, c, g, or t
tcccaccagaagcccccaannnnnnnncttcagcttcccgatatccgacggtagtgttctgataactcaggggagacaccgca

SEQ ID NO: 12 - DNA, 83 bp, Artificial Sequence
  smMIP
  misc_feature (26)..(33): n is a, c, g, or t
gcagggacagtggaatacctctatannnnnnnncttcagcttcccgatatccgacggtagtgttgctccatccagcggcggca

SEQ ID NO: 13 - DNA, 83 bp, Artificial Sequence
  smMIP
  misc_feature (28)..(35): n is a, c, g, or t
cccagagcatcgtgcagttggtccagannnnnnnncttcagcttcccgatatccgacggtagtgtcagtatgccagcaacatc

SEQ ID NO: 14 - DNA, 83 bp, Artificial Sequence
  smMIP
  misc_feature (30)..(37): n is a, c, g, or t
ccactgtcatcatggaccccttcaagatcnnnnnnnncttcagcttcccgatatccgacggtagtgtcttcgaatacctgcag

SEQ ID NO: 15 - DNA, 79 bp, Artificial Sequence
  smMIP
  misc_feature (22)..(29): n is a, c, g, or t
gcaggcaggacaggtgtggttnnnnnnnncttcagcttcccgatatccgacggtagtgtagaccgtggtgacaggacga

SEQ ID NO: 16 - DNA, 83 bp, Artificial Sequence
  smMIP
  misc_feature (19)..(26): n is a, c, g, or t
accacctcagccatccagnnnnnnnncttcagcttcccgatatccgacggtagtgtttcgtcgggcctgtggaagaagcgccg

SEQ ID NO: 17 - DNA, 83 bp, Artificial Sequence
  smMIP
  misc_feature (27)..(34): n is a, c, g, or t
gctgaccttgctgaaccccaaagggannnnnnnncttcagcttcccgatatccgacggtagtgtactgccgactacatctgca

SEQ ID NO: 18 - DNA, 80 bp, Artificial Sequence
  smMIP
  misc_feature (27)..(34): n is a, c, g, or t
gctcccgagacgagccctcagtggctnnnnnnnncttcagcttcccgatatccgacggtagtgtaaagaaggccaagcct

SEQ ID NO: 19 - DNA, 83 bp, Artificial Sequence
  smMIP
  misc_feature (26)..(33): n is a, c, g, or t
gccaagaaccaggctttgaaggaagnnnnnnnncttcagcttcccgatatccgacggtagtgtaaggagggccgcctcactaa

SEQ ID NO: 20 - DNA, 83 bp, Artificial Sequence
  smMIP
  misc_feature (29)..(36): n is a, c, g, or t
gctcgattatgcactggaagtagagaagnnnnnnnncttcagcttcccgatatccgacggtagtgtgatgaagaaggaaggga

SEQ ID NO: 21 - DNA, 83 bp, Artificial Sequence
  smMIP
  misc_feature (26)..(33): n is a, c, g, or t
cctggatgaccccgccagccaggaannnnnnnncttcagcttcccgatatccgacggtagtgtggtggcgatgagccactttg

SEQ ID NO: 22 - DNA, 80 bp, Artificial Sequence
  smMIP
  misc_feature (25)..(32): n is a, c, g, or t
cggtgaaaggtggcacaggtgcaannnnnnnncttcagcttcccgatatccgacggtagtgtgtggatgtcatggctggg

SEQ ID NO: 23 - DNA, 83 bp, Artificial Sequence
  smMIP
  misc_feature (30)..(37): n is a, c, g, or t
gctgcaccaattcaagctatgaagatatgnnnnnnnncttcagcttcccgatatccgacggtagtgttgagctgaagccacac

SEQ ID NO: 24 - DNA, 83 bp, Artificial Sequence
  smMIP
  misc_feature (26)..(33): n is a, c, g, or t
gcaaggacctggaggacctgcagatnnnnnnnncttcagcttcccgatatccgacggtagtgtaaggggagtttgacccaggg

SEQ ID NO: 25 - DNA, 82 bp, Artificial Sequence
  smMIP
  misc_feature (26)..(33): n is a, c, g, or t
cgagaccaacctgaagaaacagggcnnnnnnnncttcagcttcccgatatccgacggtagtgttggcatcaggtgggtggtg

SEQ ID NO: 26 - DNA, 83 bp, Artificial Sequence
  smMIP
  misc_feature (30)..(37): n is a, c, g, or t
gcaatgagccaggggagaccactcagatcnnnnnnnncttcagcttcccgatatccgacggtagtgtgactaaagggaaaatc

SEQ ID NO: 27 - DNA, 83 bp, Artificial Sequence
  smMIP
  misc_feature (23)..(30): n is a, c, g, or t
gctgcattgtggtcaagcacctnnnnnnnncttcagcttcccgatatccgacggtagtgttcttggattccagctgcagtctt

SEQ ID NO: 28 - DNA, 83 bp, Artificial Sequence
  smMIP
  misc_feature (23)..(30): n is a, c, g, or t
agcctgtcaccaagcatagccgnnnnnnnncttcagcttcccgatatccgacggtagtgtgtgttttgtttgaggggattccc

SEQ ID NO: 29 - DNA, 83 bp, Artificial Sequence
  smMIP
  misc_feature (19)..(26): n is a, c, g, or t
cgctttgagacaacctacnnnnnnnncttcagcttcccgatatccgacggtagtgttttcccattctttggtgtagctcctgc

SEQ ID NO: 30 - DNA, 83 bp, Artificial Sequence
  smMIP
  misc_feature (21)..(28): n is a, c, g, or t
cttgcctaaaacccgctcagnnnnnnnncttcagcttcccgatatccgacggtagtgttgcctctactgctttgtcaccttgt

SEQ ID NO: 31 - DNA, 83 bp, Artificial Sequence
  smMIP
  misc_feature (25)..(32): n is a, c, g, or t
cactgggagcattgccaagcggctnnnnnnnncttcagcttcccgatatccgacggtagtgtaacttgctactaccagcacca

SEQ ID NO: 32 - DNA, 83 bp, Artificial Sequence
  smMIP
  misc_feature (30)..(37): n is a, c, g, or t
gccatcatggaaaatgccaatgttctggcnnnnnnnncttcagcttcccgatatccgacggtagtgtagactaccacccaagg

SEQ ID NO: 33 - DNA, 83 bp, Artificial Sequence
  smMIP
  misc_feature (25)..(32): n is a, c, g, or t
gctctgagtgaccaccacatctacnnnnnnnncttcagcttcccgatatccgacggtagtgtttatgccagtatctgccagca

SEQ ID NO: 34 - DNA, 83 bp, Artificial Sequence
  smMIP
  misc_feature (28)..(35): n is a, c, g, or t
gaggcgtccatcaacctcaatgccattnnnnnnnncttcagcttcccgatatccgacggtagtgtccatgcttgcactcagaa

SEQ ID NO: 35 - DNA, 82 bp, Artificial Sequence
  smMIP
  misc_feature (29)..(36): n is a, c, g, or t
gcctgtcaaggaaagtacactccgagcgnnnnnnnncttcagcttcccgatatccgacggtagtgtgccctgaccttctcct

SEQ ID NO: 36 - DNA, 83 bp, Artificial Sequence
  smMIP
  misc_feature (30)..(37): n is a, c, g, or t
gtgcataggagatgcagaaacagatgatgnnnnnnnncttcagcttcccgatatccgacggtagtgtgacaagaccaacaaat

SEQ ID NO: 37 - DNA, 83 bp, Artificial Sequence
  smMIP
  misc_feature (25)..(32): n is a, c, g, or t
gtttgtggagcctctgctggccttnnnnnnnncttcagcttcccgatatccgacggtagtgtccaaaaagaaagaatctcagc

SEQ ID NO: 38 - DNA, 83 bp, Artificial Sequence
  smMIP
  misc_feature (30)..(37): n is a, c, g, or t
gtgaagggactgcgcagttggacagcattnnnnnnnncttcagcttcccgatatccgacggtagtgtggaagcagtagacagg

SEQ ID NO: 39 - DNA, 83 bp, Artificial Sequence
  smMIP
  misc_feature (23)..(30): n is a, c, g, or t
cagcatccttaattccagcagcnnnnnnnncttcagcttcccgatatccgacggtagtgttgactccaagcccccgtcctgca

SEQ ID NO: 40 - DNA, 83 bp, Artificial Sequence
  smMIP
  misc_feature (30)..(37): n is a, c, g, or t
gttcacagcaggcacggtcttcgataacgnnnnnnnncttcagcttcccgatatccgacggtagtgtcatccaaacctgcact

SEQ ID NO: 41 - DNA, 83 bp, Artificial Sequence
  smMIP
  misc_feature (26)..(33): n is a, c, g, or t
gctggtatggatcttagggaagcagnnnnnnnncttcagcttcccgatatccgacggtagtgtcgtagtcaagttgccggtgg

SEQ ID NO: 42 - DNA, 83 bp, Artificial Sequence
  smMIP
  misc_feature (29)..(36): n is a, c, g, or t
cagttgcacaggtgttaaaaaaacttgcnnnnnnnncttcagcttcccgatatccgacggtagtgtaagaataccaacgcatc

SEQ ID NO: 43 - DNA, 83 bp, Artificial Sequence
  smMIP
  misc_feature (30)..(37): n is a, c, g, or t
gtgttttaagatgccacagtctttaggggnnnnnnnncttcagcttcccgatatccgacggtagtgtgcttcaaaccagagta

SEQ ID NO: 44 - DNA, 83 bp, Artificial Sequence
  smMIP
  misc_feature (30)..(37): n is a, c, g, or t
tccattgcctgcagtccccacagcgaatgnnnnnnnncttcagcttcccgatatccgacggtagtgtaaaaccaaataacgcg

SEQ ID NO: 45 - DNA, 82 bp, Artificial Sequence
  smMIP
  misc_feature (28)..(35): n is a, c, g, or t
gccaagccagaagtgacaaccactgggnnnnnnnncttcagcttcccgatatccgacggtagtgtcaaagaagaaaaagact

SEQ ID NO: 46 - DNA, 83 bp, Artificial Sequence
  smMIP
  misc_feature (28)..(35): n is a, c, g, or t
gcccgcgtacatgggctgaggaatgttnnnnnnnncttcagcttcccgatatccgacggtagtgtcactcatcttcaaaagac

SEQ ID NO: 47 - DNA, 83 bp, Artificial Sequence
  smMIP
  misc_feature (30)..(37): n is a, c, g, or t
gagttggtctgaaagcccccggtatcattnnnnnnnncttcagcttcccgatatccgacggtagtgtagtgaagaggacagga

SEQ ID NO: 48 - DNA, 83 bp, Artificial Sequence
  smMIP
  misc_feature (24)..(31): n is a, c, g, or t
atgtctctgttgctccgccgaccnnnnnnnncttcagcttcccgatatccgacggtagtgtatgctgccccacttcagtacct

SEQ ID NO: 49 - DNA, 83 bp, Artificial Sequence
  smMIP
  misc_feature (30)..(37): n is a, c, g, or t
gctgcccaaaccagggctatgaagcaggtnnnnnnnncttcagcttcccgatatccgacggtagtgtcttacattccaacaaa

SEQ ID NO: 50 - DNA, 83 bp, Artificial Sequence
  smMIP
  misc_feature (28)..(35): n is a, c, g, or t
gccttgttgggcactatcagggctgatnnnnnnnncttcagcttcccgatatccgacggtagtgtggctattgaagaacaagt

SEQ ID NO: 51 - DNA, 83 bp, Artificial Sequence
  smMIP
  misc_feature (26)..(33): n is a, c, g, or t
gctgagagagagctgaaaccagctcnnnnnnnncttcagcttcccgatatccgacggtagtgtccgcaatggattcaagttcg

SEQ ID NO: 52 - DNA, 82 bp, Artificial Sequence
  smMIP
  misc_feature (27)..(34): n is a, c, g, or t
gttatgcttgttggaattggtgacaannnnnnnncttcagcttcccgatatccgacggtagtgtaagacaagaagaaacacc

SEQ ID NO: 53 - DNA, 83 bp, Artificial Sequence
  smMIP
  misc_feature (22)..(29): n is a, c, g, or t
aaattcaggtctgtcatctccnnnnnnnncttcagcttcccgatatccgacggtagtgtttctgaccagtttctggtggcatt

SEQ ID NO: 54 - DNA, 83 bp, Artificial Sequence
  smMIP
  misc_feature (28)..(35): n is a, c, g, or t
gccaggatgacagccatggacaatgccnnnnnnnncttcagcttcccgatatccgacggtagtgtaagtgctgacagcatgag

SEQ ID NO: 55 - DNA, 83 bp, Artificial Sequence
  smMIP
  misc_feature (30)..(37): n is a, c, g, or t
gttccatcctcagacaagaggtaaagaagnnnnnnnncttcagcttcccgatatccgacggtagtgtgaatgcttctgagatg

SEQ ID NO: 56 - DNA, 83 bp, Artificial Sequence
  smMIP
  misc_feature (19)..(26): n is a, c, g, or t
tagtcacaccagctaccannnnnnnncttcagcttcccgatatccgacggtagtgtccttttttgtgtttgcctgggtcctgg

SEQ ID NO: 57 - DNA, 83 bp, Artificial Sequence
  smMIP
  misc_feature (28)..(35): n is a, c, g, or t
gctgtgagggcaactctgccggtatttnnnnnnnncttcagcttcccgatatccgacggtagtgtccctggctcatcagcttt

SEQ ID NO: 58 - DNA, 83 bp, Artificial Sequence
  smMIP
  misc_feature (30)..(37): n is a, c, g, or t
gtggaactggggactgcaagatgggagggnnnnnnnncttcagcttcccgatatccgacggtagtgtcaagaagcctaccaaa

SEQ ID NO: 59 - DNA, 82 bp, Artificial Sequence
  smMIP
  misc_feature (24)..(31): n is a, c, g, or t
gcatcattcttccaggagtgacannnnnnnncttcagcttcccgatatccgacggtagtgttgggtgtcagcaggtcctgtg

SEQ ID NO: 60 - DNA, 83 bp, Artificial Sequence
  smMIP
  misc_feature (30)..(37): n is a, c, g, or t
gcgagacaatacacattccaactatggagnnnnnnnncttcagcttcccgatatccgacggtagtgtgtcagagagatacctc

SEQ ID NO: 61 - DNA, 83 bp, Artificial Sequence
  smMIP
  misc_feature (20)..(27): n is a, c, g, or t
gcccagtgggtgcctacttnnnnnnnncttcagcttcccgatatccgacggtagtgttcatcgaagtggacaaggactgggtc

SEQ ID NO: 62 - DNA, 82 bp, Artificial Sequence
  smMIP
  misc_feature (29)..(36): n is a, c, g, or t
gcctgccgagtttcgacaagctggagttnnnnnnnncttcagcttcccgatatccgacggtagtgtgcctccactactccct

SEQ ID NO: 63 - DNA, 81 bp, Artificial Sequence
  smMIP
  misc_feature (23)..(30): n is a, c, g, or t
gtgggaattatgggcccaccgtnnnnnnnncttcagcttcccgatatccgacggtagtgtcgctcctgttcgtcattctct

SEQ ID NO: 64 - DNA, 82 bp, Artificial Sequence
  smMIP
  misc_feature (26)..(33): n is a, c, g, or t
gcctggagtggtcagacagagtctannnnnnnncttcagcttcccgatatccgacggtagtgtggtcctctggctgtatggg

SEQ ID NO: 65 - DNA, 83 bp, Artificial Sequence
  smMIP
  misc_feature (24)..(31): n is a, c, g, or t
cctgtacaaagacaggaacctccnnnnnnnncttcagcttcccgatatccgacggtagtgttggggtgagttccgggtggtgg

SEQ ID NO: 66 - DNA, 82 bp, Artificial Sequence
  smMIP
  misc_feature (29)..(36): n is a, c, g, or t
cctgatggggagaatagctggtccaagannnnnnnncttcagcttcccgatatccgacggtagtgtcaggagcccgcgaaga

SEQ ID NO: 67 - DNA, 83 bp, Artificial Sequence
  smMIP
  misc_feature (22)..(29): n is a, c, g, or t
acccgcacggctctgagcacannnnnnnncttcagcttcccgatatccgacggtagtgtaacaagcagtttctcctgaccaac

SEQ ID NO: 68 - DNA, 83 bp, Artificial Sequence
  smMIP
  misc_feature (28)..(35): n is a, c, g, or t
caccttcaacatgtaaagtacaaaggcnnnnnnnncttcagcttcccgatatccgacggtagtgtccattataactcagacct

SEQ ID NO: 69 - DNA, 83 bp, Artificial Sequence
  smMIP
  misc_feature (21)..(28): n is a, c, g, or t
gctgctggctttggagacagnnnnnnnncttcagcttcccgatatccgacggtagtgtaacattgaagagctgcttccggaga

SEQ ID NO: 70 - DNA, 83 bp, Artificial Sequence
  smMIP
  misc_feature (24)..(31): n is a, c, g, or t
gtggtggtgtccatttggcttttnnnnnnnncttcagcttcccgatatccgacggtagtgtcccccagagaaatgatcaacaa

SEQ ID NO: 71 - DNA, 83 bp, Artificial Sequence
  smMIP
  misc_feature (30)..(37): n is a, c, g, or t
gcccagtgaagaggattcacccagagaggnnnnnnnncttcagcttcccgatatccgacggtagtgtctgctgctgtcactgc

SEQ ID NO: 72 - DNA, 83 bp, Artificial Sequence
  smMIP
  misc_feature (27)..(34): n is a, c, g, or t
gaggctcctggagatcctcaagaaccnnnnnnnncttcagcttcccgatatccgacggtagtgtaggatccacccggagagga

SEQ ID NO: 73 - DNA, 83 bp, Artificial Sequence
  smMIP
  misc_feature (21)..(28): n is a, c, g, or t
ccctctgacttcagccgctannnnnnnncttcagcttcccgatatccgacggtagtgttgttggccgcctttctggaggaggg

SEQ ID NO: 74 - DNA, 82 bp, Artificial Sequence
  smMIP
  misc_feature (29)..(36): n is a, c, g, or t
gcgacgcagcctttgaatgggcgagtgannnnnnnncttcagcttcccgatatccgacggtagtgttgtgcccagggtgtca

SEQ ID NO: 75 - DNA, 82 bp, Artificial Sequence
  smMIP
  misc_feature (29)..(36): n is a, c, g, or t
gcagatgagaaggcagcacagaaggggannnnnnnncttcagcttcccgatatccgacggtagtgttggagtggacagcagt

SEQ ID NO: 76 - DNA, 83 bp, Artificial Sequence
  smMIP
  misc_feature (27)..(34): n is a, c, g, or t
gttgctgatcccacaccctttcatatnnnnnnnncttcagcttcccgatatccgacggtagtgttgagcccgcgcttccacca

SEQ ID NO: 77 - DNA, 83 bp, Artificial Sequence
  smMIP
  misc_feature (21)..(28): n is a, c, g, or t
ccccaagcatcctgcgtactnnnnnnnncttcagcttcccgatatccgacggtagtgttggtcaacaacgcgggcatcgcctt

SEQ ID NO: 78 - DNA, 83 bp, Artificial Sequence
  smMIP
  misc_feature (26)..(33): n is a, c, g, or t
atctgccgctgcttaactctgggccnnnnnnnncttcagcttcccgatatccgacggtagtgttgcacagaattactccctct

SEQ ID NO: 79 - DNA, 83 bp, Artificial Sequence
  smMIP
  misc_feature (30)..(37): n is a, c, g, or t
gtctttggttgtaaactgctgtgatagttnnnnnnnncttcagcttcccgatatccgacggtagtgtaggaggaaagtccaag

SEQ ID NO: 80 - DNA, 83 bp, Artificial Sequence
  smMIP
  misc_feature (24)..(31): n is a, c, g, or t
ccctgtggatccggcccgatgctnnnnnnnncttcagcttcccgatatccgacggtagtgttcccagcatgccttctgagacc

SEQ ID NO: 81 - DNA, 82 bp, Artificial Sequence
  smMIP
  misc_feature (25)..(32): n is a, c, g, or t
gctcttggccaagtgtgagttcttnnnnnnnncttcagcttcccgatatccgacggtagtgtagtccccacatcaccacact

SEQ ID NO: 82 - DNA, 80 bp, Artificial Sequence
  smMIP
  misc_feature (20)..(27): n is a, c, g, or t
cggagtcacacgtgggggtnnnnnnnncttcagcttcccgatatccgacggtagtgttggctgcggcagtgaggggctat

SEQ ID NO: 83 - DNA, 83 bp, Artificial Sequence
  smMIP
  misc_feature (30)..(37): n is a, c, g, or t
gcaagaggggctgctgtgcggtggcagtgnnnnnnnncttcagcttcccgatatccgacggtagtgtacctacgaggtggaag

SEQ ID NO: 84 - DNA, 82 bp, Artificial Sequence
  smMIP
  misc_feature (25)..(32): n is a, c, g, or t
gctctcgcacatcctggagatggannnnnnnncttcagcttcccgatatccgacggtagtgttgggaatggtgacgcttggg

SEQ ID NO: 85 - DNA, 83 bp, Artificial Sequence
  smMIP
  misc_feature (26)..(33): n is a, c, g, or t
acaccacagccacccttggtgatgannnnnnnncttcagcttcccgatatccgacggtagtgtgcagggcctatctgtggtgc

SEQ ID NO: 86 - DNA, 83 bp, Artificial Sequence
  smMIP
  misc_feature (29)..(36): n is a, c, g, or t
gccggcgattagatactgaagaattaagnnnnnnnncttcagcttcccgatatccgacggtagtgttgcagatgggggctgag

SEQ ID NO: 87 - DNA, 83 bp, Artificial Sequence
  smMIP
  misc_feature (30)..(37): n is a, c, g, or t
gctcagttacaatctgcccttggaactggnnnnnnnncttcagcttcccgatatccgacggtagtgtggtatgaaaatgccat

SEQ ID NO: 88 - DNA, 82 bp, Artificial Sequence
  smMIP
  misc_feature (29)..(36): n is a, c, g, or t
ccagttacttgcctgcattccaaaatgannnnnnnncttcagcttcccgatatccgacggtagtgtggggattcgacattgg

SEQ ID NO: 89 - DNA, 82 bp, Artificial Sequence
  smMIP
  misc_feature (29)..(36): n is a, c, g, or t
gcaaggtttgatgcctatttccaccagannnnnnnncttcagcttcccgatatccgacggtagtgtaaagaagaaatgttgc

SEQ ID NO: 90 - DNA, 82 bp, Artificial Sequence
  smMIP
  misc_feature (22)..(29): n is a, c, g, or t
ccacctgcgggtcatctccatnnnnnnnncttcagcttcccgatatccgacggtagtgtaccacttcctcttcgacaagccc

SEQ ID NO: 91 - DNA, 83 bp, Artificial Sequence
  smMIP
  misc_feature (30)..(37): n is a, c, g, or t
gcgacgacctggaccccaactacgtgctgnnnnnnnncttcagcttcccgatatccgacggtagtgtcgacgaggagtcctac

SEQ ID NO: 92 - DNA, 83 bp, Artificial Sequence
  smMIP
  misc_feature (28)..(35): n is a, c, g, or t
ggactatgagttcatgtggaaccctcannnnnnnncttcagcttcccgatatccgacggtagtgttggtgtgggtcaacgagg

SEQ ID NO: 93 - DNA, 81 bp, Artificial Sequence
  smMIP
  misc_feature (24)..(31): n is a, c, g, or t
gcacaggcggtgtggacacggctnnnnnnnncttcagcttcccgatatccgacggtagtgtctacatcctcacctgcccat

SEQ ID NO: 94 - DNA, 82 bp, Artificial Sequence
  smMIP
  misc_feature (24)..(31): n is a, c, g, or t
gtggtggacggagtgaagctgctnnnnnnnncttcagcttcccgatatccgacggtagtgtaggtgcttaagcggctgcgac

SEQ ID NO: 95 - DNA, 83 bp, Artificial Sequence
  smMIP
  misc_feature (28)..(35): n is a, c, g, or t
ggacttcattcctggaaaaagaagttcnnnnnnnncttcagcttcccgatatccgacggtagtgtgctgactcggtactctct

SEQ ID NO: 96 - DNA, 83 bp, Artificial Sequence
  smMIP
  misc_feature (30)..(37): n is a, c, g, or t
gatctggatgggtatggtcaagatcttttnnnnnnnncttcagcttcccgatatccgacggtagtgtgtgctgtttggcaccg

SEQ ID NO: 97 - DNA, 83 bp, Artificial Sequence
  smMIP
  misc_feature (27)..(34): n is a, c, g, or t
gcacatgagagacagcaagcacatcgnnnnnnnncttcagcttcccgatatccgacggtagtgtaaactggaccgggaggaaa

SEQ ID NO: 98 - DNA, 83 bp, Artificial Sequence
  smMIP
  misc_feature (30)..(37): n is a, c, g, or t
gctggcgcactacaaggacatgggcaagtnnnnnnnncttcagcttcccgatatccgacggtagtgtaacaccgcaaatcttc

SEQ ID NO: 99 - DNA, 83 bp, Artificial Sequence
  smMIP
  misc_feature (30)..(37): n is a, c, g, or t
gtttgacttggagaataacccagagtacgnnnnnnnncttcagcttcccgatatccgacggtagtgtcacctcttctgccttt

SEQ ID NO: 100 - DNA, 82 bp, Artificial Sequence
  smMIP
  misc_feature (28)..(35): n is a, c, g, or t
ggtctctttgggcggaagacaggtcagnnnnnnnncttcagcttcccgatatccgacggtagtgtgcgactaaaaagagaat

SEQ ID NO: 101 - DNA, 83 bp, Artificial Sequence
  smMIP
  misc_feature (30)..(37): n is a, c, g, or t
gggagaggatacactgatggagtatttggnnnnnnnncttcagcttcccgatatccgacggtagtgtaccgttgaaaagggag

SEQ ID NO: 102 - DNA, 83 bp, Artificial Sequence
  smMIP
  misc_feature (30)..(37): n is a, c, g, or t
ggaagaaagggcagacttaatagcttatcnnnnnnnncttcagcttcccgatatccgacggtagtgttacacagccgccaata

SEQ ID NO: 103 - DNA, 83 bp, Artificial Sequence
  smMIP
  misc_feature (29)..(36): n is a, c, g, or t
cttttttatgtgtaccatcctttaatagnnnnnnnncttcagcttcccgatatccgacggtagtgttgatctttgtcggcatt

SEQ ID NO: 104 - DNA, 81 bp, Artificial Sequence
  smMIP
  misc_feature (27)..(34): n is a, c, g, or t
cgggcagctggtcagccagaagagtgnnnnnnnncttcagcttcccgatatccgacggtagtgtgagtacatcgtgccgtg

SEQ ID NO: 105 - DNA, 81 bp, Artificial Sequence
  smMIP
  misc_feature (26)..(33): n is a, c, g, or t
ggaacgggttatgtacgtcatgttgnnnnnnnncttcagcttcccgatatccgacggtagtgtggctgcgaaaccattggg

SEQ ID NO: 106 - DNA, 81 bp, Artificial Sequence
  smMIP
  misc_feature (26)..(33): n is a, c, g, or t
gatagactgctgtttttctggtctgnnnnnnnncttcagcttcccgatatccgacggtagtgtggagatggaagatgtgtg

SEQ ID NO: 107 - DNA, 83 bp, Artificial Sequence
  smMIP
  misc_feature (27)..(34): n is a, c, g, or t
ggtcggtaaagacgtcttctagagccnnnnnnnncttcagcttcccgatatccgacggtagtgtgcatatgctacaaggtacg

SEQ ID NO: 108 - DNA, 83 bp, Artificial Sequence
  smMIP
  misc_feature (27)..(34): n is a, c, g, or t
gtgaatacgaataaatgggataaagannnnnnnncttcagcttcccgatatccgacggtagtgtggtgaaaaaggtgtgaggg

SEQ ID NO: 109 - DNA, 83 bp, Artificial Sequence
  smMIP
  misc_feature (29)..(36): n is a, c, g, or t
gctgtgcccagtggtgcttcaactggtannnnnnnncttcagcttcccgatatccgacggtagtgtagacccagtggctagaa

SEQ ID NO: 110 - DNA, 82 bp, Artificial Sequence
  smMIP
  misc_feature (20)..(27): n is a, c, g, or t
gcggttctcatgctggcaannnnnnnncttcagcttcccgatatccgacggtagtgtttctgggggtgtcccttgccgtctg

SEQ ID NO: 111 - DNA, 83 bp, Artificial Sequence
  smMIP
  misc_feature (28)..(35): n is a, c, g, or t
gcctgaccagctggctgacctgtacaannnnnnnncttcagcttcccgatatccgacggtagtgtttgggaaagctggctaca

SEQ ID NO: 112 - DNA, 83 bp, Artificial Sequence
  smMIP
  misc_feature (29)..(36): n is a, c, g, or t
gccaatggttggggcgtcatggtgtctcnnnnnnnncttcagcttcccgatatccgacggtagtgtacagtgaccaacccaaa

SEQ ID NO: 113 - DNA, 83 bp, Artificial Sequence
  smMIP
  misc_feature (26)..(33): n is a, c, g, or t
cggcaggaacttcagaaaccccttgnnnnnnnncttcagcttcccgatatccgacggtagtgttgacctggttgtggggctgt

SEQ ID NO: 114 - DNA, 82 bp, Artificial Sequence
  smMIP
  misc_feature (19)..(26): n is a, c, g, or t
cccagcccccacccacaannnnnnnncttcagcttcccgatatccgacggtagtgttccacagcctggctgcctactacatc

SEQ ID NO: 115 - DNA, 81 bp, Artificial Sequence
  smMIP
  misc_feature (28)..(35): n is a, c, g, or t
cgtggagcagctgaggaaggagggtgtnnnnnnnncttcagcttcccgatatccgacggtagtgttggcagccgtgggctt

SEQ ID NO: 116 - DNA, 82 bp, Artificial Sequence
  smMIP
  misc_feature (25)..(32): n is a, c, g, or t
gccatccagataggcctcatagacnnnnnnnncttcagcttcccgatatccgacggtagtgtcttccgagattccatcctac

SEQ ID NO: 117 - DNA, 81 bp, Artificial Sequence
  smMIP
  misc_feature (27)..(34): n is a, c, g, or t
gcgttcttcaacgagagcagtgctgannnnnnnncttcagcttcccgatatccgacggtagtgtgcgtgaggtgcttggct

SEQ ID NO: 118 - DNA, 80 bp, Artificial Sequence
  smMIP
  misc_feature (20)..(27): n is a, c, g, or t
gtgctggctgagaaggctgnnnnnnnncttcagcttcccgatatccgacggtagtgtgtgggcattttggtggagacgat

SEQ ID NO: 119 - DNA, 79 bp, Artificial Sequence
  smMIP
  misc_feature (25)..(32): n is a, c, g, or t
gggcctagaggagcgtgtggcagcnnnnnnnncttcagcttcccgatatccgacggtagtgtagagctaccgggcaaag

SEQ ID NO: 120 - DNA, 83 bp, Artificial Sequence
  smMIP
  misc_feature (30)..(37): n is a, c, g, or t
gctgtgggcattaaactcctttgggtagcnnnnnnnncttcagcttcccgatatccgacggtagtgtcaacacattacctcca

SEQ ID NO: 121 - DNA, 82 bp, Artificial Sequence
  smMIP
  misc_feature (26)..(33): n is a, c, g, or t
gccgacctacagatttcggtgcttgnnnnnnnncttcagcttcccgatatccgacggtagtgtgataaagcagttccctgta

SEQ ID NO: 122 - DNA, 83 bp, Artificial Sequence
  smMIP
  misc_feature (19)..(26): n is a, c, g, or t
gcatctataatgccagccnnnnnnnncttcagcttcccgatatccgacggtagtgttggttgggattctgggctgtgcagctg

SEQ ID NO: 123 - DNA, 83 bp, Artificial Sequence
  smMIP
  misc_feature (20)..(27): n is a, c, g, or t
caccctttgccagcctcctnnnnnnnncttcagcttcccgatatccgacggtagtgtttaccttcttcctgttcagcttcgcc

SEQ ID NO: 124 - DNA, 82 bp, Artificial Sequence
  smMIP
  misc_feature (28)..(35): n is a, c, g, or t
cgtcttgtccttctgcaagagtgcggtnnnnnnnncttcagcttcccgatatccgacggtagtgtagagctgcaaggggaaa

SEQ ID NO: 125 - DNA, 83 bp, Artificial Sequence
  smMIP
  misc_feature (30)..(37): n is a, c, g, or t
cagagtgagcccttcttcaaggccaccccnnnnnnnncttcagcttcccgatatccgacggtagtgtacctggccaagaagaa

SEQ ID NO: 126 - DNA, 82 bp, Artificial Sequence
  smMIP
  misc_feature (26)..(33): n is a, c, g, or t
acctgcagagctctgaccggctgtcnnnnnnnncttcagcttcccgatatccgacggtagtgtccaaccgcctcttctacct

SEQ ID NO: 127 - DNA, 83 bp, Artificial Sequence
  smMIP
  misc_feature (25)..(32): n is a, c, g, or t
gtacgtggggaaccccgatggagannnnnnnncttcagcttcccgatatccgacggtagtgttgcagatgctgtgtctggtgg

SEQ ID NO: 128 - DNA, 83 bp, Artificial Sequence
  smMIP
  misc_feature (27)..(34): n is a, c, g, or t
gacgtcttctgcgggagccagatgcannnnnnnncttcagcttcccgatatccgacggtagtgtacaccaagatgatgaccaa

SEQ ID NO: 129 - DNA, 82 bp, Artificial Sequence
  smMIP
  misc_feature (25)..(32): n is a, c, g, or t
ccagtatgagggcacctacaagtgnnnnnnnncttcagcttcccgatatccgacggtagtgtgtgaggcctggcgtattttc

SEQ ID NO: 130 - DNA, 83 bp, Artificial Sequence
  smMIP
  misc_feature (28)..(35): n is a, c, g, or t
gaagagtcgccttgtgagtgccttcaannnnnnnncttcagcttcccgatatccgacggtagtgtaccccaataccactaacc

SEQ ID NO: 131 - DNA, 83 bp, Artificial Sequence
  smMIP
  misc_feature (29)..(36): n is a, c, g, or t
gcacaggtcatcctcgatttttcaaccannnnnnnncttcagcttcccgatatccgacggtagtgtactttcatcacccacac

SEQ ID NO: 132 - DNA, 83 bp, Artificial Sequence
  smMIP
  misc_feature (29)..(36): n is a, c, g, or t
gataaagtgcaatgaaagggggaaaatannnnnnnncttcagcttcccgatatccgacggtagtgtggaagttaagacaaagg

SEQ ID NO: 133 - DNA, 82 bp, Artificial Sequence
  smMIP
  misc_feature (29)..(36): n is a, c, g, or t
gatgtctcctacgacaccggggacaaggnnnnnnnncttcagcttcccgatatccgacggtagtgtaaccctcacaagatga

SEQ ID NO: 134 - DNA, 83 bp, Artificial Sequence
  smMIP
  misc_feature (28)..(35): n is a, c, g, or t
ttccggatggtcatctccaacccagccnnnnnnnncttcagcttcccgatatccgacggtagtgttgtgccagacagccctca

SEQ ID NO: 135 - DNA, 83 bp, Artificial Sequence
  smMIP
  misc_feature (30)..(37): n is a, c, g, or t
ccccttcattgacctcaactacatggtttnnnnnnnncttcagcttcccgatatccgacggtagtgtccacatcgctcagaca

SEQ ID NO: 136 - DNA, 83 bp, Artificial Sequence
  smMIP
  misc_feature (26)..(33): n is a, c, g, or t
gctggcgctgagtacgtcgtggagtnnnnnnnncttcagcttcccgatatccgacggtagtgtcaatatgattccacccatgg

SEQ ID NO: 137 - DNA, 83 bp, Artificial Sequence
  smMIP
  misc_feature (23)..(30): n is a, c, g, or t
ccatcactgccacccagaagacnnnnnnnncttcagcttcccgatatccgacggtagtgtatgagaagtatgacaacagcctc

SEQ ID NO: 138 - DNA, 82 bp, Artificial Sequence
  smMIP
  misc_feature (24)..(31): n is a, c, g, or t
gccaacgtgtcagtggtggacctnnnnnnnncttcagcttcccgatatccgacggtagtgttgtggcgtgatggccgcgggg

SEQ ID NO: 139 - DNA, 83 bp, Artificial Sequence
  smMIP
  misc_feature (29)..(36): n is a, c, g, or t
gcattgccctcaacgaccactttgtcaannnnnnnncttcagcttcccgatatccgacggtagtgtagaaggtggtgaagcag

SEQ ID NO: 140 - DNA, 83 bp, Artificial Sequence
  smMIP
  misc_feature (30)..(37): n is a, c, g, or t
gaaaataaaaaagtccggttggtcctgtcnnnnnnnncttcagcttcccgatatccgacggtagtgtaccacgtgcggcggca

SEQ ID NO: 141 - DNA, 83 bp, Artificial Sequence
  smMIP
  misc_feature (21)..(28): n is a, c, g, or t
cctcgcttcagtaccttaacnnnnnnnncttcagcttcccgatatccgacggtagtgtctctttgcacaataacttcatttcc

SEQ ID NO: 142 - DNA, 83 bp, Artificial Sequence
  smMIP
  misc_feature (30)..(37): n is a, c, g, or t
gatcagtaaatcccgatatgactcaatagnnnnnnnncttcagcttcccgatatccgacggtagtgttctcccttttaccgag

SEQ ID NO: 143 - DNA, 83 bp, Artificial Sequence
  smMIP
  misc_feature (30)..(37): n is a, c, g, or t
cctacaaattggattttctcattccactgnnnnnnnncttcagcttcccgatatccgacggtagtgtccctcctccaaactca

SEQ ID NO: 144 - DNA, 83 bp, Artificial Sequence
  smMIP
  misc_feature (28)..(35): n is a, c, g, or t
gaactaatgacagttgccagatggatgnnnnnnnncttcagcttcccgatatccgacggtagtgtggaaggtgtgtttcctgg

SEQ ID NO: 145 - DNA, 83 bp, Artificial Sequence
  smMIP
  misc_feature (30)..(37): n is a, c, g, or t
gaaatgaaagtttctgcaaaactgttcatnnnnnnnncttcagcttcccgatatccgacggtagtgttgctgaactggggccg

SEQ ID NO: 146 - DNA, 83 bp, Artificial Sequence
  smMIP
  misc_feature (27)..(34): n is a, c, g, or t
gcaaaaagattgttgccataggtaccnnnnnnnncttcagcttcccgatatccgacggtagtgtttcagtccttggagttgca

SEQ ID NO: 147 - DNA, 83 bp, Artificial Sequence
  smMIP
  misc_feature (28)..(35): n is a, c, g, or t
gctttctgaagcaagtttccaagaagcnnnnnnnncttcagcttcccgatatccgacggtagtgtcacaggtaaaaccaaata

SEQ ID NO: 148 - DNA, 83 bp, Artificial Sequence
  smMIP
  misc_feature (29)..(36): n is a, c, g, or t
gctactgcggtattcggtcattgtgaaannnnnnnncttcagcttcccgatatccgacggtagtgtacaatttgacatacagc

SEQ ID NO: 149 - DNA, 83 bp, Artificial Sequence
  smMIP
  misc_feature (30)..(37): n is a, c, g, or t
cttacctgtaatttccttcaatatgagagnnnnnnnncttcagcttcccgatatccgacggtagtgtgagtgggtgccgctgt

SEQ ID NO: 150 - DNA, 83 bp, Artificial Sequence
  smMIP
  misc_feature (26)..(33): n is a, c, g, or t
gcactggatgaagaagttcacaagcnnnnnnnncttcagcttcccgatatccgacggtagtgtggccttcagagactggagta

SEQ ID NO: 151 - DNA, 81 bp, Artificial Sequence
  smMIP
  misc_feature (28)..(35): n is a, c, g, or t
gccctctgttgattggtgtacggagtgnnnnnnnncttcagcttcccgatatccgacggtagtgtgaaagtcaagatacca

SEQ ID NO: 152 - DNA, 83 bp, Artificial Sequence
  smMIP
  misc_feature (28)..(35): n is a, c, g, or t
cactccagatggaactccagcagatcannnnnnnncttcagcttcccgatatccgacggtagtgtatagaacacaccaatcgc

SEQ ID NO: 153 - DNA, 83 bp, Artificial Sequence
  smMIP
  misc_feature (29)..(36): n is a, c, g, or t
gtttgcccttatgatgtgtgatgatcggnnnnnnnncttcagcttcccgatatccgacggtagtgtcacaaacacagttggca

SEQ ID NO: 154 - DNA, 83 bp, Artificial Sequence
  smMIP
  misc_feature (25)..(32): n is a, c, g, or t
gctcttcagcaagtggttgctcggnnnnnnnncttcagcttcccgatatccgacggtagtgttacttatatgcactctgaagg

SEQ ID NO: 155 - DNA, 83 bp, Artificial Sequence
  smMIP
  misc_feature (30)..(37): n is a, c, g, or t
gacggtccctgccaacatccgtttgaaaannnnnnnncttcagcttcccgatatccgacggtagtgtctggagcgccttctgc

SEQ ID NO: 156 - DNA, 82 bp, Artificial Sequence
  smMIP
  misc_feature (29)..(36): n is a, c, g, or t
cagacacggaggggaaggtggaagacttnnnnnnnncttcagcttcccgatatccgacggtagtgtacccacagacaatagc

SEQ ID NO: 157 - DNA, 83 bp, Artificial Sequence
  smMIP
  misc_feature (28)..(35): n is a, c, g, or t
gcatgattccactgggatcctgcaccannnnnnnncttcagcttcccgatatccgacggtagtgtgggtctgtgttcaagagg

SEQ ID NO: 158 - DNA, 82 bp, Artificial Sequence
  smMIP
  misc_feature (28)..(35): n is a, c, g, or t
gccctggagacttcgggtctgatgtctnnnnnnnncttcagcttcccgatatccgacggtagtgtacatacccatccaccaa

SEQ ID NO: 159 - DNA, 83 bp, Artificial Sequence
  smMIP
  misc_feature (29)..(36): n is a, c, g, or t
actgagtcggaggacaaggcagagctggnnnnnnnncttcagcttcccgatatccgacggtagtgtacgagacccttcaaaaa

SEQ ID NO: 160 - DNA, 82 bp, Artificial Sequence
  smMIP
  misc_feature (26)..(33): n is a, c, g, or t
gctgaaggacaagagaaaatacctgnnnnnnnncttcagcttcccgatatccgacggtagtgtaaggacggccccggggaga

SEQ ID NO: 161 - DNA, 83 bp, Artificial Sequence
  smMIP
  misc_feature (30)..(37): n is a, c, g, or t
ggttgcagattatattcctcaactggccannnnnnnncttcagcttcccgatatccgacggtagtgtcagagcaacattgttt

SEQ ID NO: 162 - DNA, 83 bp, Artificial Sequence
  smMIP
  misc_feature (26)..(33): n is a, c, g, or t
gctggagcaattgttgtgacttcacnnnnnnnncttcagcttcccgatatccgacggtagtgtgccattgctgttaatgatct

SEQ ID NO: 163 - DNA, 83 bp, Artificial Sequence
  smMIP
  misc_feature (30)..(37): n is a, c, g, or t
gcagttcgaaatacattgagtttgatgcannnnnnnncttcagcttcccgatatccgacggtagtgttagacttctacttcca

SEQ ID NO: 164 - DNA, 83 bp, Artificial Sequence
  smMIP
  misc_feature (30)..(37): n is a, c, g, or t
gaaggtggtgatcaaaggcattcctttggnnnnnnnncttcagcttcccgatatccgacggtagtgtctctggataagatggg

SEQ ID NO: 165 - DNA, 82 bp, Artificial Sequence
  smMIP
  misc_feature (29)..(36): n is a, c, g, or t
gcggcatcctgcggatcatcaagccctgnnnnnnnncttcagcttcccgatatccgacggtagtgtacgaccccaacttctt

SEQ ID NO: 166 - DNA, 83 bp, Artificial Sequence
  smMIP
  misc_feature (30)..(37): n is a, c, g, or t
gtgagcgggagatgtcctggatcgctgatnnnnnnnncttcagcttcccgatatccgacggtagtgtcaatcccaagaactat

SEQ ID NO: 167 - DNA, 83 bp, Artificial Sequence
  smMIP
  misc_feature (28)..(35): n is a, c, g, or t
gctaaatgtattgctgttggtgagtctnnnnnnnncttcagcttcccgatatccgacggtagtgtcatcaatgaagcttctta

SEQ ID NO: 168 - DNA, 82 bp, Artificial Sequence
  smMIP
  misc_feature (29)..(36): n is a, c, g, or t
gctgacaagatcttcctggagagaaacannnnnnnncttcagcttcccgatatccgacggtagtgtttggaggccgactgtg

SEQ ID NO: 169 - DNA, 83 bp, Artificial Sequence
  smMIP
  misc_feature (30)..(37): n is a, c, g, or t
gcactctggcttggcatacacaatggagcnnnnnnnncttcagcttcccgatatccgacggtagtgtttgctcatgtctgttc

SEQ ID NO: 170 - DNA, 81 bp, Artificial Sequence
  smMIP
  misc_feature (26)..(33): n is a, c, g, or t
gcgaggagcagaagcggaaccgggtnnnnnnnncttcagcttcccgatatccgacggtagtgtactacagcgagttggtgg

SEQ ID NO: 171 - DNA, 83 bp, Artificial Sequence
  smMIP
  misc_feature (30)..(37): n is a, c, g, or t
accgaaaatgaattggaaaagatcacaagnnnnnnnncttcagcttcccgatatccgacggtagtgtgcactgatgtgagtgt

SEQ ID NO: 172 - DNA, 83 bp, Artificial Sequence
  smMIP
  misc_feature (29)..(36): n is a, c, g, or t
gcattttaggaatgacaccagggtttagnnnnnnnncttcagcttcccgatatccgacggtagtgtatgcacacgcctgtgtt

SEQ ID NO: 173 - DNA, 83 bp, Artificial Sequence
  smMIP
  misc_feature (27)..(34): n is a, c, g, or t
tcgactgtgacatactgatcccagctnnnnnnnncttcagcttcccgatatccgacggtagtgtgtctgatgggagtatatgg

SEQ ID NO: 174 - DNA, 83 bp, Artificial Sequence
  smMIP
  misc_feature (30)..(37): n is a, c, g, or t
gccaggcaaattatgcacacagccatgaannnnnnnncttcagcttcccgatatccgacggtagtgtaatttggaaagcatgg

SEQ ID NO: 175 - DNA, 79 bp, Artificial Sequence
  smMIP
  misc_feature (26)..(33): n is a, c, g, or t
gacccccgcaaggtcaacctgggagnnnnnnnncttcagcttcccgatatccgacggtagtgtgggcgtggggtgaaat

SEQ ID NO: 176 - DNA, 81 bp, Artificial Sequence
  smMIP
  misc_feature (20)..(27): n is a, c, g, or t
caaacaacaagaacacaccnnnnnnnncttcagcttcccgatatccgacggtagtgtgtgcttctcgtcttgcccttgggg

SEQ ID NO: 177 - DNA, 82 bp, Artificial Sequence
  smMIP
  misc_feature (27)..(34): n is a, c, g, or t
gactcagcctatcagggcttcgcatcnnnnnnnncttcagcttcccgatatccgacggtagtgtctcctgagttctccattg

SEQ ID NO: 178 - DNA, 83 bp, Artificial Sequence
  smMIP
  misc_feature (20)..(27): n is a, c, g, or t
cctgcaagtcctttcccagnnnnnnnncttcagcttcccgatatccgacggtagtgttgcctgggccattcgctattttgtgt

SEQ ID NO: 179 - DNA, 83 bp, Artificial Sequence
  smMIP
  misc_feature (28)..(35): n is a, c, g, or t
agccctcaaaacccctgggacctggaannnnnnnncttcagcttcccgatatccgacggtagtgtagggagcacgaattgtgg

SEQ ID NO: 180 - DNA, 83 bp, Artificial Sequence
  smMIP
  misc_feature (30)..(37): n is a, c, g, or t
gctttgaccagtggggagtggagctgggannnnnnnncttcagcttcccgatatccgacggtagtgttgaaggaaatcgccca

SEQ ID NO: 181 - DNA, 83 bp, Artificial Sequence
  smMIP
  misc_feature (26)..(33): n is a, c, g, or t
gctcatcaacttcatcaagcagcagnnnnnnnncttcagcttcccgatatccgacggtagtgtcatcatctgggacatcaaca

SEQ ID NO: 182 - DNA, 83 bp, Artificial Sequence
  smMIP
  misc_feature (25)..(32): n is a, c, g, or t
gtgctcatctgcagcctcctctgtnnnnnnnncttcagcttcccgatatccgacggtagtgtaagcagctggctaagaaaata

SEQ ID NO: 183 - DNA, 78 bp, Artificial Sequence
  smMIP
  misc_feature (25)..(32): n is a, c, g, or t
ggagctgcgccagggtgtgaagaannnnnnnncttcagcttcccgatatccgacggtagtgtggagccaggcggtgag

SEQ ID NO: 184 - DNA, 82 bp, Artificial Sequence
  smMIP
  misc_feature (29)..(36): n is a, c, g, or t
gcatggactgagggcgaaggtgctgacgnnnnnnnncttcagcttcccgatatccgacggtagtgtcactaagccagaccca

SEQ ID NO: 185 - DNA, 83 bp, Artificial Sequence
  smMIP
  misc_feature (21)..(28): n is a, c, g, or t
gggcagaggcccatcaccttnnnnnnnncttcagcttcccgatatccgacggtagtgtggagagtggagtacgcagtgcgtgg

SEQ ID NO: 186 - DNA, 82 bp, Artificial Sequence
  smMIP
  misc_feature (23)..(30): n is a, c, g, or t
cgatgccaagaaaagggcggagnnnnnnnncttcagcttcccgatatccgacggtagtgttttcaccgaggtcatccgtgcc

SEQ ID NO: 187 - DNA, 78 bp, Artificial Sequence
  smMIP
  misc_feature (23)..(30): n is a, c, g, or t
gctgggtcgccctggactgtgtnnnnnnnncttcagcttcccgatatccgacggtagtgtaaggcacctaccacttcc

SEQ ID NO: 188 - DNA, 83 bp, Artificial Sequence
  smMIP
  misc_feature (28)..(35): n is a, c, g, or t
tggagaaggactgcgctgcaagacccgnnnnnnnncttcagcttcccgatatccgacggtagtgtaacgaacaccttccacca

SEQ ID NO: 189 - DNA, 83 bp, Artificial Sequence
  smMIP
  misc_feature (23)..(30): n is a, c, g, or t
acatggtgagcaaccagcacccnnnnnnnncttcagcttcccgatatccgacggtagtgttcgtgcctgctgccatgtttcgg

SEQ ID NO: 190 - DNA, 83 bp, Artificial Sequence
  smMIP
  misc_feature (28)..(35): n is a, c, g, or t
gcttgtatgctggagtcaagattgcggnnnnnnnncttcagcttcccgatatccgacggtagtgtacagatgggcaccccttt

SEQ ID NO: 191 - DNA, 82 bp, Artificial Sequence
  smMIP
  misc_feature (26)..(33): n is a, c, g, or t
cgaggaggccattgagaaactaagcnnnnnnnncttcagcttcccgatatccgacggtagtgtgtgtgaagactttggagtg

SEQ ID NO: 192 - DNA, 83 bp, Artificial Sequence
  smMIP
  misc_feature (23)..(30): n is a, c, g, or t
cctcatccgcacgtgtcttctcnnnnnnnncttcagcttcccgatatccgacggtagtgtcttttctgctggtgtagccaatc

SEQ ID NO: 193 - DNA, 82 bp, Artificial Sequence
  smMIP
  misc_feature (23)..(30): n is a, c, g, or t
gctgtcagccagaacgctgcctnnnnnnnncttcagcttcccgatatccgacggtagtgtacctcacaggagcccacttcct

SEQ ID NO: 194 - DNA, 83 bp, Artificial Sequence
  smMIP
  misc_feature (30)..(37): n is a, c, g, or t
gcagcgcagatggctccccagccctgaaannnnnnnncttcagcttcccgatatccgacggtagtgtcagcaccatcaaacag

SEQ ID NO: 195 - DNA, 83 bp, Artificial Sequence
  smMIP
  misc_feature (27)..(34): n is a, c, g, or t
gctgtttgtggatggccaggaaattgnnnnnnnncttcagcttcccgatatccgacggtagtgtgagaaggaaagaaacatat

SEQ ID NO: 196 - DNA, 83 bp, Artificial Sequence
  smMIP
  misc_feature (30)..(37): n is a, c, g, or t
gatgtgggtgaagaaggggaccaggccatnnnnnnnncttcagcttcccgatatccgacggtagtgttggctgggactaagaa

SEQ ID NO: 197 - DNA, 81 bp, Artificial Sequence
  smMIP
  misc_feature (28)..(35): n is a, c, g, or t
gcaggaaaagacactcgtgatgaacaannnnnnnncttcagcttcccgatatccgacggtagtgtcctcctacatcctcat

SEQ ID NO: 198 - DNA, 83 bp, Artificial Sequence
  smMIP
  misc_feature (30)..(37): n is a, c, g, or t
gttttttatgagcttgctcatcagttgccnnnnnnnncttcagcttcccgatatccgacggtagtgtgcggggaccgattcac

SEQ ID NO: 199 - DNA, 83 bp, Artificial Sequence
  smMIP
  misc_feature (27)..(34): n is a, c, g, or t
gcttggtgctgatttgtgaacccattnnnnnnnncttcagcttcccgatatccgacggtagtgtccgaggaagaactatgaac

SEQ ID NO: 200 - DNA, 83 bp, Artificial Sequence
  smMIP
  misc_feature (27)..(34): n is a, c, g, or t
gatgctttaactttgctggccccagcnnnnnnnncttcagcttcccgatatccgacggtagtgtcccttcaacaaacagaatg

SEQ ID NO: 201 - DNA, 83 bp, Artificial Sequence
  smMIP
  misc_feature (30)..(37): n is a, c, g, or t
caccattagaaagcagttccgcaagccctnnnnnnnncttcagcttcccgatatccgacggtagtgttgctgaagacacagaa

SEQ ID NO: 202 - DNA, 83 bp, Artificial Sequence
  smMIP
  misc_feature (30)..(37): n is a, c, g, or t
gcagctactacatcactttcttggaaacgnnnnnnnncttcagcttcccgatatccgacggtagtgtaagaactaaatccaaa

SEQ ID NO: 203 - DNA, 83 bp, Artificial Sequence
  smMIP
  misc_feature (30)..(37): n is a, c, g, or t
gcctccatcatgcgactggcaatcagcttnnnnnnnncttcagcttcccgatatccgacggtagtgtagaggaggaaggagaa

SEQ ID NO: 204 - DNA, 83 bp, Artificial Sequence
  smMIP
  misc_feature (21)..(28): n is a, c, g, or t
cacggtcaccaacagaggccnnnnnnnncttcagcttcccgatatccgacggtagtgtatctttgacttcactcatccctgcg

SEQ ID NO: 205 - DNA, 80 bp, Artificial Sequence
  smMIP
  misc_feature (23)..(30): n is a, c, g, or t
ggaccagactgaatccctgttcnnnnnnnncttcagcttcccgatatccgacggtagtgttgggggctacgtgtggctgg

SEQ ID NO: 206 - DNA, 81 bp, Artificial Sequence
  smMIP
  misc_feature (28)..(35): n is a, c, g, or t
gtctgcaaagggttttggggctcgaggnnnnnnnncttcagcttcccgatatccgacggtagtgtcagatccaccattaca

SEQ ID NO: 207 - DNA, 82 bp, Artificial Sequence
  smMIP
  misc_feature (23)..(30): n is a, c, g, or t
ttccccccacagtgctacgccannnnnnnncttcagcttcccgatatccgacggtagtgtctgagcgcaaatgtacccaatg

SEQ ID NO: 208 - DNA, 83 bp, Artificial Sequence
  smMIP
  misc_feature (28)..(35): n is a, c, g, or t
tggcctctcccgggattttaatccaacnnnnnnnncttcagcttcccgatatccgacggtagtgtcctattacttcacggagc

SEQ ID NO: 209 - DNA, 83 bp, Artificial Sequence
  smMIP
  misc_feature (27)..(34): n is a, c, g, or t
gcacattgatctggtggaaggagacgnnnnnnnncttcagcttcccgatatccgacggtagtgtaacatcgtagctgtggtga

SEQ ID NO: 210 - DNA, 83 bp, Artificial Sequence
  smMIP
  misc_feature (28)..(35): n is a, c, g, or t
gcgcttcctcctctcggagagtggcagnnnnnnnncttcagcttcccgatatccgacggtagtgtataacaagggcacaccca

SEQ ID NO: 211 - DNA, 83 bp, Artificial Sequence
  smMIP
  misc_feature (26)..(33): n is a, c, g, or t
gcgggaatcttgatcacgtggacaannnnnnnncttcagcttcccgatatccgacggtagtgtggggaagagctgtttgatca

SEQ ID NO: 212 - DNA, 83 bp, Artificial Sequence
  smMIP
  misc_feature (27)..(34): n is a, c, g, or t
gctatcctccagcagctaggtctgaannnnnnnncttcagcttcccgatatccgacggtagtgtacttcaccaagaagggatt

SEQ ID NO: 213 - DNA, 83 bp, Artificial Sequence
  smMIP
  misc_feature (23)..(30): n is a, c, g, or t
ctaccacatgcgcctctctgatnnnnnnnncttcagcttcccgatatccgacggtagtgttctcgcgtctccgcctcggtttc

SEQ ID NO: 214 - DNA, 82 bp, Artificial Sequence
  smMIP
  misc_feature (29)..(36): n is a, c, g, or t
gttgggaccatgatgacctgtggttatgnnnnnnnncttcagcttcccgatatccgacggtagtgttcatggaccaagggat

SEQ ID NO: 215 - DNA, 83 bp, Artificial Sequence
  smMIP
  misc_feature (30)..(37): n is a, c, g, or t
gctggtccgtgttcggaatgggaagtgggnnnnnnnncttcagcttcccgatatccgacggtagtgtaaggagactcatgcca

SEQ ID NO: 216 - DNA, 83 bp, Artificial Sequence
  smMIP
  misc_feature (28)..(35): n is a, c, g, or t
gtctcagattgagagtgactgcctggcnnnnnnnncttcagcttcccgatatccgacggtagtgtgtggaatgtacctgggtg

SEQ ID NO: 217 - DNA, 83 bp, Artificial Sequence
  smMIP
  misc_feature (23)..(30): n is a, c, g, or t
gcggcgctcatcactgctgtggnnnnnnnncttcagcttcccgatatccgacggtagtgtgtgggtgtggatgggaccctcta

SEQ ID NO: 218 - DNA, 79 bp, Artificial Sequence
  smMIP
  misc_feature (19)..(26): n is a, c, g, or t
cgtctgtgcggccgtgtgnnnnnnnncttcagcttcccgatatccgacggtagtgttgagccaaggcagcatcctcctg

SEQ ID NO: 219 - DNA, 82 bp, Artificial Sequence
  smMIP
  misc_feature (24)..(31): n is a, c, g, or t
ctctttcccttgtcaccagacggnnnnnnnncttcagcttcccgatatccgacggtagtgttttgtgatcccccaagaggtg

SEQ ID NO: 220 - DNA, 80 bp, Artificial Sequence
  smMIP
  misc_feature (25)..(32): n is a, c, g, or t
cggaggcctgtacctgggtgagctnnnnnnnncttcagcttcccgatatccgacggtagtgttctgcgtcagcgtcgagt

SEQ ID NO: 221 - DNA, 82 bp, Artificial Sequence
  smMIP
  misc_feature (23)..(30): n is a, c, g, or t
ggcctcattgtcggaaccggcannnnnnnncttcagcttcccgatatccgacggtagtgtgatgtcgtgagtctgttgcggg

SEQ ID NO: 222 - DNA, 82 bp, Artificial Sequence
  smMIP
  misc_feature (29)..(36): n is a, c, g, or t
gagatcgaaagtgacagcctggccctgcnnnnnnnncttcagcttcccgatatccgacggtagtgtatgtacctgggggaga

SEQ ID NO: 223 - DNA, 80 bp, Artificial Sequence
  smMIP
  misc_feature (24)..(31): n is a, c, g, or t
gcccagagcaagagaggcatcctnnnnnnnncttcagcttcccgatatccgacggtagtgtgcatgtgcaaggccggctt

SEQ ID NO: 224 - DNA, 83 bp, Artificial Sequence
  smMIP
  misc_feature (30)..(37): n is a, c, g, or t
gaagatgacccagatcatgtttgagacctnnnnnnnncttcagcttcccgatatccgacggtagtgtaccaactgggacgaca

SEQ ID NO: 225 - DNA, 83 bp, Artificial Sequence
  smMIP
  misc_feature (29)..(36): n is a, c, g, or t
gctacgtcgccctggacttcgagcaagannnnnnnncttcagcttcccgatatccgacggtagtgttgcgtctggacctggct

SEQ ID NO: 226 - DNA, 83 bp, Artificial Sequence
  smMIP
  misc_feature (29)..(36): n is a, c, g, or t
accaccatgtaccctggcattgccgacannnnnnnncttcagcttcccgatatccgacggtagtgtttccagccttccttcct

SEQ ID NO: 227 - DNA, 82 bp, Artificial Sequence
  smMIP
  misc_feature (28)..(35): n is a, c, g, or t
gtggatcagcaagcaggagtatgacgannnnnnnncttcagcttcccgatatccgacggtagtgtagaaggagatcactgcc

SEQ ID NO: 228 - DNA, 83 bp, Artificial Sequence
  smMIP
  misc_feature (26)..(33): n is a, c, g, or t
gctcaggtccttttggccagatcttnnnnnnnncttcagcttcccgatatccgacggtagtgtgaggcgagcaaaaaaattaa

SEQ ID NO: 229 - DNA, 83 bp, Artificial Sequence
  smMIP
  misc_feature (25)..(32): n is a, c, g, or t
gccttcacccaaagtgtctgacacnnnnnnnncttcagcttcccgatatccgacggtagtgtactgcctgcagggcttccagc

SEQ ID NO: 230 - DNA, 83 bp, Artificial Sequence
  smMIP
  misc_feature (30)..(37): n is a, c, g, or t
gtccccttcccacgtctccatttctttatnnnnnnnncttcagcttcccgatatccgacggtagtgttgaccacaccaaccta

SEQ ID NO: 231 - DNA, 83 bp, Artificial Sequence
  smMIP
  misc_feature (30)..(37): n is a, c, g, or t
gtggtcggatgtccatgaaggaggtcgatnnnnnnnncttcagcttcccgatatccgacggtagtgtaagccagcagtatcga

SEQ ID NO: 232 - DNA, 83 bp, Artificial Sequence
  smMIP
  misc_feature (26)..(33): n is a, c, g, or t
gccgaagaggaggcctaaggcagagnnnnnnnncttcagcttcccgatatccgacggtagtgttacacaggcgagggcatgga

SEQ ID NO: 233 - DNA, 83 bp, Artificial Sequence
  smMIP
  misc_feature (29)..(36): n is a, c, g, or t
gccattcaaggacctggaggaaagtggannnnnnnncttcagcttcccgatatccgacggtagtgtggtggtgttcagacagt

SEQ ID NO: 234 - DNA, 80 bp, Artificial Sequence
  smMIP
  misc_feature (26)..(33): n is a, c, g, or t
tagcagccggtcacccatctatgaannnnnnnncttcagcttcccgatatccgacggtagtgtttcagtgggaggagcgg

SEQ ID NO: 235 - DNA, 83 bp, Artificial Sequence
  smMIP
  misc_feature (27)..(34): n is a, c, g, or t
ccccttacaccgatgtaaatattgtgnnnnnnnncttcagcttcccgatatccgacggtagtgtgggcttgaaaggccctttg

SEQ ID NO: 236 - DNA, 47 bp, Artificial Sequence
  smMIP
cttcagcttcccgatatccgacggtagtgttgtccgaccatgtgtct

SEQ ID NO: 237 - DNA, 80 bp, Artificial Sequence
  smMIP
  misc_feature (26)..(33): n is a, c, g, or t
cggagcaacgtcacggcggtgcacannnnnnnncttcagcttcccgatatccgacggtagtgtgaaggagaatacagtgg

SEQ ID NO: 238 - DNA, 78 bp, Artificial Sequence
  smMIP
  misc_feature (24)..(31): n is a, c, g, or t
gagatgtaccttgatacagtatgnnnnnnnncttcagcttcccgatatccgacggtagtgtatgcccggaacaaccac

SEQ ID NO: 239 - DNA, 83 bp, Artificial Sequence
  smMIP
  misc_feature (28)..(35): n is a, c, g, or t
gtgacttgtgtgcaggattgatcggagnnnnnnnncttcagcttcccgatatccgacggtagtgtgcagaaagctgtaaagat

SEQ ID NO: 240 - DNA, 83 bp, Artificial Sequence
  smMIP
  misc_feature (22)..(29): n is a, c, g, or t
gtcggttcatgggacggctccnnnnnnnncttcagcttcccgatatccgacggtagtgtcccaatttgatgttcttgttatgc

SEQ ID NO: 241 - DNA, 83 bp, Artificial Sequence
  smMIP
  misc_feature (30)..(37): n is a, c, g, or t
gatgctgcgccacatgggactttttgaccnnnnnnnncttcagcttcccgatatccgacggtagtgtacaccaagtggcaaca

SEQ ID NO: 242 - DNA, 83 bp, Artificial Sequence
  smMIP
  misc_feature (27)..(34): n is a, c, g, or t
gcaaaatgctcagacttcacagaggannnnnnnncttcagcttcccgatatccgacggtagtgttcctgctcagtgccgtgat

SEQ ID NO: 243 - DNA, 81 bp, Artificial Sequence
  smMIP
  misc_feature (28)..(35): n is a, c, g, or t
tctacaactggcatttacatcagtcacnnnnnnnncttcagcttcccgatatccgacggtagtgtgaggctgcgtgttttg

SEQ ID NO: 244 - DNA, 82 bp, Artificial Sequence
  smMIP
  misc_feature (25)..(32): n is a, c, g, or t
gctgagttccatgaaggagaacaannnnnnnncttcagcttcccgatatccgacggtagtgtgtgtggggcctgagctgatg

SEQ ID NO: 245 - DNA, 83 bp, Artificial Sequence
  smMIP
  misc_feature (29)..(36): n is a, c, g, or t
gcggctgaggcgtaagttggacttatttnnnnnnnncttcagcttcccgatatccgacggtagtgtgaatatggcatctgagg

SEQ ID NO: 246 - DNA, 81 bp, Artificial Sequence
  smMIP
  misc_feature (28)..(35): n is a, c, g, or t
gtgatcattcgagagcagacagaagggnnnnnnnncttcagcttcccgatatccgacggtagtgtggagtataagggggag

SEQ ID NO: 247 - DNA, 83 bp, Artificial Sequence
  smMIP
  misc_feature (30)..(37): n is a, c, g, or t
gcggattgcaaagttcgcctttgactatgnnnnnnnncttcagcttcccgatatccgacggtagtgtcacaacaatctagacc

SEQ ID NO: 248 - DNA, 82 bp, Artificial Sequence
  smMIP
  misc_feature (25)..(32): n is a, c, g, or t
gaaacttggggatgggttgttcctnnnnnnnncttcagcttcccgatatccgacggtagtgtggggtgtgattgagtgtttg

SEQ ID NO: 249 - DNA, 83 bp, Artificial Sequence
  smMIP
  misc_feature (30)..(37): n is a, c, g, or t
gtgcagaatccttaccagtttgatgtgctnnnnnnnncttcagcttcccgatatccgacggtagtgtacaaggccaacatcat

SEQ ID NO: 250 - DNA, 83 bp, Artificial Sequence
  smMIP
  misc_feature (26)..(33): n is a, c, g, or t
gctggtgtggtccctggtgagagctnnnnnnnncttcagcttcccgatatccgacggtagtgtgagacaatgatcatagacaa

SEQ ID NO: 251 - DNA, 80 bp, Artificial Sequence
  smMIP
  misc_feature (21)..(28): n is a, c, g, or t
gccatgctgctgtcggcttcnnnnnnnncttcagcttcccgatatccgacggtagtgttggctgctggcctggttggggg

SEQ ID NO: 252 - DNA, 81 bp, Artificial Sequence
  smMIP
  misc_feature (25)..(32): n is a, c, g, or t
gcaaggtgcggactcgagacatggnnnnnnnncttcagcttcccgatatccgacggtagtgtgcagtgggcaggaatatag

SEQ ID NO: 253 - DNA, 83 bp, Artificial Sequence
  smMIP
  misc_feature (30)..(37): n is a, c, g, or t
gccctttatttcttccaaccttgcaaggannnnnnnncttcagcttcccgatatccgacggtagtgtagatgcggtgaagaag

SEQ ID NO: 254 - DNA, 82 bp, Artificial Sequence
  smMIP
  misc_feature (29)..(36): n is a, c, g, or t
gcacacggtgaccatgatcccaggggatnnnnnnnncttcagcttcccgatatccgacggtagtgtgaaggcggtgctcggg

SEQ ID NO: 255 - DNA, 83 bp, Artificial Sequence
  smMIP
  misc_feature (30)..(37): n is a, c, g, or t
gtaccagtggactttgaagaggtgcacgtnnnnnnnncttcagcttcccgatatccgacggtagtgtcagaacaaacaattcc

SEQ ID NO: 256 - DNA, 83 bp, Artificial Sequence
  smMIP
  misc_feature (24)..(31): n is a, c, g, or t
gccctgaagggcaacatcgaaacnnnnnnnncttcagcttcccgatatccgacggtagtgttgctgcatgtcaagtccgtctt

SEQ ID NO: 257 - DNA, 83 bp, Artificial Sequence
  smMIP
  misc_feature (25)..(32): n is a, c, g, or t
cgtcatccactgtaagagccttccnnnnnnnncttcagcttcccgatatccgacggtagtgtatgccatcatggccatccgcc

SEQ ID NO: 258 - DNA, 83 bp, Artificial Sequence
  smMIP
  misc_feature (26)..(33): n is a, c, g, or t
gtacagcagcctggagcatgagagtnnnnnnnncttcagcttcccgatatccgacggtagtgtaaacaacatccttcgcacca

SEQ ID NO: 259 - DNA, 83 bp, Artificial Sequence
  smMIP
  misc_feature (30)..(37): n is a, c, g, or t
gcattgccgagtatgccttcaagctggcgnnnnnnnncttcagcttcccgatatccgacggtagtgtcaaggacatagacatc

SEQ ID NO: 260 - DNA, 83 bp, Artificial Sequence
  smMIP
  misc_feature (30)..(37): n is a, c, g, or t
gcttttcctccagtgctgcagggaggtggnnnnnnnncttcagcttcccgatatccgacggtagtgtaagatcatcaccaagg

SEQ ID NO: 261 - DNA, 83 bp, Artificial Sequence
  smMIP
  misc_feature (30)..(37): n is a, c, g, or t
cggccccagcagtttgatgtcatggtgatnnnnnnnncttcagcttcccgatatccgacggtagtgtccaacatcatgaaact

SEQ ID NO: 262 - DNA, 83 bp, Artificial Sequence
  smMIP
  misc_feature (30)..(37): n is a, c, g, or t
gtggctggggccaactatggccatgtgtannnnnnnncttcagcttcccgatatccgacggtagtgttggataacaccaccat

SEQ ID NO: 263 - DNA, 83 bp, Artificial Sequence
  smMIP
  misc_feature (20)..(27): n is a, c, g, or t
ccaaccccacggccaccctnnnnnnnncttcagcttcccgatatccgacggtagtgttcgtcaacaatgtctgcgcgggactg

SEQ ID NO: 264 - DNA, 83 bp, Artificial Sequence
  smMIP
  misc_feature (28)..(35): n is a, c, g, or t
gctgtcctggcatccatggacaatgagnnnnnnnncttcagcttcccgatatccgacggtagtgttacgaggaacaccggcaa

SEQ ID NO: 265 - DNA, 82 bp, Artificial Sequence
  smMIP
  misc_feature (19)..(26): n is a, c, g, or t
cactgaccacagcccccannnnnnnncttcagcttcccgatatccgacggtagtgttgcactcctatgccacctccatccgt

SEQ ID NO: 266 - DNA, 79 bp, Artificial Sequence
  smMIP
  misc_feature (19)..(26): n is a, c, g, or t
gtcatcgttggtggcggannnnnnnncttcagcttcccgatatccgacggtagtgttttggttggtgcctgcggacggg

SEQ ID NO: 267 - DNA, 83 bp, Artificial Sequence
  smMIP
  misc_feature (30)..(37): n is a, c, g, or t
gttctggaaaaggagaaagatttagctgtnnnnnnnncttcagcttcccgatatccgacggtagtgttgtgtggaggtagccg

SEQ ID NO: 268 - DNA, 83 bp, Artificial Sequence
  smMIP
  misc_feature (26)..(33): n is a, c, g, or t
tgtgtacaaggtgcagccctcctctnnnnnnnncttcagcttcccgatatccgacggtagtgtcatccatcactttctattgg

SEQ ID NO: 269 - DNA, 83 bp, Artificial Sequence
  smMIP
  misc_feature (19)..(26): n is a, c, g, or t
ttcccagacttcaggcccnnnnnnnncttcagcttcccgatatccgacggtagtgttattataaacctgagtctctgaaagcc

SEQ ID NO: 270 - DNA, 83 bp, Artificial Sequence
  smMIP
  misc_feature (30)..(37): n is a, c, g, or t
gccatattgtaggggtctaatggctattgnnnnnnnncttcagcttcccgatatccgacggtagtgtaagcttatagtagctg

SEQ ID NO: 271 - DNA, 78 bp, Artificial Sequence
  smMIP
  misc_feature (19)..(26): n is a, c, g, or t
gcaggtggctctgtcttgnnnnnnnncttcagcttcccgatatccgacggtagtgtgaggctgatccagcaggaggat

SEQ ID NO: 272 - DNA, 83 bp, Artificial Sequence
  smMIP
  misc_feature (30)..(37): n is a, c, g, or t
gaatacaaagggagaggaaattcgatgtcnnnnnnnncttcagcttcccgatatccgacggtagtgtgcccaggatttccaag

SEQ ID NO: 273 - DNA, 83 bp, Artificial Sequence
  smMIP
  misc_feature (26)..(33): n is a, c, g, or t
ggctgcactcctgatcctcgaattgnnnnnnnncttcagcttcccgatatccgacggtagtgtccttcaagaagtatagatgg

SEQ ID NO: 274 - DNA, 83 bp, Artificial Sequence
  smMIP
  misc_feature (25)..(32): n is a, c, g, or t
gccggtttcctttcctaggagttcnnnnnnnncttcagcttcccgatatccgacggtagtgtgaccgtatttcagagttgagt

SEQ ID NO: 275 - DNA, 83 bp, Artificial Sequence
  smMIP
  misc_feature (26)..(33): n is a, c, g, or t
ccctttgacttcagtgccacagatgnnnnnnnncttcagcttcccgatatccgacggtagtgtggaaatatttatccggtccc

SEQ ID NO: 276 - DNA, 83 bp, Artificial Sequence
  smMIP
  misc_feature (29)..(36): n is a, c, g, or t
gcatgttttcttggtgcaacagtgaagtnnnnnnnncttcagcttcccgatatccgacggtagtgtaaacgagagggttacag

SEQ ID NO: 277 - DNA, 83 bp, Artificial Sequence
  smMIP
  misc_feature (24)..(31): n is a, c, g, or t
gcccagctggagtaagagcccagnnnnnnnncttcagcttcccgatatccgacggtagtgtgattaaactggcatcccagaat

SEQ ID NO: 278 - DNA, 83 bp, Artificial Sequence
  smMIP
  misc_feature (29)..(36): n is a, c, g, or t
ggggatattggaaatcgcattcttcatgnnnnnnnncttcagcttcccgatatccgacggtagtgtcttcaaaaattcatccc

SEQ ID NO: 279 - DNA, 82 bp, Artificial Sequence
  smMIP
  misc_feature (26)..(33): n is a, c, g, or t
gcagatgaagtacaacaaagatttgnnnnnnnncttcagcttcccgatatccgacggtagtgtgatggaaatctggtagaag

SEQ ID NO: 280 - DNA, 83 bp, Artificial Sequence
  smMIP
  misc_feature (30)..(37): n is a, c, g, or t
gcaacaagaatgtactaattgcattctttnnnnnnnncttcagcttcccgatatccgacggtagtgtgcaccttctcctgctg

SEQ ID NO: 281 - DNA, 83 bp, Artificial Sequence
  smMIP
  misc_feature (25)..(32): n is a, c, g, or t
gcatggcctgtgccatcagtatctnnnnnnnncttcagcttcccgatatccgacggtagtgtgcattcccgattccttttggt

SEQ ID NO: 282 - DNA, 83 bp, Artificial Sequence
  smMIP
  misc_feature (27)..(34): n is a, c, g, or t
gttattggaagcggttgcaatctggannnnnnnncttcagcttcccgatatccgacggtagtgttgaagggagagatgatgga

SEQ ID NO: 283 - DNA, 83 bp, Artificial Sequence
  smMIP
  misc_feature (28)..(35): n is a, c, g, or t
gcacccagatttagggactgataaagannnnnnnncttcagcttcccgatatccgacggtagtgttaatgggggaaaggctgg

SEQ ID NO: 284 - DNA, 83 bp, Artificial Sequence
  smMIP
  misc_feature (28)..(35): n is a, c, g, or t
ggatgatgtcttccttagtgttccttgnnnnnnnncttcagcttcccgatatccgacggtagtgtaactcaaaggctacacat

SEQ ID NO: 285 - DNA, 83 bp, Artificial Sequence
  smMIP
  misc_feature (29)..(36): n is a, c, g, or t
gcatgttgtcctttttatctgatctgtgnnnnnnnncttcagcttcccgatatccgacggtagtgtggcccgtttgaagaaga

SEQ ID NO: 286 - DNA, 82 bp, Artificial Sequence
  smMIP
  misc_feature (29)..(36): n is a, c, g, or t
gttggtatggcgtgtgctatcagcattcnnnnnnnncttcagcttcccgatatccgacggtagtgtaaaaccaggccctact

SEQ ID NO: 287 - DNA, 83 bp, Artificial Sequence
  smMIP
  misc_feature (27)..(34): n is a, c, g, or t
gcaagaaggggagagtcggctcaatcnnnnnnnncttcagcttcccgatatccgacggtagtgtaaaggagaaatgatggatc

SEQ ID NO: 288 - DNA, 81 bp, Artificial Sequence
  smMIP
  misc_feature (24)..(31): n is a, c, g, or t
gtgtggctgtgtggagtggtgtgnnnnnnnncttcagcttcccgatatccgacggtagtgtcaaacaccgcgtgattggaa

SEQ ID NO: 289 - DNA, 83 bp, Artificial Sequence
  smMIP
  misc_feature (30)..(37): n is a, c, g, or t
gtgtggctgatcttattgaatccatgttgnnnnnnnncttcagcttcccgatatccgacggtagtgtgaatccagaaatggga

SEQ ID NO: 290 - DNA, 83 bp, Artificial Sequence
  smMIP
  misc_feature (30)..(37): n is a, c, g, or t
gctcaagaaaagtgcagataccctgtgggnnnnnnnncttcagcttcccgatatccgacggtagtgtacaatggtaaagggga

SEQ ID NO: 291 - DNA, 83 bp, Artificial Sequence
  smMIP
  misc_feature (30)..(37): n is a, c, g, or t
cctataggctcaggagctcaaggaatagtnnnnnnnncttcagcttcccgatatccgacggtagtgtggatgaagccattaaa

SEQ ID NO: 292 - DNA, 83 bp, Artificial Sequence
  smMIP
  misc_feature (28)..(35): n is a, c, g, or t
gcaaatctttgccaagtgattcagatgnnnnnnnncttcagcttcccgatatccgacggtagtgtcagagagctagttcttat

SEQ ID NO: 293 - DNA, 83 bp, Artificial Sequence
  smMIP
  misc_feature (25)..(32): n is a, c, g, or t
cgttgacatttggtcagttgggtgnnnnnnnncttcagcttcccgatatccgacggtagtgtgcactttgaagattcttgact

SEQ ID NO: 294 - DNA, 83 bp, Artificial Sequence
  smMIP
  misc_feature (30)..(37): n is a, c, g, or t
gctggtaatagatgcatctaaaaggatctnnnnnnnncttcagcttcccgatatccgacggtagtgtgaaaacagacctaaat

SEQ ID NO: 295 - DNA, 83 bp, Artificial Sequence
  smMIP
  misc_feature (30)..(37): n is a, c, g, or t
gctctcagcatccatcatcatcgtcgtctnnnnnnnncttcagcttcccgatatccgacggtagtgtggaacacacaatagaa

SEQ ID NO: 296 - DNA, 83 bp, Artificial Sequence
  smMIP
  misc_feature (24)..(31): n is a, c, g, or t
cgactcggtgcagccgtatttctnnnnnnnncttcagcttcccgatatccgacggtagtgtcttctctgaaaggctctccttg

SEQ ID NO: 297 - DNA, 79 bp, Artificial Sequence
  smMIP
  misc_feature (21)..(28): n is a, c, g, or t
ttcgagctgctgcccaccccnnnnnnnncttcagcttcccgatatccgacggtagtgtacaggaactatgacctcgact

SEQ ID NO: 298 - DNA, 82 bp, Artificial Sequence
  smMIP
  misc_feature (24)..(31): n is a, c, g, or t
tctgtggaaaagaggcaggctccnnnnnnnncttcagcttcccgatatccgacggtagtgttgctctcctcgacggagtcct

SEQ ID NO: 299 - DNA, 80 bp, Artificial Sequence
  smMIP
  misc_feature (26)..(33): n is a, c, g, or t
ctggtcctcaagaggtgccacgtctnnnnnnnncttcagcttcccgatatccgacggtagtgtgaggaggaacaagaaga

SEQ ID NO: 300 - DNA, 83 bp, Artificial Sequence
  smMIP
  misc_feature (28)..(35): n is a, c, g, or t
cagtgtcagagtcctgagacagatcagnnnnnnnncttcagcttcccgatatccgacggtagtgtacagcaaacctcctcaca

SEQ ID NO: 301 - DNA, 83 bp, Artificial Sequence
  smMIP
  misc_feature (30)..(37): n is a, c, g, or t
gcgccagaggaggaacgagctaaaacggannnnnnnncttcagcttcccgatatccgacggtagtgtaagagggtcaagttgg

SEQ ID NO: 302 - DNA, 83 bp, Artificial Sequence
  smMIP
  misc_feature (27)..(34): n is a, c, g, or t
agccacagcatacatcctgtccgtccnnnnnnnncttcagcttcccgatatccgacggtagtgtcgaacacacaacgtcttgg

SEQ ID NO: 303 - DNA, 83 bp, Artificial Sequence
  smMIP
  misc_feature (28)..(35): n is a, c, g, or t
cttgaacagctacggaactcttgtgcgnnnnnnnncttcagcttcccgatatccgacggtagtgtggcccccaaggtagttat

SEQ ID NO: 304 - DNA, 83 bp, Artificial Sequence
  smMIP
  misc_feature (30)..(37): n is a, c, g, or t
ccttctaacagaaatgtcctgagcaatcannnnnnnncttcagcttcccgatatccgacggtagtgtaagcagaggagcaaaa

SEQ ID NO: 305 - DNA, 83 bp, Artificial Sequence
  smMIP
  misc_feature (29)..(36): n is a, c, g, or t
ctttgaatgccgtgaaaagaagacagaannnnnnnncttcagcttcccgatatccgacggtagtgttgtcctccggcccgaga

SEQ ID NO: 306 - DNA, 83 bp, Artificial Sequence
  smMIP
  misc_feature (30)..(37): n is a, c, g, or t
ggaaatgttctcttcacggtggaaaacacnnnnnnnncttcagcttcccgatatccgacggtagtgtacaaagaacatttcca

SEQ ID NO: 307 - DNA, 83 bp, Artificial Sequence
  smMIP
  misc_feature (23)..(30): n is a, c, g, or t
gtagcaggacttgctctaattannnnnnnncttcagcttcccgatatccgacggtagtgtgaaacttctggtaacttagatgg

SEQ ID NO: 308 - DNA, 83 bp, Artificial Sequence
  smMIP
  misc_feature (30)..(37): n is a, c, g, or t
gccaccttatcttagagttattcaaggggnnnnnnnncttcagcttcccgatatccgacggtagtgtacacaggcaccactaa

SEQ ID NO: 309 - DNA, 83 bp, Artificial Sequence
  smMIP
  misc_feature (28)..(35): n is a, c, g, or t
cgccagcagggaattttgttacactggnnnnnnnncttcagcttcccgatatccgacggtagtgtctcttgaattgttccttc

SEQ ID NO: 310 - DNA, 82 bp, Artificial Sequence
  smMIP
  misc_feature (19)..(26): n is a, c, g, or t
gcccaggtggagccactannnnnnnncttcagcttcccgatatccgacggtagtgttttccggctcctgggctctgacgggt

SEQ ID NO: 311 - DNA, 81 bp, Artificial Sequence
  smMIP
  misc_feature (24)..(31): n is a, c, g, or t
gttccaggtgccctggctggagtnnnnnnnncttcagcttcccgatatccgacggtagtgtaacttcctagcagtcgccct

SEQ ID NO: 312 - DNA, 82 bp, Artificial Sequence
  smMIP
  misc_feature (29)..(36): n is a, c, g, or t
gtcattggcattggcaccagtgtggtcannnnnnnncttcagcttcccgatatccgacggtagtgtgtcttccgagctgctg

SEQ ID NO: 313 - DNA, 83 bp, Artificial Sequence
  smMIP
  misc_feature (30)..(37): n is a, c, g, or t
cgaggaccccgagaagcagacgttgcctgnnnnnnnncttcagcttcccgatatccgacggtagtgtgagggcagtgaggtga

SEQ ID NO: 314 - DNA, 83 bp, Artificial Sequence
  smMIP
  misc_feature (26)..(33): n is a, c, g, or t
gccttcctgaaatatgagaaggccgnnnnnnnncttcagcttcccgatatccgacggtagtgttcttccctgttgcctagaag

SEQ ID NO: 315 - DNA, 83 bp, Artificial Sequence
  smMIP
  misc_feature (21)..(28): n is a, c, g, or t
cccatccagtcccgaaacacnnnnnnnncttcagcttcccgatatccgacggtagtgtctattcacatcattgcacacctgtt

SEQ ID NO: 316 - DNA, 83 bp, Artificial Sequence
  smMIP
  misc_feature (26)..(33): n is a, c, g, or t
gcaccggtcattctttatatctgtgnnnnnnnncttcagcttcccgatatccgacggtagtgtgagagcatgaatgagagtca

SEQ ID NO: 317 - DNA, 83 bp, Artificial Sequence
  smMIP
  misc_feature (25)..(32): n is a, c, g, or t
gctggttggagcaggaattggggtnnnnnnnncttcagcttcccgatatccgacggtagtgtcagcaggggactggacagaaa

SEQ ID NO: 318 - DNA, 83 bp, Artificial Sequence
  smMIP
  misc_feature (30)..(37): n is a, c, g, or t
gtctgtagtgggagttttcttatgtggccnnnnnnnncttcagcttcccgatatccgacggtagtgtggtcatgcagcattaa

SEQ ID NO: 319 - DNA, 83 bp, Artificial Sequence
  smMIP
  misc_feature (27)..(34): n is a, c, g, or t
cgagttattttgggttcaacactggcnnnnnnnncttcagcttcccgatatccgacggtagtgttggggtgctggattttgaa

SEQ ID NO: 320 - DNA, 83 bp, Artificial Sequence
  smMIP
  misc_feature (19)..(26): n is a, c, g, or t
ccccacaaacacaaccacnnnnnnnncttcagcttcccgatatccgacggtagtgtacatcgtggcgcatttcttcaacctgg

SEQ ID NO: 321 - DNA, 83 bp, Artificial Sequence
  smMIP
  misc_feature (30)..(37): n is a, c, g, or t
gcgatttcaacaagaagttgtcattaccannnnnnnncttcagcttcccgatatccgacggtagtgtgcagaatggcagacag

SEQ ID NO: 322 - DNA, 82 bp, Artificial Sequence
  smMIP
  misc_feature (28)..(35): n is a, c, g, or t
gcgttgccgcggggatcggagtcactcnnnnnnnncttcagcttcccgatatccgacggtagtgtctactggaggcctttgg

SEQ ID NO: 323 - DNA, 83 bp, Artificial Sequence
  smMIP
  misc_feature (27)..(34): n is a, c, g, or t
caagcagattgcctacaatcaccccannnnnnnncttcagcttcccgatatccgacggtagtgttttcttaccggctgggatg

SEQ ID NO: 324 - DNA, 83 bp, Artificial Sequence
  smMIP
  misc_feature (25)..(32): n is a, c, g, or t
gtcctgcttttctggaaaaccttcnnnnnnnncttcagcttcccgatatccgacggtagtgttccttctcggtccggcgggca

SEQ ID NO: 325 - DNA, 83 bp, Artificial Sequence
  smMIP
  misc_feature (25)..(32): n is a, c, g, or t
acttctcttcacaactgttcctggnnnnnnnncttcagcttcccgatatccgacggtagtgtctatctgtattttctcaggcg

SEQ ID NO: 326 - DNA, 83 bp, Artificial Sequence
  smMIP
  misc_feature (27)..(34): n is a, c, g, or t
gcccagattccaagctaattttccacnnnnnnnncttcagcttcccgatatccgacggtagtgtaccagctctcagaatattt

SEQ ID NO: 327 - DNA, 83 bp, Artificial Sequence
  smMIP
  misc_feature (24)..(31): n is a, c, g, or t
gaaattctgcccttcattcaatcnnnnnnnncttcagcttcccgatatccgacggtagtgtatcatccatttaccctcacaat

SEQ ID NO: 328 - DNA, 83 bp, Artificial Sequence
  smMIP
  misc_feature (30)..(37): n is a, c, g, or t
cggtggaaacttttgtttgatgaaatagcnnnnnnnncttcagcttcccgatatccgacggtagtgtggcaagagaacagacc

SEQ ID NO: 329 - DNA, 83 bp, Artificial Sequence
  smMIP
  misc_feature (27)..(34): n is a, c, g, or t
gcggctttgaagaagaaaggatgggannnnnnnncttcagcttcccgatatccgacggtagtgtaaccacgagcccagccaat

SEQ ID NO: 330 - DNA, 83 bp, Artificial Sequence
  smMIP
  misc_feature (29)..(36): n is a, c, g, or t
gctggaagccgcagaccttgtgatattcnnnnnnnncttcagcttcccgatatccgacggtagtgtcatttccagaaaggaca

SEQ ID NO: 331 - DNA, 83 bp, Artificial Sequence
  smMIP
  misc_feature (29)..(36): n is a, c, g, or t
catcaccactggtggcagtggctccatgnnnnnnnncttcagcttcccgatatccgacggtagtgtgtggtttggagtccctg

SEQ ID NO: 332 - DNA, 83 bp, Artificial Sequence
  smMIP
  misc_feature (30)..(37): n is a, c, g, or t
gcccgaattcaaatcctggaaggatggaannnnnnnncttcagcttcccgatatccgacggtagtgtaagggatccacgggga

SEQ ID NO: 333 - DNA, 83 bp, Artificial Sequence
  smMIP
  misc_feature (24)..(31): n is a, c, g, or t
caagtccatcccaactgacaaccnnnnnnnncttcagcttcccgatatccgacggtagtgtacaccactgtattttgctccaa

SEQ ID NO: 334 - DNA, 83 bp, Artificial Sequence
  smMIP
  misc_feature (27)..(34): n is a, c, g, or t
gattcggtgctattctgcacctgttgnnnnnnnncttcagcttcccgatatccgacggtagtgtaaaaacttcaggacaaaaa

SEQ ID NO: 335 - DNA, 83 bp, Artificial Sequence
  smMIP
  misc_feature (29)..(36): n is a, c, g, or t
gctggaaaaccccaaaagtgtacataagnnnnnnnncttcagcttcccgatatccgacggtagtgtacaaaacagaccagcag

SEQ ID NO: 336 - DNA, 83 bp, Artificial Sequence
  smMIP
  misc_feature (22)..(29): n is a, c, g, or t
ctgcctaccagagtccccttcnnnnnnnncttcagcttcccgatatccgacggtagtgtccctttctcagtgggactagttcg

SEQ ID NO: 337 - DNA, 83 bp, Artificial Sequence
  smMIP
  misc_feature (30)..(37): n is a, c, g, or t
gctgatctggactcctccgtgcccgctgannnnnnnncttcagcttcccgatatccgacggtagtgttagaagcacagcccaa

SEQ ID NO: 338 - DNA, 83 bp, Artificial Sequence
  smMIP
  misc_feature (21)..(28): n is a, c, g, or t
ttccacttgcccaccaccacnnnnnnnncttcagcttcccgatatccgacggtagtgtaccatgtagcacagctggaccccct

SEQ ID NO: 339 - DNA, 83 bp, Artificial Sequence
  smMIP
  misc_feature (28)..(35): n is a, c, g, or t
gcatattggggtggagttcatgttcatnnnnnnnncttcagcttcccgatatccgacggtagtgtatggcctggatgagtctg

SEQ ID NO: 340 - DNA, 81 bp, Artificial Sequence
  smMIP
  misc_feature (28)..(35): n is a, c, g, or t
gcagttcacaaatgaggagaaacggacnnnnnnnncttcagcttcccgatatccgacggtagtgttgcgggagatcatccg

SEQ ID NO: 341 - DNA, 83 bp, Artificial Sequence
  smMIP
  misc_feature (29)..(36): n is a, c, g, or t
gctttggtctagaaggctgcgaggtactnnnnnnnncttcagcttcccgatatccgacggtagtgtagaagtttgagacccct

SEQ ID NO: 342 - DNA, 83 bp, Artificial Sequence
  smMIP
  misc_feature (27)..(34): n is a, c, g, or t
gagggcggctgaacgtgcttgcaaatnnnnnnnncttcagcttcccgatatccgacggtagtgtgaagtggtcctctgagaag

SEQ ID NO: 343 - DNA, 82 bp, Artificial Sequence
  smMIP
  misc_feature (29)..(36): n is a, c, g, or t
gctgatgagggctccggagatgtgaagtnnnnnnnncttcagcttcccgatatccgacggtagtgtgagaatggcgtggact

SEQ ID NO: 344 - DNA, 83 bp, Artificial Sequence
  smMIP
  misc_feature (25)..(32): n is a, c, g, or t
cttgtccttggtggccaacccttcnnnnnnnncttcagcttcccgatatccgacggtagtgtagctggaacagatcttctgtc

SEQ ID NO: 345 - DNA, 83 bp, Artificial Sequence
  smMIP
  misc_feature (29)..(36): n is a, c, g, or t
gcgacactgaagggaaaaaggtaaggccnnnnnnnncttcagcttcccgatatccgacggtagtgtaccgcaggatcaatcgt

SEQ ID NO: 346 - DNA, 83 bp, Artificial Sequence
  smMIP
  misc_feature (29)..(36): n is a, c, g, or t
ggagttccgctcaccaacataacccagannnnnnnncttcagcttcccgatatccgacggtagtgttgaccccgtggtgatgg

SEQ ID NO: 347 - DNA, 83 bp, Artificial Sequence
  smMIP
  misc_feature (20)..(27): n is a, c, g, or t
agcatccccaaggactcgcnnnnnnnncttcagcttcccgatatccgacggtagtgttgtttctaggtcgtggcgtcgggctt

SEQ ID NO: 348 - DNA, 83 bp, Artificial Sequence
  smMIP
  misc_feature (30)..(37): n is a, c, g, or t
gagtggatgaagtggcgaagaagaaatctnnnnnnnncttcagcttcccgatatccgacggtagtgtcgagtacagtgcgagt

SEQ ID NO: 349 - DNA, 83 bp, Artificial Sequence
  smMIP
  misc_feature (30)..(37): n is a, c, g, or t
gcaagggccaggtcaaggaggaaggtatcnnnnnnnncttcagcttcccgatatccgacggtagtgtcaagagccttcaggag

SEQ ID NO: 350 - DNA, 83 bp, Artificial Sequence
  smMIP
  misc_feature (26)..(33): n is a, c, g, or t
gctggacatcgaggtggcctacagtnnnnnnnncttcagcttcccgatatccgacggtagtgtctctcagatcctggatctct

SEQ ID NO: 351 - DNA, 83 bp, Artificial Sequence
  smMIP
  misc_feature (29)..(36): n is a, c, g, or t
ccttcagctaacattagtctggatggtgnnnnnnnncttcagcttcccgatatccgacggtagtgtggcttaatcctgttggg

SEQ ID NO: 352 - DNA, 82 bp, Artificial Sequence
  smMIP
  misc_feature (29)..(36): n is a, c, g, or t
gtggatgtggcagctgattccatgtctgnnnnnnnncttcagcttcccgatatccgacggtagtgtaccatgctggtcagct

SEQ ID NO: 353 - DNA, 83 bp, Artificial Sequence
  smMIP
  misc_feature (23)..(30): n is a, c, g, or t
gcatgagggtggtgcacagctannnnnnnncttcagcttcccgatatccgacggtagtgtttgctgcgggtgttcccgttgtc

SEQ ID NO: 354 - DNA, 83 bp, Artificial Sequence
  smMIP
  misc_feature (27)..(34): n is a, c, g, or t
ccaaaagctgttgcactacctcggccnnnnnnnncttcagcttcccgatatccgacggtagtgtaagaccaacatcgccttcc

SEQ ID NO: 355 - DNA, 82 bp, Artificial Sequence
  smMIP
  misc_feature (28)..(35): n is a, c, g, or t
gcgcgtgtttgactacagtgagtactgnnnnnnnncttcagcttcccgatatccgacggtagtgtaggctggagctgatgtg

SEQ ID NO: 356 - DNA, 82 bp, Artificial Sequence
  smMIP
  misc_feature (29)..(36): n is a, c, g, or t
caaggacacccaggccatgaaggagatgnnnnnnnncttcagcttcccgatatccgacggtagtgttgaggtggagctggag

SEQ ID NO: 357 - DNA, 83 bp, Artificial Sequence
  smMIP
  misc_feature (29)..(36): n is a, c, g, or t
gaaattaagaaatgtgaccttcaccggcnnnnnnnncttcagcttcccgatatccgacggtagtgtcactgcctgtgcttcat

SEQ ID NO: 358 - DNA, 83 bp, Artificial Sequence
  smMIP
  misc_feature (27)..(34): n is a, c, g, or t
gctcacggctttactttcacccggggnnnnnnnncttcagcttcccgatatccgacggtagtgtcagatcagctgtataaaca

SEQ ID NO: 359 - DNA, 83 bp, Artificial Sequence
  smMIP
  misc_feature (30)..(37): n is a, c, g, or t
gtggaaattaccttgtattttcatctgtgnnnnnnnncttcagcttcccgatatccgacggtagtgtctgggcgctgggattg

SEQ ID NO: 360 - DNA, 83 bp, Artificial Sequence
  smMIP
  misc_feature (30)..(37): n is a, c, g, or t
gtagatctgggaaggggcccatcctgatgnnnnnnnncttcagcttcccgatatccgacggtagtgttgttgagagagcggca

SEQ ID NO: 361 - DNA, 83 bp, Artificial Sequence
  smMIP
  misc_feature (30)..(37): n is a, c, g, or t
ggaagagctgggctaccacatctactccannnnnnnncttcagcttcccgatatccgacggtagtgtaaggacaggatggtga

SEQ ID NO: 362 - DNA, 83 bp, Artificial Sequence
  smMIP
  misc_feature (26)..(33): n is a, c, g, or t
gataatcttctcaggacaccatccgnnnnnnnncttcagcttcccgatatccgacggtagtgtctctccatgaagcagttcct

SEQ ID NO: 363 - DNA, 83 bp, Artificial Sequence
  smMIP
  misc_feature (27)..(34): n is a, c, g, or t
gcaagatgatctttacagatactgtgnnnnnnnncttcagcttcccgatatccgacggtagtgtctggtatatccagagtctt

SEQ ID NO: 364 - DNA, 83 bp, Artificial Sequence
  smMIP
  misc_feature (26)..(33): n is a, c, g, or t
gctatgaaaatgctaggcgtctgtgnnnnnnnncttcagcttcccgatatccgacggtagtgtcaattagaatgttactcaat

SEQ ID NO: 365 - DNA, 83 bp, Artificial Sequence
  smMIP
  misc_feature (30)..(37): n is a, c, g, or t
gcgttcctttgaggaaaattgacagacttnnnnnnnncttcagcttcccgatatccgacggtagtgtcaagaatgcaatgaga

SEQ ID NO: 366 - DNA, 83 bp, Artificial Sequence
  smMIP
  misc_feature (26)..(33): n is a, c, g, or t
gcctggaagcattacaacaccaaccnnnnnnnncttcagcttcccgatatccgacggtagtgttacgcacaatacttccaagg

SEQ ID NO: 367 - DNA, 83 bp, Artificial Sequence
  smMIP
  misc_feature (30)..(37): n is a, c, g, or t
tgcgccctggcagccctgaaggatgttcannnnnnnncttcagcttcccgatatccgacggtagtgtaagaaaaaacctctag

SEQ ID NO: 368 - DNA, 83 bp, Artificial Sequence
  smMIP
  misc_feature (30)..(37): n is a, c, g, or t
gaggaactggacagccacctgtcctacatnnnnnnnncttcagcttcccgatatccgacggtagtgtcagaaaacatcaggca

SEQ ID NO: 369 - DNA, 83 bp, Artificial Sequence
  smMIP
  misc_feature (29)..(36): n is a, c, g, or t
gtcacatgaagaggaccatccagacagcnnnnnnnncttcagcttcccgatatccgacggtagtgtaactcaacatcagaggc

SEQ ID NO: 370 - DNA, 83 bp, Artificial Sequence
  smMIP
  misc_feature (30)..(37): n is a, c, g, or t
gctgtcatgcggtgcctcctggcctatttnnnnnnnncttcagcttcccgatatccgacggtagtgtaccaagataaatatcg

SEQ ID NO: 371 - DNA, 83 bp, Artificial Sequence
  smMIP
  misc_feature (20)..(27): n is a, c, g, or t
acatcacccgggaacctgannnnnnnncttcagcttcccgatatccgacggtagtgtagcttccatatctcaagtgccctctg

SEQ ID NO: 372 - DNA, 83 bp, Artificial Sequence
  smMIP
  misc_feature (30)..(37): n is a, c, g, or t
gctggggaagcttctacttccagcatgctnnnnnnnncttcagcttcccgatatccgacggtagtgtaaccgccttcacagca

SEQ ID NO: 373 - DNA, 83 bp, Artificial Sequence
  smMIP
  misc_feature (27)..(34): n is a, c, g, or t
gtggagtgacttgttgagtgacctccnnnnnnnncttcagcttcccgatatccgacggtagtgtaaggactttcgggaacgag

SEQ ID NO: 374 - DNA, 83 bp, Artificial Sequence
  smMIP
  misc_feature (26)..(33): n is a, c, g, or t
gcaggatgggtgtggaagcagtgatnnnnnnnncttcagcttcccgatatccgacggtagtgtaaccaatcacctcagaagac

SEQ ID NO: 375 - DNA, 83 bp, Artificial Sequence
  smMIP
  misc_feature (30)..(37): n is a, c, g, or t
cattgggggctttgaggcttacacaggggnnnnnnnncttcagcttcccgatatccgacggtagtgttatgttgggggctgga

SEQ ID NO: 376 - DNA, 82 bp, Artificial Sequence
  smMIP
  misc_feature (28)..(35): n is a, c, g, or t
gctgaaggaccagacagattttgagcannnnnnnncttcagcttcccgatatccgacggtagtgttgaactggatgtctggg

SEQ ID NO: 377 - DNA, 81 bp, Artificial Sequence
  smMIP
  misc_feature (28)..(35): n is a, c, g, or t
gatgtggctgccagtggtgaggacttgnnnnnnnncttcagcttcccgatatccgacggtagtgtacgaggaggcgaagcg

SEQ ID NO: 378 - DNA, 83 bp, Artificial Sequence
  smMIP
  misc_feature (28)..(35): n is a, c, g, or t
cgcaggtatgcagacctcacagaagatnnnnnnnncttcagcttcccgatatccgacggtagtgtcaataaagcagaaactgc

SEQ ID NO: 379 - DNA, 83 bp, Artificial Sequence
  smMIP
  misc_feature (30)..(37): n is a, c, g, or t
cagatcaaggaggggaaacgtgtactgatnnnnnnnncttcagcttcccgatatccgacggtagtgtacagcaacatcagtaa

SEQ ID NO: 380 - DNA, 82 bp, Artificial Sequence
  smMIP
  misc_feature (26)..(33): n is a, c, g, or t
gcgcaaagccatggaagctgtggctnnnnnnnncttcagcttcccgatatccgacggtagtgtggagggtctctctgaagag

SEQ ID NO: 381 - DNA, 83 bp, Artificial Sequence
  smMIP
  misc_feature (21)..(28): n is a, c, g, or t
gccggcggggaggatactgtnnnnnnnncttcagcttcccgatatccgacggtagtgtggtattcccattgtctatgaattgg

SEQ ID NO: 382 - DNA, 83 bp, Artificial Sequence
  smMIP
  misc_feature (30)..(37): n is a, c, g, or t
gccaatgaggcaaagggaaccaaagtggtnnnnnnnncttcagcttcccgatatccgacggtagtgtaagctgacatcgcgct

SEQ ID NO: 383 - DNA, 83 bp, Artificial Sequence
  smMIP
  misc_feature (23)..(30): n is a, c, g, or t
gctgcaaaagtgggaactggagnnnnnnnncttcagcttcccgatatccgacggtagtgtgccaagggaattttatttgtggg

SEQ ID NO: 384 - DNA, 83 bp, Artificial Sequence
  smMIP
  misc_feature (30)..(37): n is a, c, g, or t
cccgtcaccctcattggagaagctgtcttnnnnnnnncttcagcttcccgatatccgacggtagtgtcagccaatattctcaa

SEQ ID NO: 385 - DNA, 83 bp, Artificial Sequence
  smMIP
  misc_feature (26)..(33): n is a, c, g, or t
gtcagctgttgaaaactgccaggacnnnnnnnncttcagcttcccgatatccgacggtagtgtttatggtggcatcgccctga

SEQ ID NO: 386 - DNA, 83 bp, Artificial Sequence
  smMIP
  misc_feature (24)..(31): n is a, c, g, or t
ccagggcagtttatccacaccaannnnnnnncttcagcttcccgatatccgacggtagtgtttcccatgccctgttttaccac

SEQ ID NO: 387 - DNA, 83 bp, Artificial Sequence
  smMIP
  misc_feature (21)..(28): n is a, c, g, or t
accgcttcaaccacttcagcnnnnnnnncttcagcttcccgatatccgacggtagtgtctcactcagtgtaccttctagtccc

SEQ ID NO: 388 - DNA, 83 bp, Artificial Sequence
  smMIP
  misc_feature (26)..(33): n is a, c, g, or t
gtggtttctccaggcggccaaggatnnnnnnnncttcagcttcccgatatccgacggtagtgtcaacattgatggaactcaca

SEQ ID NO: 389 - DNA, 83 bp, Artificial Sequence
  smMIP
  misc_feature (29)..(36): n is a, c, g, or t
gctgggtatctggtacatcaactgctttnnnnnnnncttcagcttcccgatatccgacggtagtgtactctccattgccctgc

SEQ ID NO: 390 - DNA, 82 bp, Artificial Sequence
  smMIP
  misc_feature (25)..(32): n is a, c, g, or t
gcatcacaagatcctcctggccaannnnnnnncttcagcttcccgatatccgacggtagtgtttgtgtggggggagccaggg

SEQ ID NO: 391 - DNA, 83 bp, Artificial Sequence
  smMIP
  misc_feature (30)..(37): n is a, c, g, or t
gctggctaagaaaatagagcctgagcttgnnnnnnnncttcagcttcccgatatccgacggtagtgtaccaagctcacaccat

SEQ ID NO: 392 - DNA, 83 bp, Artificial Sequence
  smMIP
  misc_feature (27)..(34): n is a, c, g, or t
caaccagaggattaaggctgctgtccnnnnnnnncttcagcttcccgatatccgacggtagtgtcccagctgtatttccaaaa

SEQ ID NO: 393 - DNA, 83 bp, Artificial Sequence
  smMIP
  misc_feature (27)..(34): n is a, c, g, or t
gctggagaacctccgctttcatgtggnnnnnnnncttcagcttcccgatatccgacggtagtgttccttagagccagttgctg

SEQ ID NO: 394 - DNA, 83 bp, Artificial Sequence
  smMIP
  misc_feature (23)..(30): n is a, c, g, or t
gcagacaagatccagctcatcannnnnnnncttcagcttcccgatatccgacggtagtgttccatggtaggagtcaatctgcc

SEQ ID NO: 395 - DNA, 83 bp, Artificial Sequence
  smMIP
  misc_feature (26)..(33): n is a, c, g, or t
gctggctggatgggcttggactgtgnnnnnnnncttcagcttcccgatatccgacggtagtgtaaagacctaatgtccaaagc

SEQ ID NO: 396 - DNA, 83 bp, Artificial Sequence
  smMIP
  misc_feature (30)..(37): n is a, c, g, or t
gtggtgccagtttggagctcctggaaggtnnnnnnnncttcagcttcccgatatccgacggtagtgtcatggatgaggtggtg

SEQ ID NO: 397 - DNA, 83 bp, Artificial Sequence
  smMIP
  misc_feature (27)..(34): n is a, c, g, or t
ccagattacaaacaaccagaggatcannnnnnnncttcagcttcccgatatccgacggtagtgtggtgtcagcctatgtcttt

SEQ ID NO: 398 - DNA, 83 bp, Artificial Sequence
  smMIP
  misc_feature (27)..(34): n is a, c, g, or t
gttcctgaaggactgtgtaggcgcagnnnnnnnncttcagcttcccgatatccgacggtagtgtaatggagccaaggcagtag

SEQ ID NO: 399 - DNA, 83 bp, Artificial Sequence
  smMIP
  misc_feature (28)..(35): n is a, c, g, or t
gctaaagccttggaaaacccagtgagannnnnnnncttcagcttcccgatatccgacggtagtgtgctaggggacgtctatgt

SEQ ID NO: 400 - DNA, 83 bp, Artificial Sequence
  smMIP
  misc_feature (30)..(37): n is a, c, g, or t
gtttgacgagaacgctcaggttggaaaagnnnnnnnncttcagcttcccgatatccgacggtagtgtatggagattggtgctt

SEQ ID NO: 401 - DNA, 83 bp, Artificial Sequence
  smMIP
  misc_feature (27)..(34): n is a, c, g, or t
gataaagtcagccatgtcagcactggnnnnnnnncttcagcttcccgatatccgacggtagtgtgggatgcctttgctaaggg

SEQ ID NO: 402 - DNA, 83 bp, Artificial Sequence
  smMIP
  misc_feature (20)..(27): n is a, c, g, or t
cccaaccccagagaaccaannnnnnnncttcagcttcccgatatccgacggtagtgtagaagtccccagcgccgttccttcca

SEQ ID NO: 403 - DNA, 83 bp, Artificial Sequence
  smMIP
  misc_feature (25)..(32): n is a, c, g, or t
cactaaaggacctgagatccgaacnnnnnnnncttcagcttcccgatatccgacggtagtgttggctcgtctgaacttctctc

SEQ ID NO: 404 - DNA, 83 bp, Artificial Sequence
  smMIP
  misc_feature (27)..(34): n is a, c, g, or t
gcaggatgttgatatggtgtttgcgtnnnnnnnncttcagcttcccgatatccgacggtagtgtctggtgacggaggtggaaa

SEQ ID NO: 405 - DNA, 83 bp, Artificial Sequence
  smMIP
  misc_feature (24)..(31): n is a, c, g, or t
gccaaaggggactatcctctggannnnnnnncttcagcttcccgatatccgacggtagtgtctgtcatctgtgctactcagat

SEQ ID NO: 406 - DNA, 83 bp, Artificial Sequence
  smMIP
  misc_feature (30)..(37): n is a, c, g, or t
acctccgggtgaactttgccatgaatgttnnnnnnnncttcagcttcccgatatccgacggtagtgtacgtgcccccatcatt

SEQ ID NO: 407 - DNA, 83 bp, Artificial Sequence
  smMIP
  misc_feature (26)..(33): n is a, c, g, or t
gttgtgttcttcttttaccctcttgnnnnnnnncttcagcttcccgatatccgacggtagtgtgctgataggaagatgtcttc

SEQ ID NO: 408 - DNA, 83 bp, Artificial Sequence
  smMIP
  misc_feature (28)..(35): n is a, c, g, or t
cgaagcgcaccattgctcaggattatgnnnnnnnncttcagcttcccgatatccgacggtagtgtaagaaactcaactgccaa

SEQ ID NO: 409 - DNA, 83 bp, Artificial Sequence
  smMIP
  misc_feature (27)..(34): n is a, c, g, or t
gcagatcactgtaaatgacctccctgnnnnnnnncttcagcttcccgatatccgacggtagtgtcccatgaacattcctttgg

SEQ ID NO: 410 - DNA, 83 bp, Artificial Sequence
  smMIP
  misc_feature (26)..(33): n is a, c, g, or t
acaaacatggggaagtgtgcccagcnnnnnnnncttcagcttcccgatatccgacggtagtgttctcgttcaggggccttttt

SEQ ID NO: 411 - DNA, 83 bp, Artificial Sequence
  smMIP
  misc_feature (25)..(32): n is a, c, g, or t
gctgggctgttttagtgccaggctnnnnnnnncttcagcttcccgatatccgacggtagtgttagttcaggccttccagttca

SEQ ID NO: 412 - DNA, 83 bp, Artificial Sequence
  smMIP
  misc_feature (27)..(34): n is a, c, g, or t
cagaacctcaagcttttcaggcatccnnnnnnnncttcagcttcccgatatccgacggtagtgttcggcaccttcggcaaagt

SEQ ID NO: 413 - DNA, 83 bp, Artificial Sequence
  smMIP
  misc_feature (27)..(34): n is a, c, g, or t
cacccaactatgctgcaccagaagtannnnnnnncttcagcttcccgatatccgacggtagtgtggtggtccatagagatttg

SEQ ID NO: 414 - DNA, 83 bp, Artificial Sequence
  smMIP
  misc_feature (30)..(37): n is a, c, g, or t
gagtgctcagaagaggaagttctcagctgnnnnnnnncttcagcttcccgatatccgacggtagtgtaagatatcagggaaca

SEQ ID NO: 415 - DNA, 83 bp, Artificial Sequence
  smMIP
  misc_feature (30)..(37): n is a, c, g, or t
ggattatgaatggaaggttgtaaacccatnnnnnnnncttcagcttcccgatatccgacggtagtgtgaattaaatccacaga

SEQ ID NO: 416 - DNA, 83 bp, Artificial Sequence
  smMIP
  misc_feature (30)..(37): n is a, c, g, or t
gtgcaaatctaattaaaattcttgcacaannnnnnnncttcagcttcccgatatccgacggtagtgttgctgaggctcaagga

SEQ ID NO: 417 - DNA, 83 bp, Artificial Sequence
  smMIP
  misc_feature (30)..(37): n is a, c, g, or t
cgagaaattcaaaatctaaaactctttcgnnnnnnnncttcagcttcccgatatccgacggtagtgttgggcgtcggcacctt

SEQ ID NO: 418 - DNA, 83 bp, Artificial Sequence
  smMIP
  misc_feature (30)..(37): n is a, c, g, or t
gccaagatagccgatttcggattatctaannnnnnnncttcagcttcccgatatccgacggtagtgtaagagatggaagccag

SEQ ID NO: 419 - DNA, 83 bp, Artificial Sequence
  smMIP
  misc_feature (19)..(26): n is a, c, g, or t
gctgcaggttgacccactnnnnnnnncttcagcttcccgatatccgacggtagtgttgtatgctcttctttgtggcaccctcc

SEQ ID NO: 420 - DNA, 83 bp, Artificial Sequence
  smMIP
  misc_feature (24)..(31): n is a, c, g, or t
gcagacagccccaaagcaagatgnnnnnnnncttcagcttcccgatatccgacggtagtgtgaataatgaaccaagccagtga

SEQ ID NO: 421 - DNA, 83 bp, Artificial Sequence
  smMIP
  misc_feature (19)..(26): n is a, c, g, or t
ccacaactgcagagagccnnnnnnnncttcagcttcccgatatccgacggtagtgtgttgataacaggagctatcttttggac

SEQ ID NO: 422 - DNA, 82 bp, Artificial Sequence
  smMIP
  misc_feature (26)..(33): n is a, c, g, or t
ctacaattgtccatgctgtgcagcgnnnnnnnncttcagcttcccgatatccgacggtagtgtactccaacagcatctgccc

SEQ ID NO: 423 - DNA, 83 bp, Artificial Sequence
  smMIP
  misc_feature (22)..(29): n is a, c, g, or t
ctcaatctcatcaagggtggcnnnnnnnncttcagcttcccgatatccgacggtagtgtcctcgtctgtattcccacttcctt

SEQ ID NO: 424 - DNA, 83 bp, Artificial Sequence
  smMIP
  misc_feature (23)..(30): n is a, c, g, or t
gctgtgagccagaagtttggggnnnnnnnncttcagcttcccgatatccgacggtagtgtgtggctggctatgctagtcgctt

SEQ ID NO: 425 - DNA, 83 bp, Artificial Sequence
  smMIP
  misc_feature (29)..(36): n is a, c, g, or t
gtttgaccgggtacacaaatggagtgaannnnnnnncttcagcttcccgatatccgacggtagtgtggcctatgtcccagtga

SEQ ID NO: 426 - DNA, 83 bp, Artificial Sequence
  smMIP
  misc_feature (30)..(37): n is a, c, g, or t
ggagcagagtgtgttcaccttgagtctccnnnnnnnncttcagcttcccgatatccgacggtagtgtatcaaaatgatcccag

SEQ ID NO: 427 - DNA, 82 bp, Artificial Sequence
  smMIP
  misc_feature (29)..(36): n is a, c, g, or t
gggcatctgctaaagtttcagattccatnnnnnnnncttcagcttcccgatatccgacggtagtgttgtcgggggtccgggg

SEQ ID NO: 428 - DNA, 83 bp, Artificial Sequence
  smMIP
  misc_feature (28)..(35): n is a, c, g, or t
gcatttggcctttctgaggcagggtttnnnnnnnncttcagcttcccgatatccgacggtagtgtcactgttgatgggaacaa

SEQ ID NO: 429 - DNA, 83 bp, Artificial Sequence
  smMIP
  misc_feature (29)..(36): n is a, c, g, or t
gcacagctagaaaattatggcatgccgtnnnnnnnncttcagcttcccgatatccgacggtagtgttttgatgcagtggtggt

SEQ ID NO: 430 - DNA, 83 bp, Artificial Sequence
  smMIP
  misc_feature (27)..(34): n is a, c, g, or t
gcctcaagtttggaaagggcgggcagnnnnnnnncttcagcttcccgatatccgacggtagtgtagcatgtgttaccaagctg

SEQ ID NO: 431 - DNA, 83 bp, Artificial Sequence
  smMIP
  misc_feature (29)..(36): n is a, c, g, or t
gcgatatgataccagctattttgtggagnnnnnnnncttcagcttcccgatatccgacggtagtgtttatcagcgtgcatttg

SEQ ID NO: 432 - DNA, 82 bp, Artificial Sequence
  smMIP
  misc_feature (24)..(31): n is a, c, g, or t
gcatagaggacgggtccatccatnnnnnnnncttcagcttcccgatatccgacggtagtgtgactggccactcgctattgca

SEQ ID NO: 433 - DNA, 83 bp, Artificial Sequence
  smMIP
  misc_feature (20)..(27): n is a, c, g, or t
cttcagctgcacgtctgccnnnnnnnncttcagcttcccgatatccgacggtagtgtttttgccttggatctcctgatggaga

SEQ ID NO: 434 - DNA, 83 bp, Artificial Sequence
  smMIP
  misc_feature (30)..(37): n is a, c, g, or t
gttcagttccaccctacaggcatatatggnnnnnnnncttcagcttcccgatatccgacggtagtgtctgttgttgccacagg

SEQ ID NO: 435 - DNA, 82 bp, Artificial Sequence
  smMIP
  misc_feature (28)..(35): n is a, c, g, or t
gcgaaaggtttatggagcgatacgcccnnnnnnnncttcagcttcccgatatccgacggtagtgtagggcaggccttccttg

SEQ ID NO: 436 - DNA, 83 bp, Artificial Sequence
  smMIP
  misc_feature (29)..(36): n is a, c, g, or t
cgagaaggaagaggctgtggccctgagannnnnnnncttcagcttcccgatatccgacggtagtgttgtcgtggagagggagg

SEQ ID NO: 437 - DNA, 83 bp, Artificial Sequence
  smMIP
  misc_feature (22)..(29): n is a, c, g, or t
gcctggcatttcagagacagcnnnnnnnncttcagcttcccgatatccgacggtagtgttggcgtctagagatgtggtgtctc

SEQ ID NO: 438 - DNA, 82 bp, Artificial Sequence
  smMIP
  misc_feature (23)..(30): n is a, c, g, or t
gcggcattcccaccaactacaannnnnnnncttcagcttcccgatatccgacggtagtgttgcaccacctacctccagagca

SEQ ID NO: 439 - DNA, 83 bp, Artificial Sequence
  smMIP
  misc_feature (21)..(28): n is a, c, g, or t
gcctcggtacatggtgccaannnnnnnncttcagcttcccgatatccgacggtagtgttccctgtcctccccaccgtgcatta

SEQ ID NO: 440 - DNA, 83 bp, Artificial Sequence
  smMIP
  misc_feature (28)..(35): n is a, c, g, or t
gcctggagataaagtccctccaattaannnnnnnncttcagcttcccgatatccgacggtagtgttgtacgcctgtggggagg

SEQ ID NO: 441 - DNA, 83 bp, Artificial Sequence
  smMIP
  misc_feature (26)..(33): n is a, c, g, or t
gctgatggaagcataagaacatcggnnnnnnnncttcagcttcccgatatccgacggtagtgtctggttgtctttggtcgggc

SEQ ID NO: 442 - DNA, 83 bp, Artificial Sequence
  smMIP
  misc_feature (25)..(32): n is a, c, g, or t
gcgtgttgcaagaaggttgtgggannnnnnnncttcagcttcccgatatccgacggtagtgtgctggggaagaatctgtcatg

SEQ ID NO: 443 - DNA, 83 bp, Artificial Sequence
  smMIP
  misc_feature (26)..(33): n is a, c, g, or t
gtctggaacacggacctggtggagannnnnnnncttcagcttcccgatatccgacggtagtgtatgcagaagtcaatgcaaaa

SEQ ID NO: 444 - DNA, 83 bp, Artificial Sequence
  smMIP
  misc_feature (22)..(29): n is a, c, g, or t
cagaggcacggaaggagtcacnnnnnnnncttcagcttcccgatatccgacggtagtgtatcagcaagctctatggagaccta

SEQ ID NO: 445 - DNA, 83 bp, Artificial Sequence
  smMIP
  misc_feature (25)..(32): n is a, c, g, or t
gcccatccaggggcaacagaagaannnnnnnncttcagcttcccgatatccgacggtagtgttggagctgcagaacctgatgc

SEQ ID NO: 446 - DNA, 83 bp, Artificial Sequence
  smMIP
  misc_feature (30)..(37): n is a, c, g, or t
ggaaggtcactctggaatatagacccgtgnnnnnnnncttcagcttcccgatatccgacggtagtgtggaagactacaaggtg

SEQ ID NO: 447 - DNA, 83 bp, Artificial Sequence
  smMIP
  misc_feature (26)..(33): n is a, c, g, or t
gtggtgatgacagaatcagcttttgnnnnnnnncttcagcttcccgatatccgacggtagtgtgtcctatgtggacgttggca

SEQ ID NO: 448 - DNA, 83 bp, Artificial Sequence
  smMIP
  misc_feature (28)..(35): n is a, c, g, or t
cccagacaaggctggagacaaacctcannnnnnnncttcagcttcccgatatccgacggtagtgttctccttgaggcgccggt

SEQ ID NO: 449 - DNA, 83 bp, Artificial Sequence
  smMIP
  misc_feature (28)..(35): n is a, c, g, or t
tgactctactttgaccttccgaagatcnnnnnnnncttcagcttcccgatatccgacggtagtgtttgccatctatcgatggg

SEQ ID NO: 450 - DNA, 83 bp, Artificial Sequence
  smMIP
  misc_feature (27)..(34): n is a, c, g, or t
cactctagcttgcacccgaaggattgnnnnnnnncttcagcttcccgatatccgacggtagtgttgtggccccatggtattgg

SEQ ID NO: 451 - DNA, 83 bp, Artificial Sequence
  smMIP
  misc_feature (30)..(37): n is a, c, g, or t
gatcttgttcccgatttgagcaacttctannnnnnnncttcagcttcccgatatccgacggtagtgttctgtggctcttgtgc

SEQ ID NO: 452 - DNA, 83 bp, Artificial Sequence
  smMIP
  misc_feature (25)..(32): n is a, c, g, or t
gcagcagtatctgcagtccatagannnnnnnncttcagcttcccgatatccgacggtagtgtcaaaaatctaccctcttccac

SEQ ID NO: 453 - DNA, 83 bp, Artificial Sequence
  smMIP
  misc_feature (30)..(37): n is a, c, g, or t
gctactggtggaacggagacaaatatctgnnnnnnnncttcagcttcccgatatccgacggtagtgtgaagaagaaggatgaa

SEQ ID NO: 454 - DNA, 83 bp, Artificial Sequence
  smMIP
  misc_feature (20)..(27): n is a, c, g, or t
agcgcctggccaagctgcannnnnnnncttcagcttcccgatatccgacggtagtgtagtgcattctctgtgcctgctgtagc

SEQ ID NO: 455 - DNA, 82 bp, Artificial Sequence
  smMIP
  misc_feature (29)..(36): n is a, c, g, or t
gcagagatcaagaaaatgatggcaacctnnnnnnnncttcagcttcccgatatccgacggtagtgtagagatgacttcacag

SEQ ID NO: 456 - DNA, 83 bp, Artificial Sequence
  smMIP
  misc_feature (19)..(26): n is a, c, g, or t
ccagctcagagctgaacannnnnnnncttcagcttcccgatatccgacggtagtgtatgaactgcacaaggacctgtcctaag

SEQ ID NO: 457 - DNA, 82 bp, Artificial Sequence
  smMIP
  misc_feature (29)..(36): n is a, c, g, or t
gctttgagtgcaggggtctctctttttgnnnnnnnncttcagcttcccgatatccgacggtagtgtgaagagatggagcggt

SEQ ID NO: 458 - DNA, 83 bp, Artificial Sequence
  smMIP
  misc_feature (21)..(28): n is a, c, g, or t
gcactgatccacacagctaannnnnnnncttcagcttcccgatatccgacggtagtgttgtccatctgccaccgtggcactgg

SEQ ID NO: 459 - DNA, 83 bp, Artificial Sequence
  smMIP
  misc_feature (24)..(31): n is a, c, g, or t
gcctgaagattccccagctatacnnnnnnnncttcagcttcccgatatccgacggtagtgttttggaacttgtgaagtccctg

SEQ ID NO: 460 - DNA, 83 bp, Artificial Sequence
  smMIP
  misc_feature (23)..(30): n is a, c, g, or t
cccagcatcatcttcctacacannnnnnnncttcagcttcccgatatccgacggtagtgtatccgacacttgatgtgggacct

SEQ ID NO: 461 - DNA, 83 bp, Artificial Sequence
  smMIP
  misc_feature (24)..(31): n is a, c, g, or t
cacttgtcaccgagccaccattcnnnnnnnncttcagcttcccgatatccgacggtagtgttgagtgccgtttgcggtgccct

SEQ ID NO: 462 - DNA, 83 bp, Artificial Sequence
  smMIP
  misc_feature (29)..(36): n is a, c, g, or t
gtctgcttccggctgcttatttgaatccnnnnnnnncttcagcttcccgatatccgacggtagtgtaccgacctatcccagaa

SEQ ID NO: 463 - DNA, 83 bp, Artificial Sequence
  smMIP
  misc_feature (29)..(36): n is a, c, g, or t
gttgttactgactatgttcatggggatgnnnnnnnncttcagcttcccgatatccgacggtagtgtgagagggttgtcagtgt

SEQ ID NO: 464 - DNA, 83 bp, Artificial Sequence
  smMIP
  misc_feature (27)..(34): n is a, c, g, or t
gctatttcaactatcacgatgtgggcnnnnnnnncttcagcttcccgatatccgacggtagtgtcctcactcttcatggtcac

SEQ ID NO: 465 - DNA, 83 bp, Artificial Sequence
  smMIP
  misc_feature (26)..(33): n is a, c, g, or t
gtatgcctctttgcctctgctttgtnnnnnnnncttcagcttcccgatatccgacggtagtgttggcactttcagctttaacc

SEQ ID NO: 466 - DNA, 82 bp, Artificial Sequence
  smMIP
  misc_feature (23)..(30): n is a, c, g, or t
cggcttctcttatgcatttcccnnnnnnnncttcagcttcccgatatccgacggtagtgtttggatttgacctgcattttgg

SEQ ID NO: 467 - DNA, 83 bp, Artificial Sequence
  smMIP
  misc_feature (26)..(33): n is a, c, g, or t
cgtctgtattggagtcattggaggtnnnnnnnncttcagcttcccgatatccgacggtagtgttggaggtcctatcagcagta

SEQ ID NO: 468 - DNA, 82 bp, Artificial Sequence
  smMIP
  misc_feature (28)..(35): n is a, c, g, or t
cagatcttattggaagacaccctaaacnnnnnnnncttcagcttcccgatatccgacggtagtgtgttgctggagccctcat

SEQ ID NO: 469 - DNA, 83 bp, Artificial Sequence
  smMIP
  misc_feature (30)..(37): n is a, c, g, or t
gttggattctgtgtctatgcgggattcttnnnnnnnncttcagcttcccgatatccgacggtagtgtgaccatctatgggact

SEQ ID NO: 470 - DNA, 78 bp, Artificial Sequence
  smMIP
  misc_feature (24)..(31): n is a, c, g, or t
ggagggcccaaggaggaggaaagnnnnnnnncttcagcttcccgatatccgacggtagtgttggcaaaagaacagaaa

SEQ ID NO: 471 - DNA, 83 bp, Artificial Sequence
  smMIP
  misc_feature (19)..(26): n is a, c, g, or t
gcggctttgtgctttacgnnnnnnnncttcagcttcccgatatccgacggtagtgtatcctgggcggcctgctgctcaactgc

SEQ ID NO: 472 - DNA, 81 bp, Artificial Sequence
  smMIP
  misc_feature (23)..(30): n is a, c, g, or t
gctctgcagtgtgtgcgtgaacnnnnnnnncttcagcttcccgatatccgacggtagtgtcttctcctacgccttccccaa

SEQ ID NO: 473 - DNA, 83 bp, Artificial Sequence
  smMIP
  misc_feature (22)..(29): n is a, c, g, or t
cgacaccaaggccgccttcctnnnnnnnncttcagcttcccgatatccgacggtagtgtgcctgctagacctgagcgtcttcc

SEQ ID NO: 474 - DNA, 83 bp, Artificial Sequence
  smMIP
  misc_feature (26)..(33): n is a, c, g, or t
cgacccacgtctacatgtacgtgttnnnnnnnncttcagcttcccgatatccgacggtagtgttgcagttcgaggtgctcatg

SEQ ID NO: 475 - DNA, 83 bp, Artificial Sequence
  smMIP
  misc_feature (30)..(37): n is a, c, g, or t
gcatttcctgaaggctgagcctgagaaaannnnnnnncttcagcttcccgatatccgacggtagtgtctgggcaacttcttct

SEQ ID NO: 476 - DNA, 82 bp, Artificial Sequence
  smMIP
  misc_feature (20)..(27): n is a, c, g, or t
cctatgcattccccaaagcnnnnnnnncttcagcttcccgatatccgacggtagtgtctcttggtgccaacagagttactct

SEQ ID NO: 477 - DNA, 83 bp, Artificial Sequence
  smMIP
  misc_feature (29)..(36): n is a, c, g, or t
gcaacccgccttaaccataattggcaaannnnnnnncttcagcttcccgatatccgacggtagtgtggtggtgatagcaggag

SEQ ID NO: 478 - DNA, 83 bp, Artificial Sequence
  smMIP
  misc_feature (30)..(37): n is a, c, g, or t
ccctttttaagcatagaggatttctgatannnnnnnncttcagcttcccgatatccgacggtagtgtacccaatcaaaccact

SEQ ID NO: 479 - DNA, 83 bp, Artificial Sequence
  smMIP
  misc_feature (22)..(29): n is a, c, g, or t
gtgttagcagtgttctctttgnnnnnnnncttcagcttcccgatatccgacggtagtgtcgacctcgaattcagtacttcttc

SEQ ID NO: 480 - DNA, 83 bp, Artificial Sequence
  smMIP
  misc_feature (26)..(33): n is a, c, g, or t
ccttgagcaaatctaaacattcggannnnnnnncttcagcttcccgatatccgacggtagtgttgtcctgtggggctattgtg

SEQ ID NO: 481 - DNA, 83 bp, Artificial Sequence
  smMIP
  misc_feature (30)..(37): n is a, c, g, or t
gctctggtccctctcagtggccatcttttnnnnnnnncttcagcttcccgatatccgacggtagtgttccctgcagtttggct

SEQ ID NO: 482 - DNA, 83 bp, Artificial Sequence
  smMIP
  misc_feature (19)..(26): n is a, c, g, or t
tcacccacagcccttcgtnnnnnnnncttcagcttcccgatatccgacggtagtgtcttcgtgtccgccgtgctcatgggctt

SEQ ID NO: 483 - DNA, 78 bp, Artificial Sequence
  smMIP
  misc_feature (24)..(31): n is a, c, g, or t
gcatcttcgagaaggcgggggtgnnnnnnnncttcagcttcccgatatccgacggtagtgtggagaagaaggtcacca

SEQ ID NO: 484 - DNA, 81 bp, Artificial Sequence
  smMIP
  misc_feature (25)..(32): n is a, c, g, or t
gccccatcccatggttcatcgtggnnnnnnnncttcagcttcccgatatccgacggtagtgtgctggcatggcgggttgtg

SEQ ID NO: 485 - DNA, 83 bp, Artificial Sequence
  smMIP
  misc_feature (19)..(26): n is a, c, g, or t
ttccatcccctgggggctnnnnnnnncttcagcttcccgatatccgacggtagtgttgtgctcctggttctgttcttcatctt

SEQ ID NO: 486 - DNA, 83 bp, Artificial Sequence
  smMIP
  misc_feature (28)..(35): n is a, c, g, or t
cactggggtcatcaatgctcctgagaannnnnnnncttcagcttcccgatatccgacggtagtgtatcacccctagatctttc

SEQ ID NO: 487 - DNA, 78 bp, Artificial Sequence
  smMIP
  misc_feature (20)..(27): n is a, c, g, or t
gccctgcggggtgcctttgnnnnnnnncttcagcttcccgatatccgacggtagtgtggctgctttatgggactgtgt

SEQ ID NO: 488 - DNA, 83 bp, Artificial Sequence
  smMIP
  misc_feature (27)..(34): n is a, c, g, or t
ccattgtgctccagctctctcagcagnnnnnnnncttcagcttcccgatatccgacggtagtgtcacccaggatgtatcccaa

SEQ ID NO: 489 - DNA, 83 bp, Artificial Sequence
  smMIP
  misc_feature (19)..(26): n is a, c, g, or t
actcttcagccagggcccnnnnnnnncttcagcttcccgatatccgacggtagtgtcgctcatgactgtttctttgttattaa

SEQ ID NO: 490 - DNA, 83 bp, Artificial Sequence
  smMIP
  misc_feature (25)..(32): n is a, c, g, or t
gcctgctaaggagaccaccaccaannnnnnnncttcagcttcccgatatccgacggtagtgtttaccttcttcaaagtccctg

SEQ ID NO: 491 - DNA, 83 bp, Artificial Sequence
  smMIP
  misc_feature (22)..(29): n is a, c, g, or t
cattttcaccaagatctcggcnnnnnnnncttcagcttcccgatatccgacggtagtgtttgtgctgggctggctgtttgtcc

SEQ ID NO: 492 - DNA, 83 bp, Artificial Sequence
  smMIP
  misc_feature (22)..(29): n is a, c, g, or t
catcttccgagatcccctcacnnnnnnnncttcagcttcccgatatccgacggtagtgtttgcttttcacgaagtgggaggct

SEQ ID NO: 493 - DNA, 83 bp, Artificial Sequence
  smMIP
  misc_feature (26)..(33): n is a, c, g, or t
gtcatgctggcctccctcatgagctnnnnnnnncttcagcttcccgatatccgacggtagtgtattgcctgtgtcgtcccttc

SEQ ID NO: 494 - DNA, 83 bp, Artificial Sequence
  smMIP
  misc_feature (20)..(27): n is a, c, g, or t
agcccagcaactgtcccacnnnnnnnncttcagcttcccgatatccgacggtagtgtctgtcttcctgcttgctattttctgg

SEQ ID NO: 495 - DNA, 83 bp, Artificial Sequence
  smMIP
  misc_feature (27)..(34): n is a, c, g, or t
catcctggtgaccgtggctgtcttttnnnnnnnncttcagcttcccgatatccgacggtagtgtttttgtgggctagagcagc

SEQ ID NO: 496 - DNA, 83 bp, Artificial Sequence
  smMIP
  misc_feature (23)..(30): n is a, c, g, or t
gccagcaagcagatcactgcagnnnnnnnncttcagcttcccgatatccgacggtagtgttctttcaacatgacagatgccgc

SEQ ID NO: 497 - DNA, 83 bp, Artificial Sequence
  smMIP
  misc_feature (27)..(34): n is a, c, g, or t
cccagttttggctctactttgcagggnnnnnnnncttcagcttcccgatatccgacggtagtgtgggagttctgtccttctgg

SEQ ID NO: 498 - DNA, 83 bp, Artificial Sequence
  smMIP
  misc_feature (24)..(31): n is a, c, g, or t
gctttaacgtgtctgtgcagggtnnnnnnnncttcagcttcccgatatccgacggtagtgttcttgattttgcccgtacccgt

SEQ ID NO: 499 - DNA, 81 bp, Artificial Sequence
  smMIP
  misc_feature (28)..(35): n is a, c, g, or t
gcatgatgatgcagtcagggcgcaaagnnnnnnnncttcagcttcccgatatccgacggtagtgtgacactgcaaagggaa

SEQ ID NO: 500 - DNA, 83 bp, Artificial Sequence
  smMIP
  misc_feature (30)..(37): n is a, c, g, or t
cataagttatttcctaggatttttcccccnnnnnnnncttcagcttcccgatatccgacggtagtgtctggcggaagattgct

SEQ ID NO: 501 - DNA, 82 bp, Artificial Sequence
  smMIP
  misc_feature (23)..(30): n is a, c, g, or t
cacttttgatctggtggccctcnnnnnnnncttcagcttcccgatatccgacggtagtgtttcccgtcatattccagctctg

SEQ ID NO: 502 - DNA, 83 bp, Artificial Sequence
  smMIP
  misc_feature (23)..(30): n is a, c, g, or t
ccccggcgtgctggctgaaaacnnnnnnnncttcagcttcccgatatccgacggtagtgtcggctggaacttaatcctctcct

SEQ ID NO: 503 - DNA, 83 bp, Artificial Sequence
  smMIP
  misc_feature (22)..(29): n is a, c, g, or t
gctgggaaggtgccaagtacgnnnnnnnncttcagcttcccgatatccgacggtagtgtgtggggatcgtggcgtccctcttg

SEQ ID NO: 504 - DNA, 82 bp, Artificial Sequence
  smMIP
  misc_feature (25)..(32): n is a, c, g, or t
ggcaagcaccaatgattcccagctnnnnnnnncttcagcttcccgatatccgacggtagtgtctctcctggcttactcgttg

SEQ ID NO: 505 - DNA, 83 bp, Artificial Sequence
  smMIP
  misc_feature (24)..(31): n is a, c, g, or t
cgtgaacgtctatctcatgatgcnnnnnnnncttcagcttcccgatatccgacggtagtgttttctgctcgcagggtctgccc

SEQ ID NO: 506 - DNA, 82 bp, Artificial Sequence
  smMIP
  misc_feature (24)..(31): n is a, c, g, or t
tcccctcacagactcttccaccannnnnnnncttcagcttcccgatatccgacggtagtgtcagtgacagccccagctccca

SEQ ID NO: 507 - DNA, 83 bp, Artificial Sequence
  smMIP
  misc_feature (27)..(34): n is a, c, g, or t
gcctcatgaagataggtttccatgtgnnnnnnnncttcagcttcccgatatccgacggtagtgtccgccctgttaatcattcc

SEQ ID NO: 508 - DNA, 79 bp, Artificial Sequence
  smMIP
  misc_feature (23)..(30): n is a, c, g, or t
gcggggtgcttgtgggcgtggtnnnnnnnncttcagcttcccgatatccgacggtagtgtgggagtccttgctcaatga

SEQ ID NO: 509 - DNA, 82 bp, Artificial Sequence
  smMIP
  misc_feature (25)..(32): n is a, c, g, or t
gcccctggtagacctgttggctgtnnnnnnnncttcagcttcccgatatccgacggtagtgtgaggggccatcgccttctct

SEQ ID NO: 510 - DNA, 83 bp, Artificial Sequence
  smMIP
  misc_feature (30)..(37): n is a, c, g, or t
gcagctggagcagaagatcaacaactaccnnnnnnnncttcagcttcccgatatccgacggtagtgtatcctgaggaacaact

SEQ ID NO: 511 - DNA, 82 bp, Artificial Sequence
  smMIP
  misc_feature (27)..(34): n is a, c, g, or t
gcctgtgtgacaagctggggaagaatnnnnnnnncttcagcttcccgatatccgacggtagtgtgggaggagaggttagatg

SEQ ID NO: 512 - DNA, 83 bp, Artificial Sequence
  smMIP
  misc_feature (26)..(33): n is a, c, g, or t
gctggggcctgggaagaagaatgatnnnnnnnncttcagcttcccgatatccgacggtagtgttaaggctagtggccgcttgg

SEQ ID NO: 513 - DNA, 83 bp, Artificial Sequence
  smMIP
  misc_feature (29)..(36): n is a, c, g, or t
gctgatggtggatttcttcaacattttgnnnnnnnncttcagcttcccgatatccgacggtagtgtggaggagactaagatgg

SEQ ID NO: 514 - DNA, 83 bp, Artificial Sequence
  smMIP
  misc_feature (19)..(26): n is a, c, g, or t
cgtccttcctgttggagcnnnnnnnncttcagcttcccgatatccgacggtagtgtccttctccttttttgctggcattttcc

SEQ ID NO: 515 - DNA, 83 bp, Artificial Sequence
  smMIP
  misc_feature (30)..(37): n is a, c, g, or t
cgagtgcatgaagatattgaaatgaccaannnnnnnncttcagcttcccgatatccgacggtagtgttggctgtggactggct

SEQ ID NO: 516 - DNA, 81 bp, Artificial Sequence
  smMIP
  misc_feature (26)..(33): n is a, c, g, or t
ggactgactgaaggcctgcatggatnnnnnnnncttcagcttcccgatatccgacggtagtgtgtggcctagcgagttatg

SEQ ID NO: 517 - DNA, 81 bp, Artificial Sequence
  smMIP
  misc_feature (27)..(34): n is a, c, g, or t
gtgggccaaaggatgaagagaggcatnnnnnnnncttcagcttcccgatatccgacggtagtgtggtgtggggaagcatta

SEQ ID NO: 518 - DNA, 83 bp, Artificial Sequence
  smMIP
  misc_feature (24)..(31): n is a, c, g, or t
tctcactctcaggagaccattgcnnnnnnnncttcagcttcccgatatccgacggtagtgttcctcactttaatcctctatcc

SEQ ID NO: 519 - DNA, 83 bp, Artificial Sequence
  smMIP
  misc_feature (28)..(35): n is a, c, g, or t
gtacaaagacaggaaacgctggaagtcnnnnnnnncttcagcttcccgatatccgacggtagtgtggtgtggccgatgtgtct

SEQ ID NO: 520 - DNA, 83 bp, Artificial Sequence
  smMIP
  misc_feature (28)..(35): n is a, c, g, or t
cccttggatgtagtctgaggccccttannnnnnnncttcagcttcccgatatccgacggtagtgtgcacactggtggtccatg

SEQ ID NO: 521 - DNA, 82 bp, Artificial Sequence
  smMIP
  misc_feature (25)..(32): n is a, c, g, or t
gccctggaacctcacatcaacgcgnnnnnnnncttcagcttcccgatatccgacggtagtgttagcaccagcactagcagca

SEQ ID NO: 522 - DNA, 81 bp, Artificial Sequence
  smMIP
  misc_feature (27)..(34): n is a, c, g, or t
gcgttggccaagggagatgttacagcnnnnnnnncttcagcttcccgatatccgacggtagtgtacctgccctacgactac

SEQ ID NO: 523 - DNA, 82 bp, Artificial Sequence
  smMIP
  misc_feature (26)..(33): n is a, c, g, or t
gctcaggttggggttggcttggtttnnnnnnnncttcagcttcccgatatccgacggtagtgtggacaaacctcagccctaa

SEQ ID NO: 524 - DNA, 83 bp, Artificial Sequence
  smMIP
  misc_feature (30)..(37): n is a, c, g, or t
gggagaatgtaactgaaagatacatggctnnnnnnnncttcagcttcccgatatccgacggtagtgtactgcaaggaacaaca

SEQ ID NO: 525 - DNA, 83 bp, Artificial Sequence
  smMIP
  misc_feature (29)..(36): n is a, c, g, or t
gctgagtatgttaagctctttatgactgnnnnnnnncttcagcttcccgatatccgacggtagtgtcgcttactaccttcagt

SEQ ID NO: 526 - DNA, 78 bp, Artificial Sequence
  smMIP
  misc_feature (23)..(30): n is a, c, g, or t
gaagattccgggccgagtatccnnnnnnnncttcagcttcccgatatccgacggtagtgtgatgcccgcttaccagga

SEQ ID NO: 527 - DNA, 83 bp, Artificial Sequence
  smMIP
  misc_feature (24)..(31): n is a, c, g, or t
tcgaggagcagcacggcatccacnnnnnnnncttcagcttcccgatatccgacggtagtgttgataaagatgcgatggtggcc

SEQ ID NO: 528 - DNA, 82 bp, Artificial Sequence
  smMIP
  misc_feature (29)..(36): n is a, c, g, or t
gtttagctacaaaaccattgtcatgggcnnnnnnnncttcagcttcccgatatccgacggtagtgtcatctccccatttgtt

SEQ ID NO: 529 - DNA, 82 bp, Artificial Sequence
  smMIP
  misc_feature (25)..(32): n is a, c, g, or t
ccacctggatgagaagtctttccgnnnnnnnncttcagcttcccgatatccgacggtagtgtaagcactggccggctgtgac

SEQ ID NO: 530 - DNA, 82 bp, Artificial Sequence
  smMIP
  misc_feature (26)..(33): n is a, c, g, or t
gaggctggactccagatctgcaccgnnnnnnnncttcagcttcccgatatccgacggtagtgtgaggaccagatggctgtgg

SEQ ID NO: 531 - DNA, 83 bp, Artificial Sequence
  smMIP
  misc_feature (28)..(35): n is a, c, g, or t
catgaggacaaagcagaccatgcatggnnnnnnnncttcagcttcccgatatccgacggtagtgtaggagaaaataatccaag

SEQ ID NO: 532 - DNA, 82 bp, Artificial Sequence
  smMIP
  misc_feature (29)..(36): n is a, c, g, or t
cggaggagagacgctggaccaggtgaaannnnnnnncttcagcttcccgatatccgacggtagtgtgacggtaaagtatgac

SEQ ID NO: 533 - DNA, 83 bp, Artificial Sequence
  smMIP
  misc_feature (28)..(35): n is a, c, g, or t
ggattagcagccagtgtcttagttgtgnnnnnnnncttcagcttcccgatatccgacggtagtgtagcggatcaaaaagaaca

SEQ ID NO: 534 - DNA, 83 bp, Artificial Sequence
  smMIP
  misc_feature (30)..(37): n is a, c, g, or t
gaggaaggaagagaagttaaaccaacggtnnnnnnnncttcagcttcccgatatccgacggtagtgttgagaagtctgtttga

SEQ ID NO: 535 - DNA, 82 bp, Artificial Sequence
  smMIP
  misc_feature (23)..(30): n is a, c, g, or t
gtgaagtcctcctgaaggtggcnnnnnnnncttcagcttcccgatatccgacggtagtgtctgccctgtcctgtcctgccct

SEQ ID NO: 536 - DNA, 82 bp, Artificial Sequence
  smMIP
  misc_feature (29)..(36): n is a, c, g, or t
gcaacattttgggacttgaggcatctggnnnnnnnncttcagcttcccgatatccgacggtagtgttgaaggaggtggccaa

SEQ ID NO: 537 - DNA, 83 bp, Artificial Sequence
  smMIP
  misc_feature (24)..(31): n is a, c, g, or t
gccatggctctgctccccggtggnnnnnnnncttcagcttcccgatatccgacggtagtgtacttaatgcagagacaaggcca

SEQ ID NO: 538 - DNA, 83 bp, Artificial Sequence
  smMIP
  misc_feature (28)..(35): n is a, c, g, or t
gctaatccatgcaggactgagtggtgtnnnnnnnncttcagcttcccgatatccgacggtagtgtaagggctcctcatgccta

SEQ ID NO: 539 - DNA, 83 bp, Artificial Sequence
  smMIP
  misc_feature (27)..(34): n is a, c, g, or t
gcttcaaatggcagaaaagcttggagnnnnnnnncttcagcttcccgatatccgacggtagtgtggaaatgttcaggctggag

SEQ ID NO: 540 - DNA, 83 bp, Artificial Sequence
  smMIP
  misc_feature (28)..(35): n is a, c, g, or t
gctggagttaatcttattctagactgcnnnnnnnncttcagcttcccgatatccgacggtagtgttattcctctggtcacagc

SEQ ID NO: 541 - DNA, 83 bp, Artificial Sequence
  smMIP
  misc_feature (29)..(36): n is a, c, g, or t
gtcgatgggttctctatggtctgatgggnnnnnnnncttcagcttcccgatatccgacggtagtgtacaaaaaagaggatttc

SEQ ID NO: 542 - DNA, 83 bp, Artificial Sequence
  smMIP
  misc_feature (27)..(34): n is a, c, g, or t
gctgaggtctagggacaataagtacannnnnnnncttcagcttcccgatatccgacggtagtgtaagaacgtcaactgcctgg

SEQ ID NO: 543 - DNA, 83 bp, Artificial Sequence
  smMIP
  misc_feature (20)..(27): n is a, c, g, or t
agggcccccaacgtctgctnnnnnnnncttcagcttcccgatatccgacggtagtgtggcccctgttttcaaagctacttttt

SEQ ID NO: 544 - DNA, 83 bp, Artificial Sequence
  smMIP
  misc_feature (25)..(32): n is a, c, g, or t
tcgtcctggaactgccccagtgaannnnnnnncttcagcttcccgatatccgacggtagtgtcaaattctgcctcacttctcc

SEQ ID NO: 545 - DNA, 83 bp, Artificial Sequence
  smMIP
  misc_feature (20)..(27): n is a, c, g, or t
cttctcagccacgtggtgtnnnnnnnncttcagcttcccgatatccgacggtagtgttttggatccatttccatcggtcctta

SEQ ID NO: 546 - DNA, 83 bp, Artificial Sequence
  smMIP
  misc_feature (30)..(37): n is a, c, g, or t
gttttttaagaagggacaaaaggtgggtgnnnnnnnncttcagcttcccgatatccgacggtagtgtgcaggtgataaacttg

SEQ ID NO: 547 - DNA, 83 bp, Artificial Sequence
  smMIP
  misc_feature (30)..(37): n is a, c, g, or t
gttttctgaaaatataaccagccattggcnnnnnnnncttcagcttcccgatatccgacggtagtgtagagtgtgaagtcaaa

SEQ ID NO: 548 - DNA, 83 bp, Artificial Sequence
  smMIP
  misc_feature (26)..(33): n is a, c, g, or t
gccgtgatcagttggactaaggatgnnnnnnnncttcagcttcccgatatccgacggtagtgtgtttagttgaggataccaca

SEQ ID NO: 549 - DNA, 83 bp, Artificial Sequence
  smMIP
  misc_feature (30)..(37): n is a, c, g, or t
cgatggtgcggaagattttgtcagtgagannnnnnnncttcagcttcccgatatccgacggtagtgtccacgcctagagactc

SEQ ID NO: 550 - DNA, 83 bp, Artificial Sequence
  smMIP
  misc_feature (25)..(32): n is a, c, g, or t
gccggtgttaacaccacggacaaannnnnnnncttcagcttcccgatatccgacggtagtgtgacgtagagtttgtctgcaag

SEQ ID NO: 551 - DNA, 83 bp, Artificial Sequence
  smMIP
  misc_feature (29)..(36): n is a, c, g, or t
actacctggagatagccatttactgcatnnnnnnnncttcagcttcccgatatccgacggtagtgtttttgaggacgctgggg

SEQ ID NO: 552 - DNA, 83 bp, Artificial Sequence
  smMIP
  misc_feature (29)..(36): n is a, c, g, or t
gcagtgttaaaacatgaatgactgtgtcnnnnnnnncttcagcttcccgatatccgacggtagtgtcgaacagtattcaccta

SEQ ID NO: 553 - DNA, 83 bp, Artificial Sequence
  smMIP
  misc_feature (24)..(31): n is a, c, g, or t
cgtgctgcccgtatggctcaactnnnnnnnncttcagcttcccgatatccgacggtagtgtaagagtccggcccggaggaact

SEQ ID NO: 554 - DNA, 83 bp, Artificial Sequence
  smMIP
  misc_feature (24)..(31): n is a, c, g, or t
gctcttcagagatgcagggacacnnnnnnnncttcagcttcccgatatccgacggtagtgttcttctgcaatcgcagtccgcg

SEQ ID NO: 555 - DNA, 80 bp, Artificial Sequence
  smMIP
  misc_feature (22)..(29): n is a, c, g, or t
gcgccgaggaggagatggaggnnnnnnnncttcagcttcccgatatccgacggtagtgtagaactgggacgaggccgagg

SEQ ID NO: 556 - DNA, 82 bp, Artificial Sequence
  smMIP
  misc_feature (22)..(29): n is a, c, g, or t
agtcgggcgccgaggagtccgnnnnnnnncttcagcttcccgatatccgacggtagtgtggcgtccggcccgggtggtctgg

SEQ ID NO: 557 - DNA, 82 bp, Artificial Sequence
  smMIP
  misc_feature (25)..(32): n is a, c, g, or t
ctcaatgttgacggacagcctattnnnnnnnncttcagcttcccgatatccgacggtagtgttacccaacgctgccgcctgg

SEQ ID NO: 558 - DNA, 83 bp, Artificial Sequence
  smMIP
  misc_feature (30)..(37): n is a, c, g, or t
gtccggagcctagtcaagcctgagaattannnnnnnncttcagcttcccgatatccgacggtagtgtcgatgggcttctggtt

SEQ ID NO: 559 - DNA, 83 bp, Artificial Sequence
  smMIP
  misc_feature (29)..(36): n is a, c, g, or t
gcggctgacacaggagcgcattgcacatnnnnnnnncttcagcttcccgatatccgacggtagtgtaaagagcgatgcctcca

SEQ ID NO: 560 - DNA, 83 bp, Artificial Sequence
  smMIP
  misc_feature (27)..(34): n is a, c, g, or t
gcttttgatggtactgatgagtcttgnnnnnnnncttcagcttcccgatatccgacggtagtgttacgaagatctggaagacc

SEQ ID NO: 561 - DNA, 83 bp, Artificial Sequence
  smMIP
  misc_feature (22)..(29): n is a, c, g, or t
gatgtgcacgcccggctgcaannnnnnnncttcagcttcccgatatccgacggtagtgtaacacggaggcaatcgactgcatc

SEQ ID NO: 562 - DNA, 82 bp, Artificial Sequence
  smMIP
  misc_feature (29)..(36): n is a, c, g, or t
gatggtgtacctggcgggtctgcattttnnnnnnnncttcagcttcccgatatccgacggtagtgtctcaaccgcttcctcc

SEQ ID NO: 563 - DNA, 83 bp, Artificial Sequence
  smMIP
  misc_feature (30)..(37): n is a, c, g, or t
catcgtgaagagtggtctccgtttcgtggnnnnnnnncttcagcttcccgatatccgacggtagtgtatagcctccaccacct

SEQ ID NO: 564 - DNA, 83 bp, Artificial Sequence
  smMIP
  misc_feature (26)..(33): n is a, c, g, or t
gcaaaggctctgggctccaaggccannnnnnnncttcagcttcccgatatccgacggtagtgtcaacaaatgtggacggagaa

SEQ ID NO: 565 - DNA, 83 bp, Artificial Sequence
  smMIP
  misc_feature (25)..(32): n is a, c, g, or t
gcagggatatctacagcaccgactnnnnnnnncttcagcttcccgatatccgacggtagtgttggctagccaggtcgctgcgg

SEQ ID NO: 566 - DNA, 82 bp, Artificial Sequence
  smMIP
  misc_feature (20)..(27): n is a, c, g, or t
agtcaacacctcctcaaccnnnnnnnncttcagcttcccgatatccgacggtagtgtctctatactgccgtgcagcccaatg

SEQ ID NO: 567 - DNA, 80 bp, Artificial Sequence
  smMIP
  misc_feature (22)..(29): n is a, c, g, or t
cggtggtgtgggaacggatgtnnnnnnnncttcagcttcccgatatccgacggtagtgttgctgttgctgtctctcctgt

SEQ ID NO: 568 - DNA, 83 bp, Artificial Sequence
  smMIP
  misc_feature (30)..(37): n is a, c, g, or t
cgtggcttttctggtatctttgaggacagnnnnnnnncttcagcttcccgatatccgacggtagtgtcatctttctcacggaa

SEQ ID NO: 569 - DNA, 83 bp, Artificial Sequence
  smMIP
  misc_feature (28)..(35): n is a, c, g, or t
gtccgagtgctggagctaagtgagagcnnnnnnnncttcagcttcccgatatccgacggtagtgtcggtatgtgtcagagctg

SEQ ID NO: 570 - DNA, 83 bp, Artificial Sequence
  smMIP
  misc_feature (26)..(33): n is a, c, g, or t
gccaatggcatggagtttctggcctnnnnnnnncttcagcttcccgatatccgacggtagtgtccaactacatggccccttac

SEQ ID NO: 571 - DNA, 83 bp, Artificial Sequence
  smMIP
  misc_feature (19)..(26): n is a, c, g, or t
ttcggccccagcccccttnnnnnnnncttcagcttcccgatatccgacggtagtgttccccacacatgaccccagccctctac

SEQ ID NO: 572 - DNA, 83 bp, Artificial Sequence
  smMIP
  misc_feature (21)..(28): n is a, c, g, or t
gccctgggaccagctctttcnnnnnnnncttcagcttcccgatatccgacggtagtgtacaatggcgcctactcgctgaccct

SEQ ID NO: 573 - DNA, 83 bp, Artificial Sequence
  smMIP
  misc_feature (26)..(33): n is a, c, g, or t
cacgattttgtggaaggacatcttcnnnnnnnncttcagcttcccgatatccgacggtagtgtaacaataccacccctgtcac

SEQ ID NO: 574 - DNA, 83 bp, Artificial Sequence
  smMIP
  misc_feature (28)..(35): n is a, c, g, or t
gcaagaagatctttgggagcctggcatnnnnnnnncttcagcttcccgatatccgacggtagtgtatggaacacagcggtgtg

SEQ ID NO: 575 - DNA, 79 bp, Artificial Sequence
  smMIP
  misc_feature (26)..(33): n is a, c, g, or t
gctggctccgatgtatttgatggtgnnnnnnnncttcagcttcccgatatccgacggtagtgtctgggggcatggtcca

SEQ ID NO: 576 - DNA, 83 bp, Artificial Sequence
  smMIP
  misc_feature (29)..(36): n is a, c, g, or t
gcgagagccccacatgaggaagaacatcnnnnnnnncttcagcttcccgatatccgacggtagtgtaaacagccctggtacca

SEQ ID NO: 577 - DNA, 83 bp, Artificial Sequence
  smMIP
  misc_feature (28)..(35): n is a, c, g, or t
gcaacctgcagcacatcaattttacccnnnnnnnncttcagcttcccgatatccgacggtagtgtcaaaccagaaaaggttag

SEQ ID NO: 578 - DNA, 83 bp, Artificial Sequence
  smMIP
  misc_feature (28)..(35): n is a, c, g, or t
gcagatctcttgtgtggcggaaaatctnnnnnnnncttcagcttcccgatatccgacggtagtgtaggtgatccggttcctaa

SEQ ID NO: 579 - DNA, 83 bp, Artificial Sequence
  smMIP
  misc_feature (26)..(33): n is a, c, g, or t
cggggacaccacgaacagaagtaatnnnnnnnncttcagcttcccgatatccgacggtagtgtgagtatgggaaggatgagaa

SEQ ID NO: 580 - DNA, 83 bp, Artificial Sequence
  smMIP
  misc_feature (26)..(33): n is a, c, g, or t
gctgaatgctataacctctgtcctgnnnnnnnncttcagcttcccgatatccgacggtagtgtatccccagtactttggcatc

SEQ ID NO: 581 - DNA, 83 bp, Artificial Sequence
  smMIP
  misc_feature (26)..(33): n is a, c, g, or t
gcacaactgatcccgagactcctgtnnnnnnnncttcagcttcccgatatccgacggtagtgtgaatgagcttgaaggcaggc

SEQ ID NO: 582 - DNA, 82 bp, Artificial Sequence
  smMIP
  misc_feature (28)..(35): n is a, c, g, or t
gtaataatgaaacttcctggactatttnnnnnnnncttcagcttcccgatatccgacggtagtgtcatccattctggacttg

SEQ ID NO: 583 - DNA, 83 bp, Artificial Sequence
  smMIP
  misc_feature (30)..(37): n is a, c, g, or t
cgacatccagagatcactctatgatcgtcnnnnnnnncttcagcttcccgatatccgacggtagtgtaaagcacacggagcta

SEQ ID NO: 584 - DNA, 79 bp, Artificial Sequence
  smMIP
  misc_feature (25)..(32): n is a, c, g, or t
gtgggtaccggatggccaagcctgnnnnnnnncttcagcttcccgatatccgacggtagtgtacaacctctacaccaca

SEQ ID NO: 585 - DNA, 83 bp, Artificial Sequence
  smMIP
  misc_feature (25)..(32): n is a, c, g, or t
catcaagagagaggacgagaccatnnnnnnnncttcagcttcccgatatccgacggtagtgtctacatcattcctctgcctga

SEQ ID NO: 586 - DNA, 82 bp, Artificial Sequence
  smMIP
  misc_feature (29)..(36): n is a, c, g, or t
cgtcaatgtttcagatgctctcccctccnnnnnnnncttcagcttcccgatatccgacggtagtgtgaaagcaaccgcaccc

SEQ ID NO: 587 - DNA, 83 bp, Artificial Sequence
  smMIP
  misc_feature (23)..(30): n is a, c, g, or t
gcatcacaggggaggaggtggannnnnnnncttcagcttcccgatatccgacggtagtgttgtggaagtggagtccttcctgg

SEQ ID NO: 588 - DNA, 83 bp, Artificial Sequence
  smMIP
  misc_feature (19)..(26): n is a, c, g, or t
tggcaaagaattcaaaccnnnnnnnncttcagcttcccgatatccgacggtagtgtgcccgtagctccatattggacatcccc

SEQ ID NO: 589 - DNA, 83 bp, Artificial Sequence
  smMIP
  misc_feature (22)..(29): n is a, c, g, or t
cagataacaccaaaccaaaccnnnnnnnncttcagcttcccgatatccgacggtagtgttctatgcttgcgtaaccagcagcc

SEQ ID NO: 590 - DNA, 83 bp, Artificial Sequence
  smMIP
  misc_feature (24)..(31): n is a, c, g, or t
catccctctgcgcagacaggtaannnnnnnncttcagcttcccgatatccgacggtagtgttcatctattgcacaggggcctt

SEQ ID NO: 591 - DNA, 83 bp, Artificial Sequence
  smMIP
  misc_feature (25)..(32): n is a, c, g, or t
tgtgacaagccgaggcggtgagccnnnnnnnncttcagcttcccgatatccgacggtagtgttccaacatcaccatgcagatt

SEQ ID NO: 592 - DNA, 83 bp, Artificial Sequence
  smMIP
  misc_feature (25)..(32): n is a, c, g, or t
tctctcaccaggaaagactgatacnnnnnnnncttcagcttcccgatatccgacggtagtgttccaacatcaccatgcagatt

SEQ ID NO: 593 - DNA, 78 bp, Artificial Sequence
  smMIP
  misc_feature (25)..(32): n is a, c, g, or t
gaggcggtgagccgggcaggaggannnnnnnncttcagcttcccgatatccgacggtagtgtagagcggagaaagcat

SEQ ID NO: 594 - DNA, 82 bp, Artificial Sequence
  smMIP
  misc_feature (22)..(29): n is a, c, g, or t
cctgtgggccttgctcagagcnnnnnnnncttcagcttcccgatatccgacggtagtgtagtccaacatcaccatgcagatt

SEQ ID NO: 595 - DNA, 83 bp, Artificial Sequence
  smMIP
  misc_feature (23)..(30): n is a, c, g, or t
ccacgctgccgccaccacaccannnnnnnncttcagcttcccgatatccgacggtagtgttccgcagacgtgtaaatgttcct

SEQ ID NO: 596 - DNA, 82 bp, Artificial Sequence
  smMIP
  misc_feature (29)..(36): n is a, c, g, or t
gttcgaggaaagggaaaggggcaaaaacnnnnnnnncttcagcttcccgatatccgacggtagtgtccatgcagattatgcg

SEQ ID NO: 597 - DNA, 79 bp, Artificial Sequence
  smMIP
  misc_feature (24)..(31): n is a, c, g, or t
ggcgtgagccctcccccttgggannnnnnnncttcagcttcccgatatccgacggtagtgtagcaagagctccagagag

SEQ ID NO: 598 - DNA, 81 bp, Artificial Sequence
  smMIP
  misc_feature (27)..(34): n is a, c, g, or t
cgaagtggtgaagttcatggatgtctnnnnnnnncttcagcttcccgatatccgacggtagtgtcctccgaaaccatgaac

SEQ ID NO: 599 - DNA, 83 bp, Artificial Sequence
  smMIP
  misc_feature (25)..(32): n is a, c, g, or t
cgttttaatttatttttgcttgccnnnnnnnncttcagcttcccgatatccgacggtagtgtgttaggtggaccggtcagcgg

SEQ ID NO: 600 - DNA, 83 bp, Artificial Sequence
  smMIP
  misc_feature (24)..(31): n is a, c, g, or t
cactgtggattttggaaaccagcnnnnnnnncttcagcttcccgatatccgacggtagtgtccctcttcttttttcttaaaca

SEQ ID NO: 601 - DNA, 80 bp, Artificial Sequence
  smMIP
  misc_feature (26)..(33): n is a, c, g, or t
ggcgctcggaagccgggctcatggannnnnnnncttcagcttcccgatatccgacggtagtgtgcgcgggggaagccgag

SEQ ID NO: 602 - DNA, 80 bp, Artificial Sequence
  smMIP
  misc_feature (27)..(34): n is a, c, g, or t
gcctggagtgtgtgcccactgaggagnnnnnnnncttcagcttcccgatatccgacggtagtgtagctactgccatccaa

SEQ ID NO: 603 - DNA, 83 bp, Artificial Sequence
  smMIP
  misc_feature (30)..(37): n is a, c, g, or t
cctacagcacaacaaatgtgaatgcagacnnnnnnnncttcagcttcccgatatccgacggtagtgtgatgcgggggctgctg

SEQ ID NO: 604 - DNA, 82 bp, Artificial Sequence
  smMIP
  misc_feature (24)..(31): n is a, c, g, or t
ctgtgggccttgctcagagcggannnnnnnncttcagcttcccgatatccgacggtagtgtccaacatcaccatgcagatta

SEQ ID NO: 605 - DNA, 78 bp, Artificial Sequence
  smMIP
  misc_feature (21)..(28): n is a, c, g, or t
gccagagctgccaggctcggnnnnnnnncttcagcttcccgatatccgacggtagtgtcggaagaggcgcgggctagg

SEQ ID NO: 606 - DNA, 82 bp, Artificial Sequence
  smMIP
  misc_feature (23)..(30): n is a, c, g, or t
caccagccgagtgtctctgaggnnnnnnnncttcagcttcccgatatccgacggtagtgtatccatttccacacgctggtct

SEQ ID NO: 607 - DNA, 83 bp, Artificial Sequence
  smMIP
  misc_feature (22)..(29): n is a, c, g, or t
gtggggccagttaaaagctccnnnnnnnncttcagcttcccgatatccgacggtagtgtggttcttctttgcggtccagttgg

SEQ ID NO: 608 - DNA, 83 bp, Artificial Sequence
  smMIP
  misc_feature (20)..(27): n is a, c, g, or t
ttctcacccagtcagcctcnnnnnnnncttcagcttcccgatatccgacggtagtgttgacatccccactggtattccagttc

SEQ ID NO: 609 - DNA, 79 bp, Artificial Sequence
  smMIP
  misc_feature (25)..(32): n is a, c, g, or t
gcaactgtggatggacactgggccnnnnnnnncttcagcttcccgatatccgacggtagtgtggtgttcctgatgtggg

SEQ ID NO: 610 - DNA, 83 bp, Artificial Sequence
  smMIP
  misc_feature (28)..(35): n is a, c, g, or t
agtcggccctggagtgccaccccgagannnnnnnncttcagcttcccgatatccgacggtagtgtagcaagagactagcccca

SEQ ID NO: 611 - DNA, 83 bp, Artificial Sequence
  smMIP
  misc_feature (20)..(27): n is a, c, g, or t
tggcggcggcggcggcggcnnnnnnnncttcagcttcccgatatccgacggtagtgtagcctgcatggcgcgggtgcagcggg

SEQ ID NO: 612 - DNA, 83 bp, Artificial Sequence
  smMIP
  misc_feature (24)..(31): n is a, c, g, or t
gcttgtacacgtggtcaagtgggnnnnnnnncttcagcttcccgatatccgacggtagtgtgtcagcccatctttctgaatgt

SEQ ID NO: 613 - DNA, 83 bp, Artificial Sequence
  smMIP
  misc_feature (26)..(33): n is a, c, g, or t
gctcatggtgtttgccatgggctggnnnnnnnncttcagcttcccgatatccgacggtagtgttctagcctcaatgaactggg

SEQ ID NO: 614 - DNA, 83 bp, Artificial Sequence
  smMIP
  misc_feature (29)..(36): n is a, c, g, or t
catggtgagcgtggactttccggaaatgnnnnnnnncttcagcttcccgatatccgacggtagtgtaaaagaaaaaatcccac

SEQ ID NO: 615 - DNA, 83 bp, Artificial Sequence
  smMIP
  misc_feature (19)..(26): n is a, c, g, or t
ccacacccagtgaagcatnnnnnnnncttcagcttcccgatatccgacggtagtgtgctgcatcagttcacttttgacctgct

SEQ ID NO: 616 - DNA, 81 bp, Artificial Sequence
  smMIP
  misc_feature (25)..(32): n is a, c, g, or t
gcatctcaaaatgaccagaccctgnnnnnnnncttcagcttcccgatatccgacggtagtgtgtgcgccagcagaaatgat

SEQ ID NO: 617 - DNA, 83 bp, Artificial Sequence
  smMIP
  misc_feature (25)..(32): n is a, c, g, or t
gcagagatcatctctgtgcaagtgnnnnnnnncttcagcttcccgatatccgacggtagtgtagagacagcttgtacacgtgg

SEQ ID NO: 618 - DNA, 83 bp, Artificial Sequence
  smMIP
  misc_feature (21)..(28): n is a, c, g, or t
ccccaaattctcaccagtccnnnnnnnncttcagcttcccgatatccgacggtagtgtccaacttgatttgctgtttgtctcc

SEQ ID NO: 619 - DNA, 83 bp, Artificial Sequence
  smMIP
  misc_feature (30)..(37): n is a, c, g, or t
gacatgtgaatatcctactcttcatgggcnnnnnnnncttcagcttcccgatatccgacggtagtgtggaacagtctacaagg

SEQ ID NO: 620 - DNA, 83 bp, Artificial Sequence
  smMIP
  misc_feature (30)..(37): n is a, c, g, or t
gctacagtgaaatctcgatggagtgggtcnnnnnnnncttcagcttcccgatatccgacggtagtgtacgacagactgcacag

SEQ ID NO: 621 - DNA, 83 bp, Artificial Sequence
  smMIP
  misc_feature (30)..(37): n is a, c, g, or t
catacagctttcagtcagatgtatatgcannnnnnnncttcagcttcccgatatccgacggtagtgtataggtgattttggtc

SEQ ID NO: 622 - DNA, 83 bp, Artificial Sequence
  smMIP
  misc_feature (24)..(31): n is a, c, g, or t
caaacatcaacaacagggaccagnnnnnnnncttcagcttcccgatatccgacggtagtgtggatccattttgtggatggcac

SEQ ID NO: 623 - DNA, 83 bp, Artificial Sequence
  smMIP
  misc_feature (30)..(37): n is a, c, g, or t
cggacatggtctgggacttctggagcctannnnnnnncttcagcttcccgatatccgacggtagtgtgaagatggtaactggg

SEQ ID NO: 624 - DNA, 83 bp, Artificial Sequence
  smMIP
  misc_feature (19)..(26): n is a, c, g, or t
ccagggcatcaaaaacctnnnnnnnncttcagcttcccgatatccgacggtagtgtggtttctttcttgttcagtgatcgggg

SEQ ID NO: 625 - DNA, 82 bp, Artificial Sequence
  smMIP
  misc_feature (28)..(35): n is a, c, g, or t
caccaaggtttggcctcacaaggactannnnnnnncttcagcttcccgatatccgacggtagtgttgactatggcatccggg

SEQ ID NO: 626 - DNA, 83 bp, Artificial Sequence
  smMIP
  misc_feature (29)..(36): n is a, c, g, or t
cctgaaggatgcacaaattttcatccagnnnnnnnncttcagcttcccgatatccgacggtagtgttctggagaagtgcggag

SEQ ID NO: 627 - DNA, 83 bp, Artificial Sequence
  smMIP
  misc_feature (30)..(37): n is a, c, g, or t
gcggcaagggagaaggcaaatctgtgaggnnnnnnnncttcagcttcccgatatccgacggtagtgtcaagaacttcactgag

SEQ ID NO: 628 - DNA, 81 bp, Artificial Sequence
  smMIP
  misc_feature (28)..(35): n is a, c, g, or t
gagggcccggctgttgaaggaccagctnnnnnnnncttcagcttcccgatatccgacggtagtgtcccagtagaaaaacaa

SEQ ID NO: 629 - DNA, 83 bp, Artificial Sequence
  smMIP
  misc_feature (25)..(32): n is a, c, g, or t
tggttgtggatccagtcacctctgnnnnnnnncttcagcttcccgatatccgacggtagtgtagatcacagatgtgaaattgc

SEQ ID NO: 630 - DNA, 83 bp, Artificial Sequence
  smMIP
  misc_feature (29)..(36): n is a, c, g, or t
gcacttttaggagattagatcctgaggannnnnnnncttcagcttcccgatatccgacggtagtgtaagcagtgaccatcaag

SEQ ID NO: 631 - DNA, 83 bp, Artificial Sequence
  smMIP
  misc_feature (29)..(36): n is a, c, g, or t
ggcatccaagatacaaactcaaagaagcnnnnnnnncttcagcttcccgatatccgacggtagtgtcacatcctccaaatgaa

SEQ ID NO: 632 - DNA, 83 bp, Artificial Sequence
  smMIP
  misc_feature (27)..(34): n is a, c, g, or t
cttctgatcttcaagcagggattctcnnnnnnnncttcagcttcccgatatccgacggtagtgtctgacattcatcttccgtt

SEQ ID NO: 633 - DNA, 82 bp, Artificial Sequence
  smMIP
  misc_feature (28)..(35): n is a, c, g, or t
gcaaagcaatgcacgtggcccagcctgnnnnnnnncttcagcttcccgatatccgacggtagtgtaacaccgctcccataaa

SEQ ID NO: 634 - DNA, 83 bp, Artificial Sequence
  smMIP
  misc_feature (27)..(34): n is a, c, g, or t
cttcctagatgattccatctgcacggnnnnnnnncttcagcttcccgatatccgacggtagtgtgctttgtgtgtgagtatgc

SEQ ID NO: 635 - DNA, 83 bp, Artificial Sequence
  smMIP
  misc_feature (26)..(33): n is a, c, g, or t
ttgatccagaaccgtgcccagattcnnnnnnnncttcagcttcccgatatccgacggtagtgttcaagtgaacctcactatcc

SEQ ID NO: 636 - DNA, 82 bp, Artificial Sequence
  smMIP
  misc_feature (19)..(26): n is a, c, g, or t
cccccaacagagccagaannnnnnnncttcagcttcccgatatccgacggtagtgtgacttcctcctctggatccttgcagc

SEQ ID NO: 637 - DNA, 81 bp, Artificial Sequence
  smMIP
  misc_feature (21)..(28): n is a, c, g, or t
cccagctgctcaactcgctcnnnnnnnncttcagcttcccgatatccgacggtagtgtttgcacctgcagccccgcgctct

SEQ ID NO: 638 - DNA, 83 bp, Artificial Sequence
  smMIP
  misc_feature (22)..(29): n is a, c, g, or t
gatccccttgatggatcttccnnnnnnnncttcagcttcccgatatccgacggtagtgtgtcctctccaacgacctggttatg

SEQ ID NO: 639 - DNA, 83 bp, Artificial Sequence
  smMIP
  misc_feature (24)..(31): n is a, c, g, or t
gtccttgccatggactgtggggtnnnnnnnncttcagcttcccgatatccgacggtagtgtcgttggaaccatttttggcatc

SEQ ID NO: 640 - DNA, 83 bp, Artificial Sequence
  smMIP
  misc_feature (27)..(34): n is a, c, g, or t
gctccttatggggcccggtatgtgggnnnnnnnncttcagcttcccgatatccgacggtagtgtggacaaggatgtgaagata

SEQ ID NO: 641 - DNA, 82 bp, Artificial Sequence
  smMIP
  misc_feature (29)..(36): n is a, c, g, or t
ccactgggaaggaggccgtgttagacgtnnnnnnnncttcagcttcccgatatccgacggtagtgttctggtctacggaggg

SEQ ID NO: 642 - DNA, 82 bp, Artificial Sequence
  smMIP
  misc_feature (22)..(29): n is a, c, g, or t
ccacctcctccaggatatgaannnnnnnncttcagcttcccgatatccgacggtagtgttttggcctggattctgttgagct

SEQ ID NO: 643 - DNA, 83 bp, Artificial Sequence
  smMIP
  misc_feature (26)..(33): n is a, c, g, or t
cctctcacaccaggttacccagcaannnnnnnncttcagcttcccgatatccgacggtagtgttcattctctactccgaccct

SEQ ID NO: 644 - DNA, 83 bp, Artificial Sequence
  smMIP
  misc_feature (30)..(37): n is a, c, g, or t
gtggagcagctgttgttcatgaaattgtgnnnnnnnncttcagcttcccgatatccgacggtagtgtaatgaagtgacaagaa

SEQ ID NO: 645 - DNA, 83 bp, Artificial Sequence
  smMIP
  misc_feature (28)..(35): n is a, c, g, or t
gggatctggaaatgattttgaggtgttnnnnnnnncttcagcttcccgatatccgacggtagtgtacacaacctaacaaaaga

SEQ ID NO: 646 - DNA, 83 bp, Artificial Sequence
  smMIP
  misc_feature (29)..(36): n is a, c, g, or t
gttcagtgagagactccaggactttgacnnnnnnnncttcagcttcccgatatccgacggtagtgtagaaagtatgctgacaa

SEQ ID NO: 647 - DNA, 83 bp, Artificial Sequence
  smMIP
  misc_feature (30)..(37): n is a, c, g, or t
ggttctaaaacgaaagtatttgggtagtcnnnnnnnncttcagcttcccgatatccgacggtagtgtcaggtgaagatttggt

SEQ ID NO: 648 - DNA, 83 bp, Artificial Sequence
  smMIP
  misc_feature (30)..(37): n is a, c, g, or t
tattaaccaccaggtggtgccaacactggnnnnnnnncttcagcttcccgatatccgacggtagtgtacaaaatactaacaca

SEQ ID NO: 649 - DNA, 83 bp, Artificial Sequence
  smMIP
  misc_feature (30)..(37): n is a, c, g, or t
ggatatacagtggaagtgcagtttgatggnnnnnnnncttcagcttcccgatatccgacggtagtgttgaactgcaactaacg

SEQ ID NO: 650 - DNA, 83 bp, Artificial Sequence
  smMIP
  misc_feature (30)..(37): n is a, c, g, or t
gtaaaaataaagtatgggaagttcatgcgnnnnnnnncttcagcttcccgatatccgacggtagtgtatttgtgaagaagcat

SEQ ID NO: 651 - DNA, 83 bp, Artificial Sequence
  smMIP
  misc_feature (21)..(28): n is a, c, g, or t
agccagacaccggaaaccccnnnnnnnncttcagcttcccgatatccgacggtagtgtagcagcaacgaagtatcctctcctg

SEQ ID NO: 652 - DNA, 83 bp, Artificial Sequence
  smMIP
  misc_feature (30)..(37): n is a, c, g, or t
gcattgtacattgtatactgcagtgtcgtnnnnnnnncttcagcttcccgatatccgacggtagtgttcctcactgcatttaa

SEQ ID NO: 653 - DNA, 82 bp, Artificial Sequence
  smMIP
  misc_feature (27)..(34): n is a, c, g, or t
gttactgcgacgtgaggtatatgactnnnnnnnncttcagcttcccgatatccgacggtagtgtaccaaaagagaactgcaa

SEQ ID NO: 654 - DNA, 83 bp, Artificial Sequence
  smMIP
  misc_feature (30)..(37): n is a, c, g, or t
gttttattctaaaattagtgagtatagacnnnnnnnncttcagcttcccgatatccgacggtagtgttagaatgtgtgtactg

SEQ ID NO: 655 - DNA, 83 bp, Artificial Sequence
  smMIP
  misc_feature (30)..(37): n is a, c, g, or t
cgttgtgtgatttgttaattaggtgtattnnnnnnnncttcagcttcccgatatccgacggtagtgtagagatgggaatccat

SEQ ID NO: 656 - DNA, 79 bp, Artificial Sequence
  smMIP
  misc_feature (23)..(30): n is a, c, g, or t
gtggaccggtcgatgtatgtctnnnnnnnncttcagcttcccgatatccgacggtagtgtgaacagcaatacaacaaac

SEQ ID NO: 657 - DNA, 82 bp, Artificial Sequence
  smMIP
  misc_feature (29)..(36): n is a, c, g, or t
cgtagacattcgtactttggaagacctgnnnnnnnncttcagcttcccgatatccgacggtagtgtgaggaggaggatgaaa

SEQ ID NO: 658 - DNA, 82 bp, Artificial Sequence
  smMIP
  misc_feature (28)..(35): n is a, c, g, or t
gcggggtggggggggagagagagttttnnnnnnnncttcagcttcccgatatccgacggtagtgtacagccttacgcccaca

SEQ ID NO: 659 - DNA, 80 bp, Artificial Sequence
  smMIP
  misc_feature (27)..(34): n is a, c, g, or t
cattactcggggggccatcaggattgnnnnnnnncttcagcttcccgatatccgacggtagtgtagagcctcggagacct

SEQ ID NO: 660 - DNA, 82 bp, Artificial Sequence
  smMIP
  misc_feature (26)..(33): n is a, c, g, or t
gctcagatgctccaaggatgcaccannnnnnnncttcagcttcccgatatccgacggtagtgtaggagtgcccctcgggctt

SEQ ID NO: 661 - DNA, 81 bp, Artificial Sequence
  smMIP
  misc_feature (27)..(34): n is a, c, g, or t
tctctctctgggaatgggtcgtggacnnnnnnnncttcagcttcccgatatccgacggtagtgtaaaatacggatcacaag

SEQ ID NO: 662 - DNA, 82 bp, Artificial Sequence
  smMIP
  misc_feature (29)..(36): n is a, c, g, or t
ggtatgacgcgagatatctatgagacagnnnnnnnncttcagcttcccgatatccgacggtagtgtagatggccggagagat

SEQ ID NO: 663 - DNA, 83 bp, Artificial Sequence
  smMIP
  misc_feature (24)..(31): n is a, c, g, or t
gcccaataatcagagtggcagtgnnnnnnnncttcagcttcccgatatccgacggtagtgtctgtgggtttgcctagtgtttc

SEQ ID NO: 664 - DNA, 83 bp, Artificial Sequence
  smMIP
  misc_feature (28)..(35): n is a, c, g, or t
cctgtgcagcatccagtgggctgatgannnnnnnncttcagcttcccgatatccgacggtagtgtcgaagcatcagcataaga

SEQ ID NO: 665 - DNA, 81 bp, Artificial Sequence
  smMIP
  misc_feature (25)..(32): n is a, c, g, or t
gcaggagagcgtgtctttgtggtgnnnnnnnncttcagcttcccgatatccgacggtagtgtggcaaatgtgtcagctttg

SEQ ID NO: 666 - DNA, 83 bp, Artificial Sequence
  smMIP
  misc_feature (24)..(31): n is a, c, g, or t
gtgactttggcttggcccgggatnnnnnnnncttcagcttcccgatatccgacggtagtgtgagcatctcatctgttacagct

SEQ ID NO: 667 - DNA, 83 bp, Artificial Sequence
  smMIP
  misc_feature (29)..(36): n is a, c, g, or t
gcagggagtctgtggcatctgaaggctcnnnnnnnncttcagcttcccgatatccgacggtagtgtaaaagtaatcccagatg

SEQ ID NO: 668 - DNA, 83 bp, Artificial Sequence
  smMIP
  misc_feature (28)..(35): n is a, c, g, or t
cagtgtgtggacctccatgttatttccnnnnnnnncttcagcttcccgatatccgacggtagtgtgagctcacggatgctgtg

SEQ ID NO: 669 - DNA, 83 bp, Artificial Sequence
  smMIP
  misc_feature (30)..(37): n is a, c, g, or t
cctgaagaatcgattcctcaggccaggtgnnnnnnnncttcagcttcccgatatccgacggtagtgtactgcatcaggaacaa

SEQ ID NO: 670 - DNA, 83 bp, Artificial Sequence
  smMIP
  misc_feature (28)..(35): n is a, c, g, or t
gcttcaaggtatcacgtcatggggcagnnnnnnnncttcagcttcccgatatccgacggtagtgttgacgtgtgtgcgcaagt

SEQ ID NO: 671 - DNA, 81 bp, Artificial Sequence
  smMIP
  misc_feature (28)..(35): n is a, c, g, or t
gtggatcaaggacaccatcgtggccaannnnnnnncttcagcttcccgatatccgacggtagtgtgggtgattctgggggc

SEQ ID NO: 672 - DNA, 83 bp, Artificial Sequence
  smMIP
  misc_feature (22)..(29): n is a, c, g, or t
ctcaagcctccccagttctacnnnnnnnncttcagcttcccgatatccgacggtagtgtccttccctgtacaccaaggtggtg

SEQ ID NO: 673 - DNA, 82 bp, Artificial Sequence
  smMIP
  misc_feature (29)..(36): n is a, c, g, or t
gatccaacaatagaggattcctacaggannnnnnnncttcagcttcccgatatccgacggtagtgtaggtgcgggagagagg

SEQ ID NO: 674 - DNA, 80 bp, Artificial Sequence
  smMIP
  misc_feature (24)..(31): n is a, c, g, or t
gcaggtcaagaggagtacagtgcnnnnnnnncttcagcttcccgatatccgacggtagtgtgagtgccttgacgatacag

SEQ ID NO: 675 - DNA, 83 bp, Artificial Sequence
  smMIP
  misc_feature (28)..(35): n is a, c, g, or t
catttgaagatattcaccattatagagnnnnnnnncttcagcttcccgatatccgacggtagtgtgagaaacctgtctcttgg

SEQ ID NO: 676 - DNA, 83 bp, Artificial Sequence
  smMIP
  misc_feature (22)..(29): n is a, c, g, or t
gtgatttgccttctagaacagnnnnnnnncttcagcttcccgatatccgacggtagtgtgggagggctttctttgtgtatttg

SEQ ID NO: 677 - DNA, 83 bp, Artificial Sequence
  smMIP
  misc_feature (30)..(37): n is a, c, g, or t
gtggaggatgctttttatacattggtgagnnnnnnnncttcagcttcccgatatccgacggtagtgtggtcctagtaggaaat

SEQ ID NO: 678 - DNA, 83 bp, Artificial Sequence
  smMIP
  misc_feature (29)..(36): n is a, c, g, or t
gcattataatgtaatctgggtgttgatgnnnnnnnncttcagcttcccgatatccgacggtagtgtagcaaagacaagacaga

SEQ ID NO: 679 - DNA, 83 bp, Artificial Sequence
  smMIP
  misc_feature (30)..(37): n is a, c, g, or t
gcaaagatggtaaaaagaagaaaaagaagnnnnnnnncttcagcttcccgatatccgacggtagtgtgcaaagaagaaaagac

SEQ ID NO: 680 - DNA, 78 bp, Artificial Sequence
  smMIP
  misc_feature (22)..(29): n is a, c, g, or t
caaagagagcctgcgggcagannnnnnnncttcagcttcccgatatccgacggtagtgtggactgccgcttccgtgtc

SEQ ID NO: 681 - DNA, 82 bp, Artificial Sequence
  smMIP
  misc_feature (23)..(30): n is a, c, g, or t
ggacactgctcttggcccctctnnnnnnnncttcagcttcccgatatccgacggtagtgttgccctgtgtccctgagcagac

SEQ ID NO: 682 - DNA, 81 bp, Artificial Sequence
  smMIP
  misc_feature (19)..(26): n is a, c, g, or t
taccgcatgagccccagcnnnnnnnncttcagcttcccgatatccgacggtagtgtttcttagactccccagacaggccct

SEQ ID NO: 683 - DNA, 82 bp, Artificial Sequence
  smMIP
  misc_feature (27)..(34): n is a, c, g, or t
ggaggacccctcagccgtgcctgtgtnnnnnnnncttcagcttcccgatatccgacggtagtgttggtggttggtgtcgtgg

SEQ ID NO: 684 - DNA, 79 bp, Artificial Sequence
  smMIP
  misc_feature (22)..(29): n is a, c, g, or t
ccagccggccagttccaaaccnnnnnnnncttcagcttcccgatatccgacggtagtgtggcacctacctctgtggggc

SEQ ID NO: 685 - DNA, 83 bp, Artificial Sequence
  smMIP
  misc_feature (23)..(30): n is a, c, g, or t
tctggcccctcctcagcatcttnnnnnnnncttcagcttcccgatatccgacggtagtgtctgtgggttgattccacaccccc

SEQ ID NO: 686 - DNA, 83 bp, Artificial Sequence
  smMIP
  misc_feature (19)..(26): n is a, c, g, or t
cccctgcaccagccccctnnnnnnnncttcagcttcccgatatccgacggtagtgttggatgatttgatgctgtccccggacg

SEQ ID NO: 687 - DNA, 83 bp, Artificial Sequence
  smMIP
  misc_feature (23)..(30): n is a, c, g, or t
gcctgaggttggctctgactgtnnnnnnnncttcagcttcccgatatccgacggtagtgtgagcgctgctcagatagcgatgg

SEQ ID NO: 688 - DNA, 83 bp, Artificial Sequence
  smMIP
  misc_feature (25)..(32): n is a, c, g, or t
cggcgcacagaggaagagaatctcnnnnnnnncttcagcttcccgatatccgacggtagtgtagttcctgcatgggcggcatg

SEQ ID NO: 689 - DNA, 80 bp, Artificial Sequence
  smMIP
  misc_feature (20)..(27): n is a, c, g, or t
tcccacccccatctctcccnnnnnnnncttcagcttcccgatatccgacggtagtgtagcagggctcactccagccacct

SEQ ID NO: 690 - DNA, 83 bp, Artificial Sequence
  smMIP
  misc_feature (25)..(32): n is a, c, g, or t
gcttcctccacgaatttgaaagacnnnnnnnncttcagcttcccgatatccgacggtagtgttctctccctttcttacctccc

SEQ ID NO: 691 - DNA, 82 bp, Artificial Sequence
  smMIP
  misc_feature (29)..(36): n is a, c, g, or t
gcaacatggcaagacggtggtgggccaannnnnnnncttcagcttcccgatatccgacggtagtgtaaccaagaatgcatct

SEQ ID NO: 692 - DNA, 82 bp, Artificial Sequence
  smMIP
  misc_feature (29)..(36): n is a, c, g, or t
gttcttgatcctgatgagggcatccgttnnnnnnnncttcagcttcccgatatccgacggtagtgtaaggagcaggccagaa

SEQ ID NO: 693 - DNA, 81 bp, Artificial Sequence
  smMIP
  misc_feature (27)..(34): n is a, c, g, or t
gcctgagggcttattttggctgctggnnnnnnnncttcagcttcccgatatccgacggtagtgtggcatgaagggattggt

SEQ ID NO: 694 - DNA, 81 bp, Artificial Sequence
  smMIP
  misc_feature (27)..(34): n is a, c, g, or t
cccatgtggtcaccatgctggacaacnnnnnnnncttcagcttcccgatatccgacggtagtgtggctaagggtggggaag

SEQ ID NO: 695 - DNA, 79 bp, Artificial Sequence
  smMIP
  misc_feature (24)..(31): n is a, c, g, or t
gcccgagcatatgcacagggtatnnnnnnnncttcagcttcccgatatccgacggtagtgtaagagtgggcaaagaggg

SEQ ID NO: 696 - DNA, 82 bp, Artificial Sequence
  smMIP
  misc_feature (23)..(30): n is a, c, g, or t
gctaccttgtgttgcagcaaagnnnnnnnncttcagcttcccgatatccgacggtagtgtgtctcagctcagtgcagctgtt

SEQ ID NO: 697 - DNA, 83 bp, Artificial Sequence
  smMIP
  misc_feature (29)..(36): n is a, c, g, or t
ggactggtctcacaatttcaccaacatgnnnnnnnncttcagcttcccgatatccgacggtagtgtgtactgggagttgattt

SEQ ID NO: 698 - DNA, 81 bp, Artificial Sequence
  smMIP
  misc_feature (28)..(35): n is a, c, g, or t
gtgaccatgagggtggcaatgtaagtgnnnnnnnncttcagcttcccgatatccgacggtagtgtagagaaggcagcggta

SEQ ID NO: 699 - DNA, 83 bp, Artificial Sequence
  smMIP
  misc_feature (30)..(37): n is a, c, g, or t
gcctctccatggactggcaaatcaggaagnnnnnnnncttcagcttcccgatatccgacggtagtgttacctcaccatccaca

SEQ ID NO: 700 - DNA, 83 bp, Artificial Sequence
  smMIP
  misc_feature (30)..(37): n is a, c, g, or t
gttacgagactacatctggaacacactcannnnnnnncttcagcttcccgatatccgacggtagtgtctgtcctttgcagcag

SEQ ID NO: 701 - DNA, 83 bp, Artificial Sequence
  smMIP
  misc_feature (28)..(35): n is a, c, g, or t
gcgatatacctgtcagcgagagtttgcnnnnnnnncttcagcttcccgatatccgacggtagtgtagctgcagaaggaagttg

SEQ ID NO: 702 - DNA, 83 bp, Artificial Sequence
  smMIP
  misc_feature (23)..(30): n is a, c, g, or t
gtgcccaatgtcctcttagagcnnnnnnnncttcagcttcccgatatccgacggtagtgtgttgttccaggctatggccatgc

SEQ ID NO: 703 - DNA, 83 bp, Artificial Sequence
  smMIP
  misc_feature (29)..(36): n is a, c, g, or t
gatgaattactacacggtcctgtttgggnnnnnnnncttcagcttcccgatatccgacggtagtgtgttggttgctcagctgt

SEQ ID NO: 704 - DNA, 82 bp, Artificial Sequence
  smMIP
  misc_feature (27)..(34): n is a, c, g, or t
gaaaggcccaagtccatgagcacagannnnnnnncttcagcttcccgatatccgacggtagtgtgtggggtgctgctccagt

SEQ ID NO: 705 - DNA, 83 bp, Artificial Sequence
  smMIP
  misc_feature (30)..(37): n is a, c, g, or t
gagactgggtgaaagtgactaccagaaagnnnnnnnncttcagcttcccgatatccgacggtagtgtgcattgggtgtactgg

SEQ ID NO: 706 - DNA, 83 bp, Artificial Sequence
  smMIP
  misc_feature (27)..(34): n is a, c, g, or t
gtccccgtctttgacgagatcatcctnnnnnnnncttcagcttcccgatatccgacggtagtgtgctgtagcaaggtgctgct

SEQ ID NO: 707 - DNA, 78 bp, Artificial Sequence
  smMIP
  misc_feature (23)..(30): n is a, c, g, or t
gctgagccggtatgtggaggaannnnnnnncttcagcttcccgatatccgacggtagtgtaggcatggtgggtggcag

SEQ ID NO: 708 - DNA, 83 bp, Artificial Sequence
  smMIP
  misc_feature (22)..(29): n is a, c, g, or t
gctggaggcctgcggtttcttnnnnnnnncttcagcttcccgatatccgacggtagtgtaattctggtttgccaggcgggctg

SEQ ID NO: 709 - DNA, 83 bp, Artificial Sequence
  smMIP
  misc_feature (30)..(37): n is a, c, g, or t
ggaaggacaacacgggctatgacctgaagnnnnnnnncttcagcttcccgatatccgacggtagtgtaaacgtggcaaccaac

SEQ ID NO: 710 - DNA, 83 bp, Artificial Sequence
  smMIP
  misc_feature (22)..(29): n is a, c, g, or t
gctgtgaacgtggctttcctcnnnnnnnncttcagcttcccgatatccgacggtagtgttgtcctggactgcctgacctccct

SEQ ID NO: 711 - DNA, 83 bp, Artificial Sequence
  smMIP
  misc_feature (27)..(34): n is a, c, g, or t
gcattcgagttcatggatgctgtgtgnnnnnnnncttcagcttcccgatatccgacggtagtgtcggtgtccatcttgtgtcc

SEQ ID NO: 712 - DNA, 83 bp, Artificial Sequence
  smMIP
  misc_feature (21)..(28): n is a, c, g, or t
gctccaacgcaggccatgacnnnnnnnncttcagcttcccgatatccgacggtagtgtggggatgctgggtgagatcctgtct

SEQ ID NO: 713 - DNA, 82 bp, Artificial Sequence
  smMIP
  misc_feature (24)..(31): n is a, c, g, or t
gccaccgaccagaggaaagtcaannnnnnnncttcagcttcccgatatccgacggtagtgtcggtgcaagagagtccgtttt

SEQ ID NO: 714 - DNA, 83 bp, Artificial Sequence
  smMIP
  misc_feature (23)..(30): n is a, c, g, or t
tacaagtacgacctctccctccnnnnnnnncttcagcttcccgatatccgacggtagtgtttcctggagcacgcgctgggctc

SEQ ID NO: 715 - DNA, 82 bp, Artificial Sequence
  smMIP
  misc_feature (23)..(30): n is a, c, g, or t
gccaagcacgtggtgggctatgnnnnnnnncttcagcttcccgatatccgacggtagtgttgggccctgagggaaaggatca

SEQ ID NO: 716 - DNA, 83 bp, Artificial Sequence
  smMIP
  misc_feature (28)..(35): n is a, c, g, or t
gcacggagtgggcttcaggaagagggannnnnnnncttcagcttcccgatatccgacggtagtgtaccttggagatggtaacc

SEQ ID NO: 717 - DNA, 80 bp, Artificial Sequence
  smMIP
  misc_feature (23)..(30): n is a, c, g, or t
gtattatggcgcccagaccgtgnnnnnnnncttcagcttcccgatatccgacggtagtgtttcggctcccggcttgggtg

SEQ ID NO: 718 - DNA, 81 bp, Artificial Sequence
  smMIP
  misc_feature (27)..(34): n is a, c, g, or t
gaagcgagcggccgctgaagtaaaccnnnnnnnncttcagcttcccgatatccgacggtagtgtggtgaactaaaggtgcc

SEQ ID NO: 719 - DNA, 83 bp, Artificial Sequence
  smMIP
  misc_feature (30)..(37): n is a, c, g, or t
cattttcctctcgtggtatggcagactggnnnnnnnncttcagcttcccgatatccgacggtagtgtaagcttttggcatctt

SEQ ID NO: 720 - DNA, 83 bp, Artificial Sequence
  smMIP
  misc_feature (28)..(35): n is a, c, g, or t
gtgaacttggcagcaagatacctgtgcnnnnnnnncttcagcttcccgatatccgacggtagtgtgaggtagctgaaggtaaa

SEQ ID NO: 721 - DNA, 83 bp, Artificial Sequence
  smMIP
  misc_feature (29)..(36): n is a, c, g, or t
gctgcaatagaagttcatgaagtactgtnnnnnnnncttcagcttcccgatatccgacggtagtgtagcaatagagcaattga

SEQ ID NO: 722 - DNA, 83 bp, Artificial Sequence
  smMIP
  misc_feature (27)..(34): n is a, c, g, or t
cgtactcatactcaggatgctgttccnnnnnnnncttcagcttcccgatatccgacggtagtgtttcccacagcaatgcacat

SEQ ID NO: 723 - DNA, 83 bp, Artificial Sequence
  smMIP
  misc_feature (30)..(37): n is a, c, g, or t
gccaagaatctatgagctcgcagctggagnnnnnnnncttcagcttcccgatatccgacggtagtgtgcacagatcatcaaga

SEQ ID NO: 724 - DNA, 83 bp, Artificial Sequence
  smMIP
  misc_feature (29)..(36): n is a, c, g, or t
gtggctgcacttacaggcttgccttttgnnnnnnnncttcagcttcccgatatccgacggtagtgtaaatatgcaatgacaag

SEQ ID NO: 725 - DNA, 83 bp, Artificial Sequence
  smMIP
  misc_feature (29)..(36): n is a, c, g, or t
gcctgcagtctgatgaagatagcaaatgnnnnnnnncttcagcttcccgatatccgacggtagtgtgaaaaggttgctgcaaa

SEQ ID NO: 726 - DNA, 83 bp, Artificial Sequence
  smMIP
  misc_feature (29)..(36): n is a, c, g, or t
accaggaagcagtatcatgccaggcaagnnnnnnnncttcagcttcccgatatccgacggtagtgtggttgagctcagtggag

SEQ ID NO: 727 - DNA, 80 bp, Artificial Sequence
  smMIP
  misc_feature (27)..(34): n is a, c, g, or t
gttgctgtcactgtcggaggcagcaannnnnnnncttcagcttcccgatatccgacggtagtgtggtcaggtctgggaga

SEQ ID NO: 728 - DNA, 80 bp, Artificial Sequence
  smMIP
  misc_feature (24)..(31): n is a, c, g, or t
gctgctgggggatgcttcagtttnnnnnnnncttcagcttcccgatatccgacggtagtgtgcaatgaccatggttgcag

SEQ ID NO: 729 - DNA, 83 bp, Artificial Sequence
  smMIP
  misc_feature (30)..(37): n is a, c, g, or t
gctgatgaatgagtctctaatgttggtgannnnnnnncttcagcttcccgatatccgacggtagtgtgttttcaagccaatga

SEQ ID NO: 730 - DNA, 82 bp, Artificial Sequence
  smMIP
  misc_feature (29)..(36): n is a, c, g, or t
gcacacaaaaatggatcaaccttaaaggnnnnnnnncttcagcttcccgatatccgacggtagtgttgcgtggtgggaatcc

SEQ ID NO: 731 - DNA, 83 bp, Artificial Sequence
  smMIP
  misc_feature (28)..(35): n is a, c, g, or t
ggacatgctgggtccaaagtgatttacnnnnnnnncttcagcttcccgatatccgacggtagtgttagggtatgacaaggcag

SEQ ID NO: 732 - DNA, 83 bp, Artificial Sequence
  smMIP
  misc_feature (30)..(37): n is a, c, g, or t
ctacgtggaattggatctacatagctatgnnnnnnnncttcagcttcccgatatccgacggtagtgtctgtcaaggtttattg

SEQ ID NO: 733 - DNA, 83 bp, Artificial Sequence
  smMIP
  misc_feature (29)..(36): n is a, c, g, or t
gcataatgttggcgtcaaatgtgccactnnnnnnnncttcagcttcccgatatccgacggtagtgtgattaaagagaaactca

SEQ ID NO: 734 - DNA, 83 bp, Artificial Sequence
  smMIP
  misc_feature (29)..(36): n is a, c, g, or t
attctgggtggcacggtcttcagagaagnnnnnnnncttcagcttcccgatatccgacggtagtgtgcagaagctataaagaa

SEQ ID NO: 735 - DNA, 83 bp, Artificial Sequence
  smMIP
  misc_feature (29)..(36): n is a, c, g, or t
gcttatggggatcaatacagagcaactgnnnnnnnncttcagcttcccgatatccgacggtagtgtaaatcaccaaatggcac

SEQ ID NO: 736 - DNA, 83 bp, Artificial Sequence
  smMIP
  misc_feature (26)..(33): n is a, c, g, or t
gaacccaaaaggtgacatacctggtnnnnnnnncttcagcttcccgatatccgacggtagtgtggcttgtgagtggatgggta

SEQ ID NO: 737 - DNA, 83 bp, Artificial Sequence
  smMIP
  misc_feature (28)..(35): n is a, c, g, or t
gttccttccaaatggctctgtctaaggnnnnnnnncttcagcttcccgatatccgacggtagtgtataacctacacaccaagt

SEQ ID NO: 738 - DNA, 83 bp, Artificial Sequence
  smMIP
  misc_feature (26)..(33): n is a, c, g, or t
gcgttttaaagacatctttcaggagnnnnnnnncttcagcttcccgatatccgacggtagtgtcatggggatgtataatcaag

SEQ ID NO: 739 - DNA, 83 bp, Artificial Sequence
  smMIP
  misc_feature (29)..(36): n is a, c, g, or t
cgacgacatggtggcccaagctatgaaannnnnnnncttcagcttcccgatatccgacggtagtgtcaccaaaaacactattc

SEQ ID NO: 740 - DNA, 83 bp, Artificial Sequence
  smMIP
  misc_feature (26)..(33): n is a, c, g, or t
gtcggactctgtggcccaagggtatnnnnnnnncttcagcttcccgatatccgacggtagtgtcaagtcccagtttgaagctc

SEQ ID NO: 741 - DNA, 83 bp, Artificial Sequence
  smMIP
  misc_feature (26)..(33): n is a, c, g, or t
gcagaggctgcccacgggactgtaannnnnnnncttcagcttcccgatatccgacggtagtgtggaggcttcatctgggcctg

SEQ ID NO: 742 - DNA, 83 bp, Artificial Sequence
  smMIP
  misc_feature (29)..(36): n is a, c, g, or t
gcttccatttttgcctggaccagagggtnnnnnnnncttcagcttcccgatatccgacggtagtgtatgatgaccagcgtgct

SEQ ID NO: 743 - DNA, 83 bp, Artificial Sequence
  smMIP
  misc_feature (30)..(37): n is a, c, g, or t
gaagtctctattgagacaattgaggctggnnnnnnnncttcagcttcccgatatccgacggtagtgtagaaaggacaggagac

SEQ ID NO: 744 - DNA, 83 bp, Artificial Sequence
  smMIP
  misc_feature (20)..(27): n is a, c, g, or t
gcaacgttctgactacttgnnnnnnnncttcagcttcccgatatccgacggtagtgtcagagcaaagcttgataacaataaag

SEQ ID NO: 745 - DNA, 83 bp, Artificial Sequence
  smMIP
  misc_feature (28)..(35): n is a, c, g, or t
gttcatacctgagctaagaaggataatnnnnnnnncttcagcttcccgatatccgacggtagtgtggacttggctgcttgcat

SEQ ID NO: 746 - DNA, 83 bp, Artificial Sequence
  smMIP
  misc_feature (30)..(37): n is a, c, g, or t
acccctgatgaggcccgtgtggaagagttnnnnnnnncttcagcttcccgatatccgacggtagtgtacatccagctaaagta

SEQ ID NO: 747 - DNA, 83 bp, Artificial Sequence
  smMIP
  misc_feature (27)..(34): n is a, c, g, or t
gagcccatcatctgcaaaaacatcccnnnnnnnncttcagcttcccgatatccgacggtagtgtgtgtggctgtcaagtgtgc

SEQ ID NO: 748 - DNA, 83 bp, Artificial Sequence
  smMIP
  misc_feature (23)..(30): n is a, c, g, or t
gcgaccagtacaaggccacagannnnnnnncttcagcttcccgatatccgacggtagtgtaaagtcccaatggaactatccgg

SEQ ID NO: 749 - DNA, 83 bp, Artificial Sequence
  smMIP
  misc_feature (29)..(36): n is a, c, g, or t
gagtgggaagtgtacaacttccccgcagnnnnnnnncttcagcttcccgatatccgacggtagtgtaccaagcccatcaccat

SEQ ID NO: 750 - DNA, 83 bp, Artificial Sequence
  smMIP
  misc_feature (30)..(37): n is a, c, g, or t
gtatgccatccagaagaaatggccgctgtnnnnnnnncttcagcttcccgatatccgacggtagtgtaccccaaaagatggca

SEQ ID NO: 751 - DNA, 83 bp, Artificial Sequence
  smMIP
  misc_feature (26)..(33): n is a, c, g, or t
gcactataagaccgacttcgacaagnnnnnnnncttcagcttcccgatatccgacggtagtgtttttgcgcacagctgcttcc

SEQ ID NO: 752 - DNA, 83 bp, Artificial Sequence
  smMIP
  misc_feature (28)..(35): n is a, c, g, or t
gctttgtgtgggcctgcaagaactatgnnnnnnnncttcagcttcccgatatccgacggtagtgtttcaaggacatcttccag

SEQ ID NO: 753 - DNA, 83 bp, Artificial Sequence
  smMIP
  misc_feature (23)..(30): n is a, c, g, or t
gccctgatgggaagacgattgannnnnnnncttcagcttcccgatatccgacggtagtgttggtggctcaggtcctcaagtct

SEQ ID NO: 754 - DNA, 83 bp, Artificial Sequence
  smMIP
  misc_feature (19)..(26): n is a, c, g, or t
ccaccagcaccaaccccannnnnnnncttcagcttcccgatatccgacggtagtgtatcctggcccagggctttggctccctt

SEQ ID NO: 755 - DNA, 81 bp, Artificial Sequence
  smMIP
  misc_feature (28)..(35): n is a, c, g, or t
gctggagaaggtgtgcgtggagacggtnnnnnnnncttcagcttcccgatatccgacggtagtgtgggagcaccagaaggg

SEQ ID NO: 756 - DNA, 83 bp, Artificial Sequence
  smMIP
  misc_feature (30)..(37): n is a, c, g, or t
gcaatgtgaagctgaacgagcacttcctgnnnnnnnncttcagcttcccgatatccgacggtagtgtggggaagctggatggg

SEQ ID NO: 757 - DNA, 83 bp, Artificial Sequence
  smMIP
  misc_feature (29)..(36): n is a, c, g, or t
gtgactggagcagctggtcaaattgcatnnnnnnnncttcagcttcccgatatccgacggtagtgttgggagaggagcgatct

SEQ ID NO: 758 - DNA, 83 bp, Artificial Sequence
  smMIP
  misc_feature (28)..(35): n is a, c, g, or t
gctgttggatatcacccccatgatgggnnnnnnnncttcagcttcccgatatccgacggtagtgtaggacgataagtctgaac

SEQ ID NO: 759 - DNA, 83 bp, Artificial Sequence
  smMIP
  misc_feature (27)..(34): n is a, c, g, or t
gcaacagataaagaagacgttgccttnnnnnnnncttcagcttcccgatatccgacggtagtgtctgtctttggtaaagatca

SEQ ID NO: 760 - DNA, 83 bp, Artificial Sequence
  smMIP
  misc_feature (30)..(37): n is a, c, g, or t
gcaaatgtgaaaatcttcaaatcccagggnnnnnnnncttcagcttcccgatatccgacggtagtgtccctcctgaaagatgt

SEQ ID NO: 761 - DNA, 83 bp, Artificial Sequence
  smMIP
  misc_feature (30)..(37): n is a, c, g, or t
gccaataccaactgcctgactgcttccaannnnnnnncttcagcttcccgatatccgacggtagtgtgaagggaaggcatgga

SEQ ID NO: 762 - DNA, 83 bp, Artificial Sequence
  smMIP
  misc_feature (29)..(36): n is a, c, g, or t
gatcacaaccgagctaaagctcaaattgnnnnnnnncttcagcttcccgatatccgacggtagtgtaaatacgccaagaagtc

SEQ ID NO: 763 - DNA, 82 bp, Artificial Sequence
  smMIP
  misc_feature (29)..(36): n is a, c, g, or t
gaaaccattcctcgactcagtatccagannnnnnnncttcagcttcccgatatccgacggtagtgtctccatccatccccaa

SEQ ID NO: 764 - DNA, 83 bp, Artificial Sequence
  smMIP
  misc_feature (29)..(36): n is a, c, g, or t
gctctgaaagatgacagctggctcaaggnnnnnnnncttcagcttcccgatatccgacggtagtgtcttggtgtgactgctaa

SEQ ID NO: 765 - DNA, 83 bp, Artificial Sequence
  smMIP
  misc_feature (30)..(37): n is a, c, g, or t
gccatgtctgctgcaaaagccatctgtgannnnnnnncttcagcttcccgatatccgacggtagtgttgcaaggaaaggaagt

SEQ ID NO: 766 - DNA, 83 bp, Artificial Sequence
  smMIP
  misc_feature (30)..(37): n is a, c, g, or t
gcaactcctatggtgttcctgatgatctgnnnnnnnncttcagcttcccgatatccgacggtagtgtcatcaaggctcgaaaa

SEQ ID NO: 767 - DNA, 83 bp, Artificial Sequence
  smMIP
  misc_feature (28)..(35): n is a, c, g, or t
gatttctcacgtgagaagatggatcttnnnnnnnncttcagcttcccgatatccgacggtagtgtgtttgtgtccatgggtgt

SEQ ID NO: 768 - DNA, 83 bp, Artificial Sequence
  smMIP
  misc_feature (30)..(37): n is a, c, g, or t
gcctgactagacaatgatgttactaaatgnnnnnnnncttcagcttcccgatatccgacggtagtgtagaataagacctggaa

SEQ ID NO: 769 - DNA, 83 bp, Artificial Sequence
  smMIP
  misc_feature (30)..(37): n is a, c, g, or t
gctatacttaaattacttgtgaaaaacaannnnnnnncttcagcttcccgatatccgacggtagtgtgaagaaaaagaaagtg

SEQ ID NO: 770 - DNA, 83 bp, Artificial Sequence
  smMIP
  misc_feature (26)..(33): n is a, c, g, or t
gccactttcacttctcctgaagaacnnnnnnnncttcagcttcccgatatccgacggtagtgttcccgctccagccatgctct

SEQ ID NO: 771 - DNA, 83 bp, Artificial Sequence
  smMIP
  misc_feature (20)..(27): n is a, c, g, or t
ccacatcgagaccaaagccnnnnnnnncttcagcttcccgatatccgacggtagtgttaaagtagctgtgctaggggcctctg

SEQ ID NO: 772 - DNA, 83 bp, Artificial Sequence
  smMIP
  misc_feature (26)..(33): n is a, c, g, or t
gtggtagttattccggctggagtccnnnnnnnncttcagcttcccgatatccgacggtagtgtctgaccctctatgatatcgc

SEQ ID NO: 773 - DNA, 83 bp, Artificial Sequence
  smMIP
  misc_feature (22)..(29): n is a, c, g, or t
gctgcctgtgcccagcactgcnnnnnnnncttcagcttcccgatatccgacggtagtgtacctgaacagctgcctgactgcct

SEQ ID NO: 774 - DNA, 83 bp, Artificial Sequence
  smMIP
  misc_feature (30)..(37): n is a, c, g, or t
cattggtggccatgctgggaagaccatcannnnnnnncttcagcttcccgatatccgacggtagtgtttcaacaccaatgcca

SEQ ID NO: 775 - DNA, 83 bp, Artificial Sequence
  smMIP
  misc_feature (21)..(28): n is a, c, g, or t
cagctgacagcactcactggnnnnnnnncttcagcttcccgatatccgacggtagtgttgatctgcgtcattgccaatccggg

SEQ ID NO: 776 - DNA, 83 bp, Artificial Sequence
  smMIP
  misc_feature (25)..(32): n is a, c, g, or t
gctttgtcttctcccttgtggatgnnnnnnnncttcagcttcccgatatccgacggtagtgtaaggtggactttccccaggac

SEQ ID NO: 777 - DNA, 83 bp, Artificial Sequence
  smMIP
  misc_feature (30)..(37): n is a, c, g, or t
gctgctgcttgggaaaaagggcatcgagannnnnnnncttcagcttcccgatatccgacggtagtgtatggcgtatgccggcg

SEQ ID NO: 778 - DNA, 82 bp, Artificial Sequence
  smMIP
  misc_feature (28)..(35): n is a, c, g, or t
gctgaaggcctccatcaagaagggggannnnnnnncttcagcttcccgatatccgacggtagtgtaggaaacggaatgtacc

SEQ ID NO: 779 - DNA, 83 bp, Artificial Sequence
  smMIP
  misc_feature (30)..(37): n is a, c, g, or t
gcatcatgtcactgcaaagccgttgcagannnnnnnncttcagcttcccgatatccgacggtagtgtaggagaagatgatctc

SEQ ID NO: 780 - DNA, 83 bp, Artificial Sequence
  smMIP
  misc_feature (25)..(32): n is a, c, g, or t
aaagacctggagcggctgacacagnnnnnnnncttcagcttcccgatatccgacggtagtgtccgagtgtatactctgaaaga

SEQ ID NO: 781 - DNA, 83 bp, Artificial Sequence
  smMIP
  misc_feature (29)..(36): n is a, c, g, or t
gcttttgatggtactgatgagtcttgatnnnnnnnncttcagcttcccgatatccgacggtagtgtacgaagatctggaagac

SEQ ID NO: 782 - DNA, 83 bp, Artificial Sequence
  smMIP
  misc_feature (25)..(32): n is a, c, g, or t
gtgacttctgccacattacctgacnnnnnnnncttcagcttcccgatatccgacggtagtgtcctgtagcaagtattttcgcc

SEQ ID NO: 783 - DNA, 83 bp, Artificial Sequence
  smMIP
  misc_feature (26)..(33): n is a, c, g, or t
cacacacacacacacacacaccagcnnnnnnnncttcagcttcccgatatccgacggtagtgtgatagcgctctcatggcttg

SEQ ID NO: 784 - DNA, 83 bp, Artificial Sequence
  smMIP
  misc_feature (29)..(36): n is a, c, g, or t
gcatttgaaggatcaaacaatcaacatcnnnnnnnncttcagcttcccgatatccgacggtagtgtggaaagatacctgataa

SEQ ID NO: 785 - DNA, 83 bp, Artificial Sequence
  smMIP
  misc_feature (24)..(31): n is a, c, g, or t
gccctggggatcggcctcttcatnnnnnnnncttcagcttcccgatatccgacggtagtgtacctgtgccatccaaactgcac

SEQ ID NO: 786 - DNA, 83 bp, Artificial Sequence
  smMIP
  misc_feature (26)..(33): n is a, c, g, or t
gcacggtgtataagggactctggatnnnnnnnncttcagcttcccgatatccgacggtagtgttgctgcaggagagggagctt

SEQ ID NO: 787 - DNA, 83 bp, Artificial Sequence
  smMIP
  misc_feature (27)..(34): n is a, c, g, or t
gccaacaaggaaatcctcgatgaagcnnnnnnnncttcagcttcccgatatccgacggtagtgtaaaagatcaaagtgctggg

SEQ ID NO: 788 - DNA, 83 bp, Artificial Sequence
  smMIP
  misc_feature (23)..(30): n is a, c, g, or t
tctgcctcacctccaccgtgcannnnnnnncttcagcttcccgatatccgacggtagtgtaagttaaaattcccgtcgctatc

SEQ ID NO: 789 - DNA, 82 bp, Artificial Sequence
  smMIP
  misc_feature (29)..(36): n is a, c, g, or t
gctcccagtacctgctcaactggtgtgtnnnnnnnncttcagcttcccgatatccgacggtagtgttggacaacccccacgt

SEQ ID NO: 790 - DNA, 83 bp, Artificial Sequence
  smMIP
  misc_feature (27)..(34): n is a, c, g, or t
gcagaaggaggcaaagtgcctatcaannnnnnnncttcagcttcccgatatccgacggtagtgtaggaccgtcgcttggtgca

SEQ ID NO: 791 - DNA, 83 bp, Artificial Sequence
  smMIP
  misc_feature (27)..(34): n is a, c, g, or t
gagttgatgacctttggatccaagccnnnnnnnncttcagcttcccgatatccgacggtagtgtcggaagagaaagaatacca

SEQ ID NO: 792 - DNA, 83 bp, Artificial Sequence
  smMIP
  misc_feature (23)..(30): n is a, c, g, or t
gccaagtcctacagactccaacnnnnnnnncttcagcttcccgatatccgacggtagtgtcatggtcaagtgctggatgatag

SEQ ID NO: 793 - DNA, 83 bp, Artificial Sequence
  smMIP
  misc_feature (29)..(36): n is a, c, g, or t
gacagcatagacgacaccttcctcccagnnnnnnnncttcagcttcccgatatccgacggtagtgtagtgcaaccagcaacaa

SEQ ID NO: 794 - DNA, 82 bp, Artificial Sequence
  smMIP
  misc_feature (28)..(35): n is a, c, g, or t
gccaccaaattagcctggacaaccctgnnnnnnnncttcagcttcccgatatccgacggtagtgtagagacccacactacca

SEQ ID NO: 795 - DNA, 83 bp, Artificial Sequence
  smMIP
  misc_feature (30)..(37): n is a, c, g, or t
ggaaattacctatgtgcagaggaattatgnnnnnnnncttcagcttcccgatatccgacggtagtgtctggaggaaaagaaag

SEQ ID NO: 796 - DNA, 83 bp, Artificial Sequence
  smMIP
  misc_feature (26)..(33): n is a, c, g, or t
gcaaataaaaccggactgaaggagcnnnnnnnncttcagcttcccgatatccgacggtagtgtgtggctggttatgtcctcat

SEQ ID NO: 797 - DNA, 83 bp, Artificial Sequence
  smMIP
  misc_feature (25)..(32): n is a, c, g, or t
gccctgtgcaacgtggagagcatcnnnnnnnncttcagcttcccgatatccgacggtagtgtctacgaaaattcctatgcctt

SEQ ID NO: 798 - DNA, 83 bp, Artificial Sequence
  smMIP
  misc_feature (30)..(37): n is a, c, g, or t
gcctggtctgccgcaaattccgagacgaannnnnnnncttcagcttcccgatatccgacggtagtgtccagaaactgaccaaa

SEQ ID NO: 799 - DNA, 82 bp, Artificial Sequence
  smMIP
  misc_feature (26)..(33): n is a, c, g, or t
gtcactggtattcatggggacccttnnnnnnnncttcagcttcccgatatccgacggtagtgtcactgacatttgcccaaaa

SEQ ID NO: 800 - DNA, 83 bp, Artificial Sequence
  smMIP
  misc_feature (29)..(36): n is a, c, g, or t
acaacactcttcagcacaatcaaccagannnnnnnncttcagcttcccgatatccgacggtagtgttgcttatcctcaagcaa

SEQ ID NO: 801 - DNA, 82 bp, Artificial Sequence
  smMIP
  misc_feature (29)..(36): n is a, c, g, or t
gtgggctcttcattctggtcattgtgggnnnnnnnncttcagcttcccgatatccgacggtagtgtacccatgccatccaaa

SEQ ID NO: 802 - DNA, 83 bp, Artificial Sequence
  smMIP
  misc_feature (28)..(35): n is a, c, g, or t
gccaattaaatggatggctctggagtgnnnnnnnncttcagcttcccgatatccgacggtagtgtgcagcccgtaatgtctta

SEQ ID NO: 803 - DNA, 83 bp, Artificial Sequence
  smMIP
  misc_feature (25)..(32): n is a, c, g, or t
tgcctcagcctcccatctgcactannnnnnnncttcagcttcccgatatccgacggtagtgtgagtgacgtttggagctatgg

SEQ ID NO: 804 - DNA, 80 bp, Artificial Sequence
  smMIP
  misc_feature (26)..(33): n is a, c, g, or t
gctgagttttcaaggatggctcgagnnnnnnnncttcagcttcccgatatccgacggtagtgtagagaaaggagaacgtt

SEQ ID NO: 805 - DNA, 83 bp, Artificial Sequence
  smMIP
  misc_feature (26)..(33): n is a, c, g, or t
gcttcccagtccaaatgacagcaagnnnnnnnncttcagcttcccgatatccgacggtagtgtgttggatgattgatgctgac

SEQ ID NO: 806 - DNA, 83 bp, Artificial Sequence
  smMIP
  misc_feature (30)..(37): n is a, c, g, or t
gggtgctactgctgagatttttgatgactnnnnnnnncttcagcttcccgatatccgacggtagtgtccatgtcaggaaacca

SEQ ID NO: 807 - DNA, 83 bp, Artificial Sequence
  smMIP
  misc_feature (30)..(37): n is a, c, g, or t
cagtagcacccagaggtacagtgctgaccnnnnnnnncttcagcttcccgatatccgacggtagtgtccaactagcacaattc

SEQ ID NO: 808 - DNA, 83 bp, Artificial Sequence
  smMIP
  misc_feature (30)..(37): n is a, c, g, or t
gcaagatattgttcggaacccatggccttnnnnnnnncttcagcttcccgatatccgacggtagtgtacagaaaagatggaaa

SEQ ID NO: 809 - DNA, 83 bp, Artificial Sequence
  smMIP
  misc_feature (29)..(36): n is a, c, g, or t
gctgagtaatggctcagtcatgatttttnnnnnnnncttcagcttcccgatatccgacggtagtgtcccaccaactgaagtca

SEQ ID NO: 810 - DNA, 82 bp, Artificial Sequence
  smMIP
  misc_feature (29)..(36): n is a, c, g, or t
gtccacaatgctacgtgcacagtgaggannnnnnnncttcagcttcccgatatccgacggtagtgtaagcagcaggatggag

SEQ ID NO: 811 - DNA, 83 bp, Artificial Sequence
  smMIP
  misc_feature (23)..(30): n is a, c, g, or t
aatccttctgtcggcgagccatnnnnnnnncttcagcttcccgatatccgacggtagtgtgtggatttattttgattgggttg

SEQ ID NO: 812 - DNA, 80 bp, Artificial Sequence
  smMIP
  misc_feature (27)..(34): n is a, c, g, or t
gcgagatgacatgactgtctgtgttgnnnnnnnncttcagcttcccgatatccgacggtagtgtacaggaccaaagcata

SEQ ID NO: 813 - DNA, 83 bp, Artificial Sequence
  smMIP
  misc_feature (24)..(31): n is a, c, g, or t
gcctgttaaatggatcgccatagnnnnnnnncttcagcttcccgatatccgacggtagtgtcttcatcgagatttagctgctc

SEQ ID NO: 814 - DNA, 83 bp, Artificial Sequence
  smMIP
  misc_feature (27)..(34): n is a, c, g, or t
gaagactgcctggatgaactgtatgannnnnnnncttcagcttcccgatatccgacggtagtgtgtgatgtgtgggcatttgg

SEQ ID NO: 815 - DNA, 83 bp, Artificial Sequence
  smMIP
  misc_feature (28)..(35): n is a, c, g, or t
ctcttagaaagtttgcctgacgttcggnnnnnnnncttcagcttcccgatatccgacggtagtgttggccacaggttgaagca

SEQ ID NO: 816 - DNA, 82 bp, Artificial Sequence
  smMIP
  misc_feature (26)..(33): n is a, c, g, or t
gctgacgactcctcagaaggctcagnnnnnnnncttcagcttcccgatatccgacggtagtgttctgctgcagtcacagctg

SEQ ID NO: 817 - DNA, 83 bp, Artificial Sequence
  smMIP
  misc_feature (27)..(34): n is a, c, g, or t
tcgcttccttcagcataaccagtgtgnnnnnnnncttcagcttcccgatatccgacggtagtgtctcaatcagtgtacctaat

SEQ ID NO: 818 - DNA, 83 bp, Artificial Sequence
  smMIP
  misc_feature (23)..(30): n is a, c, g, or t
cgaacagcctgaaaaatcccccnnnnnnnncttcagcttcccgatatccgacggtagtgttcctcactttactaagcagcctg

SEQ ID NO: 819 - DNA, 82 bp, Artificial Sequence
  smMIP
  misc_feature (21)..(28): n is a, c, g, or t
ttccgcccttcccccccaacnnnnnnnncttcagcttcccgatatccgacggtagtgtcagcctgcccagcctcagtggcat

SEQ ID NO: 820 - DNA, 83 bp, Artificial Sequence
  smMIP
  misc_feature (22)..(29): n is a, c, g, or t
tcaccatctacgactgcagccnnnnnnnncttcagcttcccgatatccgacggtagtgttttggtcaccagattgcctactgc

SEQ ID NO: 821 - DNA, 83 bp, Artificial Sequence
  smMIP
  misc_feature (22)..(29): n is a, c, g, or t
cagacccctgcacggagctgannnnnnnncttcagcttcccgatatccgacggtagtgtttctcctacgtgctgcccctggtc

SEQ ID NO: 822 - DNA, 81 bp, Artificial Sequence
  smMIP
  misc_feature (25)..(32): n is a, c, g, or t
ccggggagcctctcaccctcgttannnnnnnncttcagcttcccgatatccgacggtagtgtgaggtggctgtggctgagg

SEQ ID NO: 823 - DNA, 83 bp, Artificial Sequence
  smMIP
  misc_feature (30)..(37): n is a, c, g, or t
gctgcgacatccagattgtctctgacagannnnnnnncttcagcttcccgatatccgacggtagtgtggccaagagggagaag

SEQ ID NO: 824 - DNA, 83 bp, Artificial Sequence
  smMIP
  misc_feature (23)..(30): n is a, c, g, or t
ttcaaccagaccatcgccacacnnnnnnnncttcagcttcccgatatccgacggtagtgttaccgggtcaagataggccaagt

SEQ ID NO: 825 - DNA, 83 bp, Artificial Sequence
  smMIP
  misc_feature (25)..(32): n is a, c, g, or t
gcaaaggcttcgctgagctgcagannnnnnnncttcagcttcccgatatccgacggtagtgtgtcctgctgctgctctccgtg

SEQ ID NO: 826 - DNA, 82 bp, Artificial Sequence
  smMIP
  misc_feature (28)..(35): n is a, c, g, or t
ggagtataagcacttcgtgacccgcacnnnnnnnncttcagcttcccgatatccgacggtagtgttgctgcagatggaggag

SEQ ID NO: 827 - DNA, 83 bp, Artificial Sequence
  smMIP
  misc_feature (24)..(31): n is a, c, g, or t
tcccagaccctcaactcccagggnnnnnnnncttcagcttcccgatatccgacggtagtgtacatgacagatctcaccaagga

SEQ ID NO: 828 - DNA, 83 bp, Artificial Sequence
  smMIP
  misc_feature (30)..(37): n is a, c, g, or t
gtccatctgcatgtacagctgtctgcgggnnnnnnnncttcagcttcccgatatccgacggtagtgttactacaccagcatca

SEQ ID NO: 829 - DNA, 83 bp, Artificial Sequence
  smMIP
  misc_feature (20)..(27): n is a, c, g, or t
ttcgcctccagcacacagannnnnnnncttcagcttcccgatatccgacggtagtgtatggactcgctgagcgtgcgggccat

SEQ ID NO: 830 - DNA, 83 bp, Artificial Sequence
  smMIP
  misc_feature (28)..(35): n is a, c, g, or t
ctttttcgacttcctggaggagcaggcnnnnnnnncttcagcttcccgatatccgacggtagtgttgctcccggaaatctacc

SEQ ID NO: 831 - DNA, 83 bp, Artificial Sequence
  smMIP
  misc_feature (26)..(33): n is a, c, g, or t
tcatcgcgcaggccttcatcgacgcnnnnnnnncttcagcttcccgatatccgacggtagtgtaccccgacaccctacacatc

SEQ ID NO: 832 - DNA, 83 bp, Artificial Sequence
  smMIP
  misc_feature (30)..(37): n is a, c, g, or t
ctggccgaggagtcgaggaaataccagaannnnnnnncttcagcttcccgatatccgacggtagtgtattcgccaaccaacaa

SEQ ID NO: 833 - DNA, 83 bp, Artificial Sequence
  smMIP
  misc_feature (30)..(37): n is a, c, g, or t
ggtggtggctttgatggaggacaacatctnnnnnnnncttcagcttcccgatatccgacggtagtgtaacaccaatgtggcca

SEQ ID NO: 834 - DNA, 81 bp, Artificial Sequence
  smMIP
  misc_feature (19)..(26): n is a, c, g, or t
tctcccagcaccaagaccnnnnnnnncttcagcttcccgatatccgacggtagtgtctgccccctgtcctgtgcagtcagc

SEQ ID NO: 835 - DNA, 82 bp, Artificial Sequence
  smMIP
  misc_feature (29)..(36): n is a, c, g, or t
gcttccctgaggaggagaagtgcttctgnnnnnnnncttcagcttcccgatatccgacggtagtgtgcgatgttgtggagac

SEQ ID NO: 836 - DNA, 78 bp, Artificial Sequence
  smMIP
  misc_feature (24)..(31): n is a, c, g, or t
attgtatggggcctgcagccaggnnnnnnnncttcagcttcccgatatccgacggtagtgtaaaggcagagcagggta

SEQ ID NO: 837 - DNA, 82 bp, Artificial Sequence
  smMIP
  misc_feature (24)..(31): n is a, c, g, or t
cggcttgtcccgagatgtttatgnnnnnnnncttcagcttcccgatatccgacggtagtgtctcatctcatttgcctggcag

SEQ ID NO: 838 - DNA, 82 bp, Artificial Sequence
  smMIP
  misc_feature (29)..(36): n is a, c, g, or t
gatcatatctacaccacgcaaagtgatgnnnnnnnncttcagcttcccgatatccgacggtagtgtgaggggcggaagatga

SEQ ID NO: 839 - DNA, 83 bp, Artificial Sequence
  smMIP
  misc_feature (21)..(28): n is a, c, g, or t
ggagatgtaccgcctgatgcnnnnnnnncttcagcttcccgatatccgacggtagtgttggtcttttggtgtcctgctgtggg

SEQ ID NO: 840 - DNA, 82 bp, Artificial Sequence
  smMIP
  misc_feature (27)..(34): n is a, c, g, or t
caccgctggtggactgtaataatgccnnnnnnnncttcagcttcccgatatccgacggtagtgtggtgtttgcggacatcag

SEQ ID NO: 841 - DNA, 83 bp, Artificial Sequence
  smMIP
  misc_feature (28)..(35): n is a, c, g, or t
ggatgctttcaccctcagcggcaaaatnnnnnnnncttcagcttcccgatatccgacggtagtgtgaaaacaaactctatggc

SEQ ID NO: 842 - DNA, 82 bp, Artificial Sequence
  smMIP
  misc_feature (29)..(36): n is a, c, g, or t
gtgaaaggtaatggactcacaaggggaannnnnnnncttcagcttcccgatatccgacggtagtgtacgagagctgatggca

SEQ ID NO: 843 - DNA, 79 bp, Artificial Sequence
  smMIP
  misc_feature (21)..(28): n is a, c, g, or t
gctcctgggagaagctcagtnnnnnnnncttcagcttcccgatatccgacggtagtgttgaggaggtgcccagcttccg

SEQ ID NO: 844 - DNA, 83 bp, Artificial Sequence
  smMIP
  misc_feature (23)..(30): n is a, c, g, or t
tcgtcggaccactgaagctaccnnnnnnnncttcagcttcccgatatccgacggtagtgtctgtgtcctcatcttggctctct

SEQ ID NO: 845 - DNA, 83 bp, Artificial Sequence
  smMIP
  misc_feature (20)..(27): n is a, c, g, or t
tcctcctctattcccggctnnnnnnnncttcagcttcccgatatccgacggtagtgttctgcatgaaggaatttgaccatccc

SEQ ID NO: 846 - DNA, 82 bp, Artificial Sequence
  smMIP
  misc_feature (23)..(30): n is a, c, g, or t
gtccgtgtgtgtggcggacttcnnnnnnnncttcagcttcccgatatccgacggtagtgtagtgtacctgcccactcagatg

SEQ ID NO: 847 - DNA, 83 bp, Artificial Sequence
  smMIP
  misc_feature (29)..(36): n is a, c, g, or t
gccattgagagtctagctgaccgtgtctnnnnnnnncttcagcttcccgatatccgacggtagtgtaggaactgcatgctgaa

SEQ ID NO: 848 - DNA, 83 bp, Artificial Sequence
  smMIP
  misc_feature (28)..(35): n is a, c, g, or t
cgggcgtggagaacagcgagatttatgnnnnnnnncttcagcttcccgatatccgacggtagtgtaagatgccagtcaagtgg

SEQ ID NO: 849 - DNA, 82 bp, Artificial Sequence
  smMIP
  misc_feature (29)..(36): n is a, c, g, or t
ggactgtatgccttgatgtcgcggtgctnnnnnnnncttcagcttcccgatatccgacggtagtgtggggtgacaatgtggg

SEQ ID NO: 850 - DNA, 83 bp, Artificial Sequence
  smMIP
  misc_feature (19)..(26): n is a, c, g, or t
agctgaccccccaacccannnnnnnncttcagcttcccgatatccgacggtagtgtgttttacagagctgcgggaagatttgg

SEQ ID NO: 851 - DNA, 82 bp, Artificial Sequence
  smMIP
  misc_feature (21)..(28): n is a, c, g, or t
ttcccaccccacgccttatcnnnnnnnncttcagcttcccgatatccgacggtagtgttcagcctgctgataggggctcccc

SEQ ID NO: 852 - DNA, 81 bp, Artificial Sequence
  smMIP
  misc_feature (22)..(29): n is a, c, g, or t
gcccgaagacaggactgtggcnnnnnnnncttcagcttcccgatatccgacggtagtgtagctcagaatcacctccctgca

SEQ ID NO: 853 - DNA, 82 bp, Artificial Sequence
  smMIP
  misc_feature (21)..(28): n is a, c, g, or t
tccccctggccacggctccannnnnnnncttcagcttcccgatatccgacggtagtgtgctggagggcttgccttacttcct

SEQ ID NO: 854 - DNA, 80 bp, Artificial Sequence
  smMIP
  misc_feature (24)..(31): n is a, c, g, or t
gccaggtcttgaaggctgtccaannnnnnnncttcagcttcccgatatccgacggtagtgtgtctgccatgccttgtgct

SEQ ID NO: 855 - DNA, 83 bp, Artificial Sequence
  smMIP
  misc_feature (29)..(36): n is a, c, g, or t
gccctggggatcggcctcttcatgcgaannnnnnnncttcagcttcccgatatccgacggtagtgtgacaagtgcaaccttct

SEQ ID NO: 856 - DNA, 81 bp, Artificial Sequence
  smMIP
  misc_feature (24)..(31): n is a, c, g, or t
gtggtgacagatcacggctcgtgnnnnnnnncttcagcttcccgatatccgacggtagtgtgagagccggagcgagctctt

SEQ ID NO: 857 - DNA, 81 bp, Artificial Sequence
  smMIP
  misc_feature (28)..(35): n is a, c, g, or t
gccgcaaagtgtgtaacggaataggtannnnnnnncttcagcttcccgatatccgacggtagtgtctggaggaaaagaaag

SEQ ID NO: 858 - DNA, 83 bp, Artificial Sequence
  smMIP
  misc_feature (30)..(37): n is a, c, g, or t
gccaagggagtttgtggagaactctgagtnnnnnnnncttcagcttcccgatatccgacggtagtgtattctgaaaaccgtaa

SEQ ID NO: 859 - DNA, 83 bp, Artificial Sequence
  smMIP
  misc_feature (29)..(36): n is a, c, g, or t
cggggaccagacaactgtatccagtgtgnnnnnnnncttcagcttcccgatatccgacggtagtgtaacctagaaatcatacg

SEQ ID NO: 860 - DNA, 83 bp, Artificial Sequence
  smMIP
  misc_feature (21)..(28): n is a, c, g, or t
cacaatcagcctctgaacccnnnnnnnncttcagcttcccgatatccgacggtagtgtccaaagttccgtgagttgatcatcg

SEQ ID NO: 861 - DNA, 83 bp, Artificial Sequence
  smMIP
  misc_feature (29)..(36): n is a, c, g, or t
gtttcctaattcatctcagaacggttcannnnnnnncttcagcttcccgatatccgacggtagtgtaatagttcaaccagatc

SEQ ID NO: 862 - DNA, 83 bp, Artificial Sequence
  smMIP
  misc_feature (30)..(37): n is a, c, g, or t
cagtccattactgcaaaatactgtccacannnnnnnncttcagcttcccgatatccgacggtagtgtaaaaagagaaagcaaa

SEQ ID NO: 863 - DNA, 83 bp, Artificial Sequence
  smMIP
  misc_feature (30)..(37): n is a, c, g, or t
gcaggttttcccaaatagtgcaccccttgnnnnnnnncttcagcttcccgatatccgacggtagtgtgctttgcagcgcgttg

SEQ ID NO: 864 - DNA, 83 bp, Artificial Sequence
  smMIP
  misc_feature (28)..(35): n is a, c, g, or t
actagagttctccttggaaatgagagcnnnnnnnncttcagcttcccgatatccgacggtagtgtgacatcagagggtcgctt

SEQ ID NO: 865 - DNA, 83 bp, Artificial Sequence
  smMIP
  misc_feature (26)..(33): n is a, c, g, or t
gcacgatgaatactgtgtcaaacagnnnnnnnncttcagcttcccgatatccgacggtagtgtttgaaggagggacaaggctg

SEQ ID NO: 866 - DNA, 83 bp, Artificial Sequence
  smMIP
  misc_feature (26)..(33): n is a, c, g, or t
gccaaccgagagacaagcatcttcannnnnnnncttcagcttcccgatatccgacggtagtgtaatgagagctgcaccttgac

SEQ ID NO: 867 - DNA, 83 bp, Artificial Sequence
  smMIP
  misc_feature (30)..(37): n is a, c, g, or t
attagtacttggtggaaagaacctctcaannnnnnnncttcagcttcccgatatccgacggtagtgtcccaaaccatttcaac

SEQ ID NO: 868 - DNA, 83 bp, Artificial Sequence
  smMIP
  misc_feature (29)..(36): n is a, c, g, or t
cagttagtgtcccgagaatggtcataaannnnnnnncttcagcttcccgatatccgacggtagtgtaaattcatccaaccaaa

SEQ ID NO: 869 - DNA, 83 bp, Artificial Sequence
  smMIP
  misc_feature (28)..(35): n is a, c, g, or t
gtggtgggagcacaataacaggtgttgnnnnnnnncttcagcttcccgatatccgacggtagtgtcaaaccatttcaactgag

SEQ ID NO: 870 - DNA, 83 bp, Artificial Sequence
  smMIP
  misc_feature (26)..(33): n is a, c, g, or t
gcatgtcaacatcgctctaattcagnnnnnnnncttcagcttcccgatatccgacggtagtgtattcatccaaccaaatcttt

SEQ ID NO: 871 - DNA, 83 bp, Artificial Sequence
  smMIP
  misc_feature (26)..(33): n is a, c, g, or t
gcatgtcaacatcgctctaattcagnnnnnnnncttcagcttcccgatatccgacggtagtgtccaaaccatttcaactgagt

SEQ ID NO: 872 - DNA, 83 bp, Artificial Sequence
  smMIP
  misc_feature (29)..(36): n is a, c, g, or t
gcctttttcatgttagatgggatcctttnnnnnnnncttcagcttcccgatatccgacggtagtgtctatgaaattcatccaa

SEQ ID NO: 873 - DNA, 83 bp, Artificial Sequence
  smMIP
  misc_feature (27)..(34): n is a, c, g, or t
gtcacaacaaccttggaagtagtagannnnnnnncttcagcttcccgatatccgacggtagtgtataatagctggcatcacgg

SEQ ID NO: 874 - DNA, 83 bp, Artificial Sequence
  smMIP
  misc_feature (28)..(35): n is a, c, g, or t
ccgaaggaggcacttacacattcctagnnnnnnnncttcagcttcccgatatccgacggtagtgtgaacaccagcagtggatc

SEQ ID NO: 875 - DNA, 83 bp, Artificial Sequence
  smMIP
  misc_feature (27)..(34): n is a, c, g, or t
gcacaatggcacggttgaatgtaaggnnnnnnnncttcagcttcccgatatccgacggtagtgttgtccaggaactgagcaga

SEQ ID NO: 876 - DNA, 83 bp, Artificial Sequence
  smMIP
  misc_feature (30)..(37): n is a, c, g, or t
caaatgggagtttcccagaaacaggctgannnnnnnncttcagcttcccgatatccgacggtagtgtgtgatgattctgacct

SEQ ID NO: 877 - DNA, 83 bp, Artificial Sequence
  smMIP
  misc_feature (29)..(36): n is a, c, g, or t
gctatggtgatcttttgaattttttgagnnnnnnnncttcagcttcccgatatccgacggtagtgtaacgggaagccctcatg

SEQ ID NO: 878 - DNA, 83 bp, Artificial Sequence
  smMIP
  misc_feature (30)..(37): n is a, c, g, or t
gccgacaaaaggagatctgtgagaataggnnnnnnnncttcagcttcccgatatccgacggtagtgtaagatcatgcagaagc

SEQ ID NO: 879 - DNA, 83 bp, Artificial Sequence
  smMIP
  misc_feature (26)..(33): n is a, c, g, or t
gtgaagtggatggcacctgaaagcannnnnnnncttcagcttcccgatatccgacggtagtgtagagacttggcagccagaaa

SEQ ID NO: 880 - DNA, 83 bp, Artificial Sequence
  smMIP
  misc_feature (25)..(32): n is a, c, g, or t
gctgttatgcactgatccgggcttnnnnnnnncttcagcttcccgatatccgacggtagtgtttctgctcctactgcttcgcg

SEQ ID NO: 881 - DNA, 83 bp, Artificial Sequence
  smMIP
  misc_feature (29)..(36): n is a, c, g, or t
tgccaagcttttccttgttgaccgctccnnnnnnnncttcagcttcccgatatccgacggtagtgtaacgaatgagaataagc

SEQ ID NO: 882 - DNA, 83 bp, Artificial Sequence
  smMIP
  misc_feature (23)..(30): n is a, c, g, or t
gctgtgcctgttgtgtctgtgtnnnnnnnncttcagcttcccgatatccgacggtagtgtaaggcgggcatcatgatcaaaag

SEQ ID NO: 883 - DNA, 83 bp, Artificial Sequence
  smMIP
  misc_feature (30)..(37): n is a, c, g, or t
ggattcaaagcataaaaaccattacaagannnnnnnncttcagcttcccgatatccgacggtagtgtcaagaggatggattcg

SEQ ID NO: 884 - DNA, 83 bp, Artificial Sequence
  smMIP
  misc_feature (30)..(37): n is a, c, g, or t
catgttgcagcaattcactgtaaagctggnnnnnnnncttcagcttcccgatatccgacggtagtgtacaccgccaaatttaa

SEQ ID NO: 885 - DNA, 83 bp, Artificial Sequence
  smMIP
  misc_feature (28)..(35): n is a, c, g, or t
gccctagatttctatggggaagtaaggnnnnnnnncttcagcttcccgatatccgacggtagtgtccaatggctaagtgaaga

SEQ ID NO: 886 - DNA, 82 bp, Artificial Sequence
  smMIP
  misc_feature (29)..(36): n is a, c, g, or t
ggattatagaccagtggcactgttgtttnnnnnnnncttcagcttcccgatatccgacggtagtgttttaaaggcacaagag

SEQ ID NO: 887 - DNA, 82 bp, Artificial Sequence
  smMIP
  misc_feature (24)..(31): n is a, c, g, or t
cctcagtttgtggtctgccagctnnnnnnnncttcagcttcccgatatccgacggtagtgtgtcagaggcgctatgtgtatt

SEQ ID NO: 888 - DNA, 81 bp, Artificial Sequence
  smMIP
  misc_feature (25)..(32): n is a, c, g, or t
gccgttacctgtgtgtggtgatatnnnnnnnncttcagcttcccgatatccgacggtagtgtttccaatgttcagtggcgg

SEQ ID NO: 889 - DNA, 83 bp, Artificial Sequence
  smMIP
  misc_feature (23)..(30): n is a, c, g, or t
accaggaccagaggaaacctcannnnnnnncttcagcttcccgatatccgacggtagtgtgttcatgtactttgagttccctc

SEQ ID NO: 890 - DNA, 83 bp, Artificial Sequence
  smMIP
  misc_feature (24)..(31): n is a, c, g, or t
agccaaccgatacttttctccaannnnnnnncttcagcttcccgatatccgacggtagtgtgtagaaaatggaagtctatgtg

SEQ ID NO: 891 - DNA, 83 bp, Artificial Sequence
  smMIP
  misc_feature (30)..(37): n is a, c, g, or t
gatcagcatacacaaattacaaaagtctgnnnnnnnncttcagcttcccgatatccgacggtagtgtcgtcaaatccagaggc

SEQ ID NO: 892 - DNA, 83 bp, Artificial Sequence
  smMIP
  misc_feature (29)..(36): n is a, c, g, or t
ggacctttttttttttaatggcaataggnnnnnnnncttcagcttcccgatatccgacggtagtgttgactctgatccagaga

SEQ ID NO: 893 - DNA, 83 bp, Artificial Sequence
  smMIP
  misc_feature (26)..(33): n is a, c, g, or t
ttgctcctcctgagcgcaagtactcnnnnnnnncttcagcttcccgatatccgacggtagtgtacatccgcaaagacctgtac

SEQ ID NO: 894 - DNA, 81 bp, Artificial Sequence
  smMIP
  misc_feature (25)..(32): n is a, c, g, or t
tctggcaccacaccttctacaatgnnnnnnnncttcagcttcccgatatccgacggtagtgtgtgatggtgggcatgggtc

SEQ ID NO: 895 - DNA, 83 bp, Artificial Sequence
  smMIP
  misc_feature (21)..(28): n is a, c, g, or t
aaccccaaggccaaccgcgannnnnnnncttcagcttcccgatatccgacggtagtgttgaagtaccccatcgagcacggcat

SEQ ID NO: 896 - DNA, 83 bp, Artificial Sequence
  smMIP
  misc_feature (27)..(34): n is a, c, g, or t
ggtcatcaccattggcaatgagcggtnnnnnnnncttcagcttcccgatatccgacggtagtgtgagcgggaaatcgtgcgtg

SEQ ID NO: 897 - DNA, 82 bp, Artificial Sequence
  smMIP
  misc_feature (25)..(32): n is a, c, g, or t
ggcatccacgaaactaccttcaacnnnnnnnncttcagcttcccgatatccgacggtagtgttgcttccagctcctccctgg

SEQ ID NO: 898 - DNA, 82 bp, Artificial Sequence
  smMIP
  misc_feature (24)..(31): n is a, c, g, or t
ccaccatgtaccctggcattgccnnnnnnnncttcagcttcccgatatccgacggtagtgtactcttccagccttccttcct

SEQ ID NO: 899 - DNA, 83 bp, Artificial Sequence
  smMIP
  misc_feature (30)..(37): n is a, c, g, or t
gttccataaactctggattgcattcctacnnnnnnnncttcagcttcccgatatccgacggtagtgtcagagattcttacccc

SEQ ID NO: 900 - DNA, 83 bp, Artificial Sequence
  smMIP
  misc_feature (27)..(34): n is a, c, g, or t
gtgagatgtctccagcatttttacggnnnnnnnncttcagcttcccgatatccgacggtagtgtttcttttcggggtgttcgc

SEQ ID NO: 901 - DNA, 83 bp, Artificial Sequence
  smMIP
  misc_feature (19)..(26): n is a, c, g, or t
actcccatccagtgtctcnnnnnnnncttcagcttcccgatatccgacggtagtgtctcttaacatctatatccaccttcatt

SEQ ID NO: 902 - DNA, 83 bp, Artificial Sequence
  smMIP
  misc_feature (30)..(37): n is a, c, g, or t
gctgaccatatgtggctgggactttggatnnnnnnnncttcagcttcccgatatccgacggtagtgttggtgccacgacaaat

SEQ ID NO: 903 - DNA, 83 bp, Artificial Sequence
  smMIP
  misc_feature (24)..(31): n is a, c, g, or t
gctggtggcactttacttactttnnnnnnnncttcagcttcccgatatccgacggtagtgtgtcctgccatgaataagcattt

SEQ ID NO: 904 - DNA, 81 bp, Artificial Sequence
  smMIP
  misc_feature (27)..(34): n is a, c, g, or t
gctttgccagtggtgggagcacaatannnnnnnncttcagcttcccgatatccgacggtagtgtagccaaccgagagacaa

SEQ ID NO: 905 - DNA, 83 bp, Artificial Sequence
  smMIP
  misc_feature (26)..(33): n is a, c, g, or t
gccttttgaaaagccagtgatgatcnnnnnnnncttcagcttcccgatatccgacggtagtgtttgtaccactccttccctgc

SEQ ID NO: 906 - DNA, 83 bp, Artificial Sequence
  smMIP
  misc_feature (30)..(37): n is a, c, g, or t
gcaaattaaagatctgggcagtgaattagnnnnnnnncttcagcttcccgatatccgacggtagtgtgtccttggaaaagtaa

SEQ ID NO: 907 - DNA, 83 bp, Artificial Sequence
  smMIP
  misc_feature (27)..(34): n is a, c, g, or t
cccaactacagaaatggtttcaaatgnnnnnnnncttcagcttcccgatatccgacggtagtgtcttgggtttttcctgtggc

SEQ ID NO: 908 - DNA, 83 bp, Artificial Sequence
  smMIP
  misc_feature (26)..(33): n is a, c, g, or t
gcagtatcctctgacagacatgtccnnnnnnnncttcagcttcccgatatccgacggtagtgtgcttgtaagtgcccgaagtg

SEQ ID NO: 909 - DNA, 83 bp, Artificial Sequence
  smMIP
  misc_feature (29)..(36): n is a, c, g, or t
caatttctgaccgagggaatcatcatgannnnnnnncttcagcttcccgatatccgacggtagtgtgaagtcataggaagagg

SEQ ID NO: 910 - DNA, 83 bp, Artificial Sequence
  smMIP
  misc_feature (28)..(35): n is a, c, g, or t
gcaaactcaaaagtttaccaccaagtcnnnnnnnncttcagcttcccgatatccgacggtagtgtaaaaattcacagtcaagg

SEQ ID NO: 911 - DNA, 83 bp, Artificial Sequence
  smMIP
  misc_feature (28)..(35): n is a, c, g, or t
actttcattggggagcactatgtccatnnnnnnnncttcagcttcccgatatccgacggtagtgtactcctacaacccgaata

SEQ ID NO: 912 - DNA, 83 bp, Artificial Sequence
  smMIP
  misc_feature (29)..(36): n is a, c, g, or t
gtattgttatttaaattactggattctannnnnnnncttcagcttcccgatatccgacggtagtgtcatagtgctagtactat

SEQ ID NO: 913 - DNA, 83 bp, Artificial Sequence
  smMIP
  misc_feature (24)..(31): n is a, c, g, or t
cggttcatcaacttctttgtaggnnnnnnnncttcagcttcccgatatccgacggtagtgtacaatcatactgctgacataca

SEQ ID NO: 914 - DNA, 83 bp, Artificial Sequence
  smMIP
  misc_feature (25)..(32): n is a, c, g, or t
tccgccggaaggccttcctccactnnnnnnnncttcagcttcccgatatccgacggtagtgtaacaatgtcaagacagccgtc

SEQ ID NO: 915 - DNA, 83 bp, Artificial Sequence
  smMIP
  misc_feature (20)..(27): n is a, c, g, or t
cagctgacccactcactggnnnnnnnncttcagcttcccgatatccgacggtagtgttttgtatttggtcagtctggggcagg

SEQ ID NO: 916 - DNA, 83 bp, Artificial Sequence
  smMIP
  misc_feature (21)..(28): n is a, c, g, or t
ccaccttgtctcagccaccannnnnnnncttcagcttcccgatatccgacggtagtgttacaatgccaccctctccgtccatc

SEQ ID NO: 917 - DNA, 83 bp, Artificial Sequence
  smMIP
  misc_feature (19)..(26): n is a, c, g, or t
tacctcaccgtggctgctnnnnnnnncttcagcttcccgatatccgacggtagtgtctttatgcctggctttgcccctctcac

SEQ ID NO: 918 - DNA, 83 bp, Artificial Sequence
  smMIP
  misc_feature (26)..(33): n is a, c, g, or t
ccaccactctttgaactggaccaagnnnnnnnncttcagcttcccgatatccgacggtagtgtcggggcttctcattgttgat

SEQ ID NO: 919 - DNA, 81 bp, Artificial Sequence
  smMIP
  misc_feature (22)..(29): n is a, c, g, or t
gccgaggaggtgtctgtgtgannnnnnnncttcagcttcccgatatccgacggtagtgtagacatcaagcataatcggccg

SEQ ID NO: 920 - DNA, 83 bp, Artificial Sequence
  smMIP
  misc_feature (27)..(34): n is a, c, g, or t
cccatctgacaatggctttgacagtgnnnnnnnncttcagcttcccgatatccgacggtagtgtcccaatctacaagtaccca

SEQ ID NO: 921 - DNA, 81 bp, Artificial Sequence
  smMIP
  misc_feature (27)..(34): n is a, c, g, or t
gccaagggaatgtactaccttgaggannnnnnnncttcagcttcccgatatccgacggtagtgtgtcatctctgcagcttg

SEQ ID NO: 922 - DNA, 83 bp, Artificial Sequence
  smMIP
  misc_feature (28)..(35): n is a, c, g, or t
gtggatggcccttgagagtatccacttnnnnnnnncttcagcttcccgatatccgacggtagtgtaaacgtgctactcaagtc

SEQ ID NO: 923 - DNA, 81 bp, Artificial Sequence
  smMIP
  misc_feature (28)..(35): n is a, c, g, or t
gcagtttctgggagcagtgaacggtgcnnnnnnnncttcagcttcccgatatccgacggtagtgtagcctaccagttggaa

SEQ ID NO: 924 - DNA, 79 bp, Artificial Sequence
  smMIP
  misc_feature (24)..(31): n is a, c, g, or t
tactccctcctcccgggaaggcannnnnnnncttcagcttcccgatatccgacggtagtgtcggagatagcgcctacca

SEQ ID NO: 925 - DNA, 80 bp, Artificial Sequence
  smMIP
  misc_feature (22)..(29): n is a, c, g, or t
ctcctgctccctgtggcactcnnnnnnnncttcagcttcccgatatccgacggtagtgtccccccatgtccattatgccc

SEQ ID NO: 926 - DNA, 82 bp, Artificial Sequence
  smMIP
  misc_feature (28)..(35): n is a, c, g, or t
gctttgtcacatggacacaattgactgnnnnnnnncttcagcttcccgatatccgacggtagtgtggaagtttgccatcttc

SEQ ID NO: 927 - DNA, 82 bp, Artificial Sequence
  smMIP
  misc_feature (29)..(36): n is a, c, g, or t
gcctgccggcacttcaatgacagtggagnnnnnnnncttcagcttcccgatatccgacggtagtgtacattgaccaagacca

SEQ ID NO: 928 - DNA, 83 bp, Artificial Sequence
  smMIP
  misc_feature (19)..(26): n is a, c, g, or t
ttttgccccaacccgcctnnnnnnnncttcagcttcccgatatccgacggtagtgtccccaactctgtcgtctgtgccttccc

SEQ ID NO: 929 - DNA, 82 bp, Artificial Sequence
  smMIP
  misc_feature (24)..(31): n is a, c, g, or t
aactggagcccttgggcacccagnnnnnnnncttcagcttcccgatatccgacggtagtgtttctggtctggtgcctgaggg

SEQ ID NO: 930 - DNA, 83 bp, Artificial Sequence
  smMIP
  misc_feature (25)..(32): n is a, c, g, or t
ggcacctgtctcactcttgaaggcnnnnnnnncttcagcttcccgatatccgacggtagtgtcctcaccgtgactaacatgcc

SEQ ID NO: 931 - DNA, 83 bp, Artificial Sequence
  smMIP
  misc_feature (27)..(34): n is a, c, g, or t
ggagctgctggctttacactgcctggnnnnnnnncttcagcttcccgatatccgacggtagtgtggcttagggcagtggaaag

SEQ ID NO: 932 - DNA, 79 bp, Artificial Sequence
  smMIP
  misc_feature (25)..(32): n is a, c, g, or t
gcactggtcttcagctactggtggnnnnnnnncttcagcttcccgatatccgacggtagtgtggtctgcgtagatggtg

SEQ ID NO: 933 - DNA, 83 bp, Artificial Sequence
  smMIP
  misc_feature (27)..(34): n is a, c, g, or t
gtggaggccttcctgcgagaggggctnnnnnnnncttcagcttcccgatatccgacggtagtgtacagtgaccgagtcattgg

SEQ ID NO: 934 - DNA, 82 bp, Artificial Sequence
  smMIP
  misc_feature (26)..(33): n is a, c, g, or t
cctcatcagctttggcctgcaggtannnnnnnncttcagcttcccgatatccgacggtagtgttgtgctggctctcattggt

SEQ ID NO: 935 - DNA, 79 bp, Artificial Sequence
  smMIP
  misc_feature (25)..(32): n is a, c, g, or t
cagtcaaggtggctgactttggttnnnnnnnncttcagcttcccgatatccgacggtagtgtaaccccaccgtgaagga

SEQ ID NO: 936 - DNA, 79 bp, Artificial Sequence
  smMIP
  misc_feature (25)..(32): n is a, c, g, or t
ctcacccatgccagggaatgtacgnnnnnnnncttcagcttcccgatatccgacggtagtgttgggggaggtggagcag

SEQ ID NO: 937 - DNA, 82 bp, Artificial Sequence
  smMIP
  misc_feature (24)..(31): n is a, c, g, or t
ccacacgggagccttcgtatactnnnnnnnncttcagcttcccgatatccgacggtagtgtttcagcccacgctcagtgtct

SEQ ID NO: 938 - DNA, 82 bp, Artificial Sequence
  smMIP
  misc_feature (22)..(29): n is a, c, g, or t
tgcccagaggctcctttctccnnnnnnnncttcagcttcccgatatccgacggtagtgttgtgagctggagtattcccctcc

SEQ ID NO: 939 - DNA, 83 bp, Artificial Sequence
  smMIP
  misc_feature (29)..(36): n is a, c, g, or t
gtggaaaccgcagcttgtctgcagtggannnnnnnncttcagcttcccgatatccgacggtagtgtacaacgaggctgcaaga

SEQ ID NO: 940 - DNA, 81 bp, Artificial Sequence
  smMIP
  misc_feature (21)..(28): n is a, c, g, or t
cgtgtccttggtgctagtggnnnnnnnncttcagcttcccgatatccgacggtagtgtttgctcagtaccactgatgtccc

SEQ ID NO: 941 - DNA, 80 bp, Artificial Sequence
  smMIP
  misc_feature (24)..(31): n is a, c, g, or t
gcctgtggcagtggatggtgttgnnnnnnnncttcagcttcccgatatccgacggtagtgttgagctccgaatgtcctgg

SEQ ID NO: 942 - DNA, 82 bp, Artificial Sequence
  smMIP
  misc_feature (28)..(35): n is a, c, g, or t
gcgggaaaggcgggaagaacaccatgannnnnnnncttcagcttcccgatatccgacggtagtgtaacaacgcctaccagaa

SEQ ID NO: 943 - DNA, 83 bp, Artificial Sequence
  smMIP
  misc_feature (29)..(36): n is a, c, g, or t
gctgtacatcctggttgggcagcagggannnnnnnncttcagcttcccgatatccgacggtagtgtagccaccgacacctaca

SEQ ID NO: 944 - DNA, 82 bp, Artificial Sequence
  smMIP
  misc_feature (24)..(31): n is a, c, g, or t
ctgccccggttcatcctgctggannnnnnnncttcagcttcccgatatccgacggtagtgttggctgtgaagacgctgcctg

SEQ ID NO: 945 - DNA, 80 bp, Artificial Sequence
  smMIP
  misc_feature (27)..(34): n is a, c, g, or t
cagacacatggtcctttggagtgctgnnnnnnnncttcagcttcccgatatccgacggtagtgttggagacttcgggatg

SEQ ID NO: 946 - DNA, 83 bp, Artificial Sequence
  smMIP
  misc_feature (22)..(29): n is a, c, g, or t
cccaacgtacggctcctggttnnnnnnnncttcagcttcccgatatccgacggtagtgttctctgttcgagtccctagagggc

SEQ ID NO: 947 - DNA, 83 bp, Artificial Sequence
  smMIP
  misc_feature (24)..(31): n is a, c, g, or t
gcccctggagctggtcattacgannnnnnnncttcagcttcccgatatccgacggtagtgttgctcctagagccctcttcgct

SEQ ID NO: 948 - DNA, 83 bp, Artificial Sequence
  smMIP
  misc_feature (30)..(37): n is a, c, g, or t
gcctgtggggccgacagctatgagatggannnnnnnncttcagcttcccgatatccgacggtagtgttctacaaccccaccac

SEQ ID NO: 949 - DNA, 83 bp, Artificial Sequence
  smMIP
  misc_feature (30)..(37): n is a, c, g, or t
cgtaaaggaaatcacagggtttttgctgannnnnnnncttcagcttcccgatatccgacggtagtgtaaacacttcaaaaact

SEQ ID NO: 950 - DNA, 20 bp, Artificial Sequence
  forward primer HMBSFw
ctggtaacggcaatgcggct

SEQ ID NO: 951 - DNA, 20 bp, Artificial Sequence
  reverse primer HMBSRv
ttcttctccagggcatgttc